European Patent Specification EP 3 458 104 B1, published June 10, 2026. Title: POLYNUCLEOTIDES ENCODING PORPHOBILINOGEN DEAMINASE FOR THE TREATMENT OF ACUTE INTERMITTENT PORPHYRIA. Applicant: MODERNATX, INC. FUNDACION PARA LA INVESTIGACION MEDICA APLICADA. The sequence listing filed with the application follows.

SEQUENCE LISTING (199 sequences)

SEQ ID NO: 1 - protein, 361 aa, Artificial Sequence [sequence omitted]

SEQ ID NO: 2 - DNA, 1083 bp, Artificial Sequence
  nucleotide sequence of wild type PBGD, isoform 1
atgtctggtaacggcaatgcggctgcaacggcggaagaaaacagcccaaagatgagagtgattcgcgtgggtacccgcaagagccagcttgctcgcatacagacggacagtgtggtggcaacattgaaagcctcgtaccctggcctgcagtttgaaatcattgctatgtccaccacaggggacaagattcttgatactgcactctctaagattggagagaaaagcctgtttaccaaggagcttgaacatgccctggagaagaatgaagtggacctggttgttcactccttgaaggacctgcccactgtgcttcctcctggcttcaccatcggagccatctgcaagcgggaaaaccctcatgatgctgttgtctttcacccaaaatttgttgggaagaccctagaaaccctgccagagaagagtgtggtgggaaccagctccctgcgaagagcagcccagctgcagagaaagttcccgcatctggagttcaggagtattcggggaaacctcaacacccggcttcggaagctggacgagcagcaggagttcagtgccatcatcctggcaacagctggcctgcagcgcatgggctggcacaaccgggtggggcagatcctgcaccctgaggaatgcatgtatgctgtgggccagggggccttgggcgtggaagtgcgagccaaggaccaggacatcttggatctggtgggtgtgctgcacgatcccgagactctgcttcgctgcatcgctgaaagggccttcctgaggcacctggaaggaggctgcagtgtgccagtagccgtgcatacagctatgaaggatgggcaactgtacctgactggaggagtctggagcctagacggctcagatagcatacaagagaccatgcaggctaccatccatgtccctgcccagcatgaagatggccctgaggatgacccacagttggtaggcatcactgctcgtaacattccacgagggccccagttggctgcccagaacttgggcatcagcctggccaacttgttgctgagcaaaggagccaaaaacatcctggatgttgcacggcagcttaacgatgcccat

SEQ ID NO: 3 - protein, 344 aa, Artificial Sequence
  polypeptide sequence of wild type PBGD, isoform 2
MRVIRVGTRKSQLARIQTDSVVATLKASYPGLQFEIIAMSTTGDKILDTALSKIGEKSLFTKELEHALEKNEVDLVVHSLKDLPTVLPPGFTIGAICKRENPHDAVVFHPKFVGKTLETLPEKSVVGTSSLRRAAQLQRKFPHLEFRSIRGNLNTRLRKLDEQQEFSAIILATAGLQRMGWHNRVGQILHPEECMYAVGQGALGVEVRAKDQDILDLVGVLHDPETLLRCIAERAFLRHLEGGCSVPVAVHTAMKDGQLYLTGGVWSLDGSDSIQETMQATIHVPAQHEDGPEDDPQLVGITARNIPRGPQLAAQNLGISLANLLLSKGAKNILDVARQLNDAH

SEQ ID NO: 4 - DNA, 1032 bp, Artificial Sequence
  nucleotide sequence of wild type PBGD, isoform 2
atgagagtgattcgcgtgggtacccgcaagagccagcttgctcgcatacagacggacagtgtggtggcaacattgaaagcctcgtaccctggcctgcagtttgaaatcattgctatgtccaccacaggggacaagattcttgatactgcactctctaagattggagagaaaagcctgtttaccaaggagcttgaacatgccctggagaagaatgaagtggacctggttgttcactccttgaaggacctgcccactgtgcttcctcctggcttcaccatcggagccatctgcaagcgggaaaaccctcatgatgctgttgtctttcacccaaaatttgttgggaagaccctagaaaccctgccagagaagagtgtggtgggaaccagctccctgcgaagagcagcccagctgcagagaaagttcccgcatctggagttcaggagtattcggggaaacctcaacacccggcttcggaagctggacgagcagcaggagttcagtgccatcatcctggcaacagctggcctgcagcgcatgggctggcacaaccgggtggggcagatcctgcaccctgaggaatgcatgtatgctgtgggccagggggccttgggcgtggaagtgcgagccaaggaccaggacatcttggatctggtgggtgtgctgcacgatcccgagactctgcttcgctgcatcgctgaaagggccttcctgaggcacctggaaggaggctgcagtgtgccagtagccgtgcatacagctatgaaggatgggcaactgtacctgactggaggagtctggagcctagacggctcagatagcatacaagagaccatgcaggctaccatccatgtccctgcccagcatgaagatggccctgaggatgacccacagttggtaggcatcactgctcgtaacattccacgagggccccagttggctgcccagaacttgggcatcagcctggccaacttgttgctgagcaaaggagccaaaaacatcctggatgttgcacggcagcttaacgatgcccat

SEQ ID NO: 5 - protein, 321 aa, Artificial Sequence
  polypeptide sequence of wild type PBGD, isoform 3
MSGNGNAAATAEENSPKMRVIRVGTRKSQLARIQTDSVVATLKASYPGLQFEIIAMSTTGDKILDTALSKIGEKSLFTKELEHALEKNEVDLVVHSLKDLPTVLPPGFTIGAICKRENPHDAVVFHPKFVGKTLETLPEKSVVGTSSLRRAAQLQRKFPHLEFRSIRGNLNTRLRKLDEQQEFSAIILATAGLQRMGWHNRVGQILHPEECMYAVGQEGGCSVPVAVHTAMKDGQLYLTGGVWSLDGSDSIQETMQATIHVPAQHEDGPEDDPQLVGITARNIPRGPQLAAQNLGISLANLLLSKGAKNILDVARQLNDAH

SEQ ID NO: 6 - DNA, 963 bp, Artificial Sequence
  nucleotide sequence of wild type PBGD, isoform 3
atgtctggtaacggcaatgcggctgcaacggcggaagaaaacagcccaaagatgagagtgattcgcgtgggtacccgcaagagccagcttgctcgcatacagacggacagtgtggtggcaacattgaaagcctcgtaccctggcctgcagtttgaaatcattgctatgtccaccacaggggacaagattcttgatactgcactctctaagattggagagaaaagcctgtttaccaaggagcttgaacatgccctggagaagaatgaagtggacctggttgttcactccttgaaggacctgcccactgtgcttcctcctggcttcaccatcggagccatctgcaagcgggaaaaccctcatgatgctgttgtctttcacccaaaatttgttgggaagaccctagaaaccctgccagagaagagtgtggtgggaaccagctccctgcgaagagcagcccagctgcagagaaagttcccgcatctggagttcaggagtattcggggaaacctcaacacccggcttcggaagctggacgagcagcaggagttcagtgccatcatcctggcaacagctggcctgcagcgcatgggctggcacaaccgggtggggcagatcctgcaccctgaggaatgcatgtatgctgtgggccaggaaggaggctgcagtgtgccagtagccgtgcatacagctatgaaggatgggcaactgtacctgactggaggagtctggagcctagacggctcagatagcatacaagagaccatgcaggctaccatccatgtccctgcccagcatgaagatggccctgaggatgacccacagttggtaggcatcactgctcgtaacattccacgagggccccagttggctgcccagaacttgggcatcagcctggccaacttgttgctgagcaaaggagccaaaaacatcctggatgttgcacggcagcttaacgatgcccat

SEQ ID NO: 7 - protein, 304 aa, Artificial Sequence
  polypeptide sequence of wild type PBGD, isoform 4
MRVIRVGTRKSQLARIQTDSVVATLKASYPGLQFEIIAMSTTGDKILDTALSKIGEKSLFTKELEHALEKNEVDLVVHSLKDLPTVLPPGFTIGAICKRENPHDAVVFHPKFVGKTLETLPEKSVVGTSSLRRAAQLQRKFPHLEFRSIRGNLNTRLRKLDEQQEFSAIILATAGLQRMGWHNRVGQILHPEECMYAVGQEGGCSVPVAVHTAMKDGQLYLTGGVWSLDGSDSIQETMQATIHVPAQHEDGPEDDPQLVGITARNIPRGPQLAAQNLGISLANLLLSKGAKNILDVARQLNDAH

SEQ ID NO: 8 - DNA, 912 bp, Artificial Sequence
  nucleotide sequence of wild type PBGD, isoform 4
atgagagtgattcgcgtgggtacccgcaagagccagcttgctcgcatacagacggacagtgtggtggcaacattgaaagcctcgtaccctggcctgcagtttgaaatcattgctatgtccaccacaggggacaagattcttgatactgcactctctaagattggagagaaaagcctgtttaccaaggagcttgaacatgccctggagaagaatgaagtggacctggttgttcactccttgaaggacctgcccactgtgcttcctcctggcttcaccatcggagccatctgcaagcgggaaaaccctcatgatgctgttgtctttcacccaaaatttgttgggaagaccctagaaaccctgccagagaagagtgtggtgggaaccagctccctgcgaagagcagcccagctgcagagaaagttcccgcatctggagttcaggagtattcggggaaacctcaacacccggcttcggaagctggacgagcagcaggagttcagtgccatcatcctggcaacagctggcctgcagcgcatgggctggcacaaccgggtggggcagatcctgcaccctgaggaatgcatgtatgctgtgggccaggaaggaggctgcagtgtgccagtagccgtgcatacagctatgaaggatgggcaactgtacctgactggaggagtctggagcctagacggctcagatagcatacaagagaccatgcaggctaccatccatgtccctgcccagcatgaagatggccctgaggatgacccacagttggtaggcatcactgctcgtaacattccacgagggccccagttggctgcccagaacttgggcatcagcctggccaacttgttgctgagcaaaggagccaaaaacatcctggatgttgcacggcagcttaacgatgcccat

SEQ ID NO: 9 - RNA, 1083 nt, Artificial Sequence
  PBGD-CO01
augagcgggaacggcaacgccgcagccaccgccgaggagaacagccccaagaugcgggucaucagggugggcacgcggaagucccaguuggcacgcauacagaccgacagcguaguggcgacccugaaggccuccuaccccggccuccaguucgagaucaucgccaugagcaccaccggggacaagauccucgauaccgcccuguccaagaucggcgagaaguccuuguuuaccaaggagcuggagcacgcccuggagaagaaugagguggaccuuguggugcacagccucaaggaccugcccaccgugcugccccccggguucaccauaggagccaucugcaagagggagaacccgcacgacgcagucguguuccaccccaaguuuguggguaagacacuggagacccugcccgagaagagcgugguggguaccuccagccuccgccgagcagcccagcugcagaggaaguucccgcaccuggaauuccgauccaucaggggcaaucugaacaccagacugaggaagcuggaugagcagcaggaauuuuccgcgauaauccucgcgaccgccgggcugcagaggaugggcuggcauaacagggugggccaaauccugcaccccgaggagugcauguacgccgugggccagggcgcccucggcguggaggugagggccaaagaccaagacauccuggaccugguggggguccugcacgauccggagacucugcugaggugcaucgccgagcgggcguuucucaggcaccucgagggcggcugcuccgugcccguggccguccauaccgccaugaaggacggccagcuguaccucaccggcggcguguggagccuggacggcagcgacuccauacaggaaaccaugcaagcgaccauacauguccccgcccagcacgaggacgggcccgaggaugacccgcagcuggucgguaucaccgcaaggaauaucccccggggcccacagcuggccgcccagaaucugggcaucucccuggccaaucugcugcuguccaagggcgccaagaacauccucgacguggccaggcaacugaacgacgcacac

SEQ ID NO: 10 - RNA, 1083 nt, Artificial Sequence
  PBGD-CO02
augagcggcaacgguaacgccgccgccaccgccgaggagaacucgcccaagaugcgggucaucagggugggaacgaggaagucccagcuggccaggauccagaccgacagcgugguggcgacgcugaaggccagcuaccccggccugcaguuugagauaaucgccaugucaaccaccggcgacaagauccucgacaccgcgcugagcaagaucggcgagaagucccuguucaccaaggagcuggagcacgccuuggaaaagaacgagguggaucuggucgugcacagccugaaggaccugcccaccgugcugccccccggcuucaccaucggcgccaucugcaagcgggaaaauccccaugacgccgugguguuccaccccaaguucguggggaagacccuggagacccugccggagaagagcguggugggaaccagcucacugcggcgggccgcccagcugcaacguaaguucccccaucuggaguuccgauccauccgaggcaaucugaacaccaggcugagaaagcuggaugaacaacaggaguucagcgccaucauccuggcaaccgccggucugcagaggaugggcuggcacaacagggugggccaaauccugcaccccgaggagugcauguaugcaguggggcagggcgcgcugggugucgaggugcgagcgaaggaccaggacauccucgaccuggugggagugcugcacgaccccgagacccugcugcggugcaucgccgagagggccuuccugcgccaccucgagggcggcugcucagugcccguggccgugcauaccgccaugaaggacggccagcuguaccugaccggcgguguguggagccucgacggcagcgacuccauccaggaaacgaugcaggcgacuauccacgugcccgcacagcacgaggacggcccggaagacgacccccagcuggucgggaucaccgccaggaacaucccccgagggccccagcuggcggcccaaaaccucggcauaucccuggccaaccugcugcuguccaagggcgccaagaacauccuggauguggcccgccaacugaacgacgcccac

SEQ ID NO: 11 - RNA, 1083 nt, Artificial Sequence
  PBGD-CO03
augagcgguaacggcaacgccgccgccacagccgaagagaacucccccaagaugagggugauuaggguggguacccgaaagagccagcuggcccggauccagaccgacuccgugguggccacccucaaggcaagcuaccccggccugcaguucgagaucaucgccaugagcaccaccggggacaaaauucucgacaccgcccugagcaagaucggcgagaaguccuuguucaccaaggagcuagagcacgcccucgaaaagaacgagguggaucuggucgugcacucccugaaggaccugcccaccgugcugccccccggcuucacgaucggcgcgaucugcaagagggagaacccgcaugacgccgugguguuucaucccaaauuugugggaaaaacccuggagacucuccccgagaagagcgucgucgggaccuccucccugcggcgggccgcccagcugcagcgcaaguucccgcaccuggaguuccgcagcaucaggggaaaccugaacacccggcugaggaagcuggacgagcagcaggaguucagcgcuaucauccucgccaccgccggccuccagcgaaugggcuggcauaaccgggugggccagauccugcacccggaagaauguauguacgcggugggccagggcgcgcugggcguggaggugagggccaaggaccaggacauccuggaucucgugggcgugcugcacgaccccgagacccugcugagaugcaucgcagaacgggccuuccugaggcaccuggagggcggcugcuccgugccgguggccguacauaccgcaaugaaagacggccagcucuaccugacgggggggguguggagccucgacggcuccgacuccauccaggagaccaugcaggcgacgauccauguacccgcccagcacgaggacggccccgaggaugauccccaacucgugggcaucaccgcccgcaacaucccgaggggcccccagcuggccgcacagaaccugggaauaucacuggccaaccuccugcucagcaagggcgccaagaauauccucgacguggccaggcagcugaaugacgcccac

SEQ ID NO: 12 - RNA, 1083 nt, Artificial Sequence
  PBGD-CO04
augagcggcaacggcaacgccgccgccaccgccgaggagaacagccccaaaaugcgcgugaucagggugggcaccaggaagagccagcuggcccgcauccagaccgacagugucguggccacccucaaggccagcuauccgggccugcaauucgagaucaucgccaugagcaccaccggcgacaagauccucgacaccgcccucagcaagaucggcgagaagucccuguucaccaaggagcuggagcacgcccuggagaagaacgagguggaccugguggugcacagccucaaggaccugcccaccgugcugccccccggcuucaccaucggcgccaucugcaagcgggagaacccccacgacgccgugguguuccaucccaaguucgugggcaagacccuggagacccugcccgagaagagcguggucggcaccagcucccucaggagagccgcccagcugcagcgaaaguucccccaccuggaauuccgcagcauccgggggaaccugaacacccgccugaggaagcuggacgagcagcaagaauucagcgccaucauccuggccaccgcgggccugcagaggaugggguggcacaaccgcgucggccagauccugcacccagaggagugcauguacgcgguggggcagggggccuuggggguggaagugcgcgccaaggaccaggacauccuggaccuggucggcgugcugcaugaccccgagacccugcucaggugcaucgccgagagggccuuucugcgccaccucgagggggguugcagcgugccggucgccguccauacggccaugaaggacgggcagcuguaccugaccggcggcguguggucccuggacggcuccgacagcauccaggagaccaugcaggccaccauccacgugcccgcccaacacgaggacggccccgaggacgacccgcagcucgucggcaucaccgccaggaauauaccccguggcccccagcuggccgcccagaaucucggcaucagccuggccaaucugcugcugagcaagggggccaagaacauccuggacguggccaggcagcugaaugaugcccac

SEQ ID NO: 13 - RNA, 1083 nt, Artificial Sequence
  PBGD-CO05
augagcggcaacggaaacgccgccgcgacggccgaggagaacucccccaaaaugagggucaucagggugggcacccggaagagccagcuggcgcggauccagaccgacagcgucguggccacccucaaagccagcuacccaggccugcaguucgagaucaucgccaugucgaccaccggggacaagauccuggauaccgcccucagcaagaucggcgagaagucccuguucaccaaggagcucgagcacgcccuggagaagaaugagguggaucugguggugcauucccugaaagaccugccgaccguccugccccccggcuucacgaucggagccaucugcaaacgggagaacccccacgacgcugugguguuccacccgaaguucguggguaagacccuggaaacacugcccgagaaguccguggugggcaccagcagccugaggcgggcggcccaacugcagaggaaguucccccaccucgaguucagaagcauccgggggaaccugaauacccggcugcgcaagcuggacgagcagcaggaguucagcgccaucauccuggccaccgcuggccugcagaggaugggauggcacaaccgugugggccagauccugcacccggaggagugcauguacgccguggggcagggcgcgcugggcguggaggugcgcgcgaaggaccaggacauccuggaccuugucggcgugcugcacgaucccgagacgcugcugaggugcaucgccgagagggccuuccugaggcaccuggaagggggcuguagcguccccguggcuguccacaccgccaugaaggacggccagcuguaccugaccggcggcguguggucccuggacggcagcgacagcauccaggagaccaugcaggccaccauccacguccccgcccaacacgaagacggcccggaggacgacccccagcugguaggcauaacugcccgcaauauccccagggggccccaacuggccgcccagaaccugggcauaagccuggcgaaccugcugcuguccaagggcgccaagaacauccuggacgucgcccgccagcugaacgacgcccac

SEQ ID NO: 14 - RNA, 1083 nt, Artificial Sequence
  PBGD-CO06
augagcggcaacggcaacgccgccgccaccgccgaggagaauucccccaaaaugagggugauccgcgugggcacgaggaagagccagcuggcccggauccagacggacagcgugguggccacccugaaggccucguaucccgggcugcaguucgagaucaucgccaugagcaccaccggcgacaagauccucgacaccgcccuguccaagaucggcgagaaaagccuguucaccaaggaacuggagcacgcacuggaaaagaacgagguagaccucguggugcauucccugaaggaccugcccaccgugcugcccccaggcuucaccaucggcgccaucugcaagcgagagaacccccaugaugccgugguguuccacccgaaguuuguuggcaagacgcuggagacccugcccgagaagagcguagugggcaccagcucgcugcggagggccgcccagcugcagaggaaguucccccaccuggaguuuaggagcauuaggggcaaccugaacaccaggcucaggaagcuggacgagcagcaggaguucuccgcuauaauccuggccaccgccgggcugcagaggaugggguggcacaacaggguggggcaaauccugcaccccgaagagugcauguacgccgucggccagggggcccugggcguugagguucgcgccaaggaucaggacauccuggaccuggugggggugcugcaugaccccgagacccugcugaggugcaucgcggaaagggccuuccugcgccaccuggagggcggcugcagcgugcccguggccgugcacaccgcgaugaaggacggccagcuguaccugaccgggggggucuggucccuggacggcuccgacagcauccaggagacgaugcaggccacgauccacgugcccgcccaacacgaggacggucccgaagaugauccccagcuggucggcaucaccgcaaggaacauccccaggggcccccagcuggccgcacagaaccugggcaucucgcuggccaaccugcugcugagcaagggggccaagaacauccucgacguggccaggcagcuaaacgacgcccac

SEQ ID NO: 15 - RNA, 1083 nt, Artificial Sequence
  PBGD-CO07
auguccggcaacggcaacgcugccgccacggccgaggagaacagccccaagaugagggugauccgggugggcaccagaaagucccagcucgccaggauccagacugauagcguggucgccacccucaaagccagcuacccgggccugcaguuugagaucaucgccauguccacaaccggcgacaagauccuggacacagcgcugucgaagaucggcgaaaaaagccucuucaccaaggagcuggagcacgcccuggagaagaaugagguggaccugguggugcauucccugaaggaccugcccaccgugcugccccccggcuucaccaucggcgccaucugcaagagggagaacccacacgacgccguggucuuccaccccaaguucguggggaaaacccucgaaacccuccccgaaaaguccguggugggcaccuccagccugaggcgggcggcccagcugcagaggaaguucccacaccucgaguuccgcagcauccggggcaaucugaacaccaggcucaggaagcuggacgagcagcaggaguucagcgccaucauccuggccaccgcgggccuccagaggaugggcuggcacaacagggugggccagauccuccaccccgaggaauguauguacgccguggggcaaggcgcccugggcguggagguccgggcgaaggaccaggacauccuggaccuggucggcgugcugcacgaucccgagacgcugcucaggugcaucgccgaacgcgccuuccuccggcaccucgaggggggcugcagcgugccgguggccguccacaccgccaugaaggacggccagcuguaccugaccggcggcgucuggagccuggacggcuccgacuccauccaggagacgaugcaggccaccauccaugugccagcccagcaugaggacggcccggaagacgacccccaacuggugggcaucaccgcccggaacauccccaggggcccucagcucgccgcacagaaucuuggcaucagccucgccaaucuccugcugagcaagggagccaagaacauccucgacguggccaggcagcugaacgacgcccau

SEQ ID NO: 16 - RNA, 1083 nt, Artificial Sequence
  PBGD-CO08
augagcggcaacggcaacgccgccgccaccgccgaggagaauagccccaagaugcgggugauccgcgugggcacccgcaagagccagcuggcccggauccagaccgacuccgucguggccacccugaaggccagcuaccccggacuccaguucgagaucaucgccaugucgaccacgggcgacaagauccucgacaccgcccucagcaaaaucggagagaagucccuguucaccaaggagcucgaacacgcccuggaaaagaacgagguggaccugguggugcacucccugaaggaccugcccaccgugcucccccccggauuuaccaucggagccaucugcaagcgggagaacccucacgacgccgugguguuccaucccaaguucguggggaagacgcuggaaacccugccggagaagagcguagugggcaccagcagccugcggagggccgcccagcugcagaggaaguucccccaccuggaguuucguagcauccgcggcaaucugaacacgcggcugcgcaagcucgacgagcagcaggaguucuccgcgaucauacuggccaccgccggccugcagcggaugggguggcacaaccgggucggccagauccugcaccccgaggagugcauguacgccgugggccagggggccuugggcguggaggugagggccaaggaccaggacauccuggaccucgugggcgucuugcacgaccccgaaacccugcugaggugcaucgccgagcgggccuuucugaggcaccuggagggcgggugcagcgugcccguggccguccacaccgcaaugaaggacgggcagcuguaccugaccggcggggucuggagccuggacggcagcgauucgauacaggagacaaugcaagccacgauccacguccccgcccagcacgaggacgggcccgaggacgacccccaacuggucgggaucaccgcccggaacauccccagggggccgcagcuggccgcccagaaccugggcaucucccuggccaaccugcugcugagcaaaggcgccaagaacauucuggauguggcccgccagcugaacgaugcccac

SEQ ID NO: 17 - RNA, 1083 nt, Artificial Sequence
  PBGD-CO09
augagcgggaacggcaacgccgccgccaccgccgaggagaacaguccgaagaugaggguaaucagggucgggacccguaagagccagcucgccaggauccagaccgacagcgugguggccacccugaaggccagcuauccagggcugcaguucgagaucaucgccauguccaccaccggggacaaaauccuggacaccgcccugagcaagauaggcgagaagagccuguucaccaaggaacuggagcaugcccuggaaaagaacgagguggaccuggucgugcacagccugaaggaccugcccaccgugcugccccccggcuucaccaucggcgcgaucugcaaaagggagaacccccacgacgcuguggucuuccacccaaaauucguggggaagacucucgagacccugcccgagaagagcgugguggguacuuccagccugaggagggccgcccagcugcaaaggaaguucccccaucuggaguucaggagcauccggggcaaccugaauaccaggcugcgcaagcuggaugagcagcaggaauucagcgccaucauccuggccaccgccggccugcagaggaugggcuggcacaacagggucggccagauccugcaccccgaggagugcauguaugccgugggccagggugcccugggaguggaggucagggcgaaggaccaggacauccuugaccuugucggcgugcugcacgaccccgagacccugcucaggugcaucgccgagagggccuuccugaggcaucuggaggggggguguagcgugcccgucgcagugcacaccgccaugaaggacggccaacuguaccugaccggcggcguguggagccuggacggcucugauucgauccaagagaccaugcaagccacuauacacgugcccgcccagcacgaggacgggcccgaggaugacccacagcuggucggaaucaccgcccggaacauccccaggggaccccagcuggccgcgcagaaucugggcaucucacuggccaaccugcugcucuccaagggggccaagaacauccuggacguggcuaggcagcugaacgacgcccac

SEQ ID NO: 18 - RNA, 1083 nt, Artificial Sequence
  PBGD-CO10
augagcggcaacggaaacgccgccgccaccgccgaggaaaacucccccaaaaugcgggucaucagggugggcaccaggaagucccagcucgccaggauacaaaccgacuccgugguagccacccugaaggccagcuaccccgggcuccaguucgagaucaucgccaugagcacaaccggugacaagauucuugacaccgcccucagcaagauaggcgagaagagccuguucaccaaggagcuggaacaugcccuggaaaagaacgaggucgaccucgucgugcacagccugaaggaccugcccacggugcugccacccggcuucacgaucggcgccaucugcaaaagagagaauccccaugacgcggugguguuucaccccaaguuuguggggaagacccuggagacccugcccgagaagagcgugguggggacgagcagccugcgcagggccgcccagcugcagcggaaguucccccaucuggaguuuaggagcaucagggggaaccugaacacgaggcugaggaagcuggacgagcagcaggaauucagcgccaucauccuggcgaccgccggccugcagcggaugggcuggcauaaccgcgugggacagauacugcaccccgaggaaugcauguacgcggucggccaaggcgcgcugggcguggaggugagggccaaagaucaggauauccuagaccucgugggcgugcuucacgaccccgagacacugcugaggugcaucgccgagagggcguuucugcggcaccuggagggcgggugcagcgugccgguggccgugcauaccgccaugaaggacggccagcuguaccugacgggggggguguggagccucgacggcucggacagcauccaggagacgaugcaggccacgauacacgugcccgcccagcacgaagacggacccgaggaugacccccagcugguggggaucacagccaggaacauccccaggggcccccaacucgccgcccagaaccuggggauuagccuggccaaccugcuccucuccaagggcgccaagaacauccuggacguggccaggcagcugaacgaugcccau

SEQ ID NO: 19 - RNA, 1083 nt, Artificial Sequence
  PBGD-CO011
auguccggcaacgggaacgcagccgcgaccgccgaggagaacucccccaagaugcgcgugauuagggucgggacgaggaagagccagcuggccaggauacagaccgauuccgugguggccacccucaaggccagcuacccugggcugcaauucgagaucauagccaugagcaccaccggcgauaagauacuggacaccgcccucagcaagaucggugagaagucgcuguuuaccaaggaacuggagcacgcccuggagaagaaugaaguggaucuggucguacacagcuugaaggaccugcccaccgugcugccccccggauucaccaucggggccaucugcaagagggagaacccccacgacgccgugguguuccaccccaaauucgucggcaagacccuggaaacccugcccgaaaagagcguggugggcaccuccagccugcgcagggccgcccagcugcagaggaaguucccccaccuggaguucaggagcauacggggcaaccugaacacccgacugaggaagcuggacgaacagcaagaguucagcgccaucauccuggcaaccgccggccugcagaggaugggcuggcacaacagggugggccagauccugcaccccgaggaguguauguacgccguaggccagggcgcccucggaguggaggucagggccaaggaccaggacauccucgaccuggugggugugcugcacgaccccgagacacugcugaggugcaucgccgagagggccuuucugaggcaccucgaaggcggcugcuccgugcccguggccgugcacaccgccaugaaagacggucagcuguacuugaccgguggcguguggagccucgacggcagcgacagcauccaggagacaaugcaggccaccauccacguccccgcacagcacgaagacgggccugaggacgacccccagcuggugggaaucaccgccaggaauaucccccgaggcccccagcuggcggcccagaaccugggcauuucccuggccaaccuccugcugagcaaaggugccaagaauauccuggacguggcccggcagcugaaugacgcccac

SEQ ID NO: 20 - RNA, 1083 nt, Artificial Sequence
  PBGD-CO012
augagcgggaacgggaacgccgccgccaccgccgaggagaauucccccaagaugagggugauaaggguagggaccaggaagagccagcuggccaggauccagacugacagcgugguugccacccugaaggccagcuaccccggucugcaguucgagaucaucgccauguccaccaccggugacaagauucuggacaccgcccuguccaagaucggagaaaagagccuguucaccaaggaacucgaacacgcccuugagaagaaugaaguggaccugguggugcacucccucaaggaccuacccaccgugcugccccccggcuuuaccaucggcgccaucugcaagagggagaacccccaugacgcggugguguuucaccccaaauucgugggaaagacccuggagacacugcccgagaaguccguggugggcaccagcagccugaggagggccgcccagcugcagaggaaguucccccaucuggaguuuaggagcaucaggggcaaccugaacacccggcugaggaagcuggaugaacagcaggaguucagcgccaucauccuggccacggcgggccugcagcggaugggguggcauaaccggguggggcagauccugcaccccgaagaaugcauguaugcgguagggcaaggggcccugggcgucgaggugcgggccaaggaccaggacauacuggaccuggugggggugcugcaugaucccgaaacccugcuccggugcaucgccgagagggccuuccucaggcaccuggagggcggaugcucggugcccgucgccgugcauaccgccaugaaggacggccagcucuaccucaccggcggcguuuggucccuggauggaagcgacagcauucaggaaaccaugcaggccaccauccacgugccagcgcagcacgaggacggccccgaggacgacccccagcuagugggcaucaccgccaggaacaucccccggggcccccagcuggccgcacagaaccuaggcaucagccuggccaaccuccugcugagcaagggcgccaagaacauccuggauguggccaggcagcugaacgacgcccac

SEQ ID NO: 21 - RNA, 1083 nt, Artificial Sequence
  PBGD-CO013
auguccgguaacggcaacgcggccgccaccgccgaggagaacagccccaagaugagggugauccgcgugggcaccaggaagagccagcuggccaggauccaaaccgacagcguggucgccacgcugaaggccagcuacccaggucugcaauucgagaucaucgccaugagcaccaccggggacaaaauccuggauaccgcccuguccaagaucggcgagaagagccuguucaccaaggagcuggaacacgcccuggagaagaacgagguggaccuggucgugcacagccugaaggaccugcccaccguccugccccccggguucaccaucggcgccauuugcaagcgagagaacccacacgacgccgucguguuccaccccaaguucgucggcaagacgcucgagacccugcccgagaagagcguggucgggacgagcucccuccggcgcgccgcccagcuccagcgcaaauuuccccauuuagaguuccguagcauccguggcaaccugaacacgcgucugaggaagcuggaugaacaacaggaguucagcgccaucauccuggccaccgccggccugcagaggaugggcuggcacaaccgugugggccagauccuucaucccgaggagugcauguacgcugucggccagggggcucuggggguggaagucagggccaaggaccaggacauccuggaucuggucggcgugcuccacgaccccgagacucugcugagguguaucgcagagagggcguuccucaggcaccucgagggcgggugcagcgucccuguggcggugcacaccgccaugaaggacgggcagcuguaccucaccggcggcguguggucccuggauggcagcgacagcauccaggagacgaugcaggccaccauccacgugcccgcccagcacgaggacggccccgaggacgacccccaacuggucggcaucaccgcccgcaacauccccagggggccccaacuggccgcccagaaucugggcaucucccuggccaaccugcuccugagcaagggugccaagaacauccucgacguggccaggcagcucaacgacgcccac

SEQ ID NO: 22 - RNA, 1083 nt, Artificial Sequence
  PBGD-CO014
augagcggcaacggcaacgccgcagccaccgccgaggagaacucccccaagaugagggugaucagggugggcaccaggaagucccaacuggcgcggauccagaccgacagcgugguggccacccugaaggcguccuaccccggccuccaguucgagauuaucgccaugagcaccaccggcgacaagauccuggauaccgcccugagcaagaucggggaaaaaagccuguucaccaaggagcuggagcacgcccuggagaagaacgagguggaucucgugguacacucccugaaggauuugcccaccgugcugccccccggguucaccaucggggccaucuguaaaagggagaauccccacgacgccgugguguuccaccccaaguucgugggcaagacccuggagacccuccccgagaagagcguggucggaaccagcagccugcgccgcgccgcucagcuacaacgcaaguucccccaccuggaguuccggagcaucagggggaaccugaacacccgucugcggaagcucgacgagcagcaggaguucagcgcuaucauccuggcuacggccgggcugcagaggaugggauggcacaacagggucgggcagauccugcaucccgaggagugcauguacgccgugggccaaggcgcccucggaguggaagucagggccaaagaccaagacauccuggaccuagucggcgugcugcaugaccccgagacccugcuccgcugcaucgccgagagggcguuccugcgccaucuggaggggggcugcagcgugccgguggccgugcauacagcuaugaaagauggccaacuguaccucaccggcggcgucuggagccuggacggcucggacuccauucaagagacgaugcaggccacgauccacgugcccgcgcagcacgaggaugggcccgaggacgauccccagcugguaggcaucaccgcccggaacaucccccggggcccgcagcuggccgcccagaaccuggggaucucccuggccaaccuccugcugucgaagggggccaagaacauccuggaugucgccaggcagcugaacgacgcccac

SEQ ID NO: 23 - RNA, 1083 nt, Artificial Sequence
  PBGD-CO015
auguccgggaacgggaacgcggccgccacggcggaggagaacucccccaaaaugagggugauaagggugggcacccggaaaagccagcuggcucgaauccagaccgacagcgugguggccacccugaaagccuccuaccccggccuccaguuugagaucaucgccaugagcaccaccggcgacaagauccucgacaccgcccugagcaagaucggugaaaagucgcuguucacgaaggagcuggagcacgcccuagagaagaacgaggucgaccuggugguccacagccugaaggaccugcccaccguccucccccccggauuuaccauuggagccauaugcaaacgggagaacccccaugacgccguggucuuccaccccaaguucgucggcaagacccuggagacccucccggagaaguccgugguggggaccagcagccugcgcagggccgcccagcugcagaggaaauucccccaucuggaauucagguccaucagggggaaccucaacacccggcugcggaagcucgacgaacaacaggaauucagcgccaucauccuggccaccgcggggcugcagaggaugggguggcacaacagggugggacagauccugcaccccgaggaguguauguacgccguggggcagggagcccugggcgucgagguaagggcgaaggaucaggacauccuggaucuggugggggugcugcacgaccccgagacccugcuccggugcauugccgagagggccuuccugaggcaccuggagggcggcuguagcgugcccguggccgugcacacagcgaugaaagacggccagcuguaucugaccgggggcguguggucccucgauggcucagacuccauccaggagacgaugcaggccaccauccaugugcccgcccagcacgaggacggccccgaggacgacccccagcucguggggaucaccgcccguaacauacccaggggcccccagcuggccgcccagaaucuggggauuagccucgccaaccugcugcugagcaagggcgccaagaacauccuggacguggcccggcagcugaacgacgcccau

SEQ ID NO: 24 - RNA, 1083 nt, Artificial Sequence
  PBGD-CO016
auguccggcaacgggaacgccgccgccacugccgaggagaacagccccaagaugagggugauuagggugggcacccguaagagccagcucgccaggauccagaccgacagcguggucgcgacccucaaggccuccuaccccggccugcaguucgaaaucaucgccaugagcaccacgggggacaaaauccuggauaccgcccugagcaagauaggugagaagagccuguucaccaaggaacuggagcacgcccuggaaaagaacgaagucgaccucguggugcacucccugaaggaccuccccaccgugcugccgcccggcuucaccaucggagccaucugcaagagggagaacccccacgacgccgugguauuucaccccaaguucgucggcaagacccuggagacccugcccgagaagagcgugguaggcaccagcucccuccgcagggccgcccaacuccaaaggaaguucccccaccucgaguuccggagcaucaggggaaaucugaacaccaggcugaggaagcucgaugagcagcaggaguucuccgccaucauccuggccaccgccggacugcaaaggaugggguggcacaaccgcguugggcaaauccugcaccccgaagagugcauguacgccguggggcagggcgcacucgggguggaggugagggccaaggaccaggacauccuggaccucguaggcguacugcacgaccccgagacccugcugcgcuguaucgcugagagggccuuucugcggcaccuggagggcggcugcagcgugcccgucgccgugcacaccgccaugaaagacggccagcucuaucugacgggggggguguggagccuggacggcagcgacagcauccaggagacaaugcaggccaccauccacgugcccgcccagcacgaggacgggcccgaagacgacccccagcucgugggcaucacggcccguaacauccccaggggcccgcaacuggccgcgcagaaccugggcaucucgcuggccaaucugcugcugagcaagggugccaagaacauccuggauguugcccgacagcugaaugacgcccac

SEQ ID NO: 25 - RNA, 1083 nt, Artificial Sequence
  PBGD-CO017
augagcggcaacgguaacgccgccgcgaccgcggaggagaacucacccaagaugcgggucaucaggguaggcaccaggaagagccagcuggccaggauacagaccgacagcgugguggccacgcugaaggcguccuauccgggccugcaauucgaaauuaucgccaugagcacgaccggggacaagauccuggacaccgcgcugagcaaaaucggcgagaagagccucuucaccaaagagcuggagcaugcccuggagaagaacgagguggaccuggucgugcauucacugaaggaucuccccaccgugcugcccccuggcuuuaccaucggagccaucugcaagcgcgaaaacccccacgaugccguggucuuccaccccaaguucguagggaagacccuugagacccugccggagaagucgguggucgggaccagcagccugcggagggccgcccagcuccagaggaaguucccgcaccuugaguucaggagcauccggggcaaucugaauaccaggcugaggaagcuggacgagcagcaagaguucagugccaucauccucgccaccgccggccugcagaggaugggguggcacaacagggugggacagauccugcaucccgaggagugcauguacgccgugggccagggcgcccucggcguggaagugcgggccaaggaccaggacauucuggaccuggugggcgugcugcacgaucccgagacccugcugcgaugcaucgccgagcgcgccuucuuaaggcaccucgagggggguugcagcgugcccguggcagugcacaccgccaugaaggacggccagcuguaccugaccgggggcguguggagccuggacggcucggacagcauccaggagacaaugcaggccaccauccacgugccagcucaacaugaggauggccccgaggacgauccgcagcuggugggaaucaccgcccggaacaucccuaggggcccccaacuggcagcccaaaaccugggcauaagccuggccaaccugcugcucuccaagggcgccaagaacauucuggacgucgcgaggcagcugaacgacgcccac

SEQ ID NO: 26 - RNA, 1083 nt, Artificial Sequence
  PBGD-CO018
augagcggcaacggcaacgccgccgcgaccgccgaggagaauagccccaaaaugagggugauccgggugggcacccggaagucccagcuggcccggauccagaccgacagcgugguggccacccucaaggccagcuaccccggccugcaauucgaaaucaucgccaugagcaccaccggcgacaagauccuggauaccgcccugagcaagaucggcgagaaaagccucuucacuaaggagcuggagcacgcccuggagaaaaacgaaguggaccuggugguccauagccuuaaggaccugcccaccgugcugccccccggcuucaccaucggcgccaucuguaagcgugagaacccgcacgacgccgugguguuccaccccaaguuuguggggaagacccucgagacucuccccgagaaaagcguggugggcacuagcucucugaggagggcagcccagcuccagaggaaauucccccaccucgaguucaggagcaucaggggcaaccugaacacccggcugaggaagcuggacgagcagcaggaguucuccgcgaucauccuggccaccgcgggacugcagcgaaugggcuggcacaaccgggugggccaaauccugcaccccgaggagugcauguacgccgugggccagggggcacuagggguggaggugcgggccaaggaucaggacauccuggaccuggucggggugcugcacgaccccgagacccugcucagaugcaucgccgagcgggcguuccuccggcauuuggaggguggcuguagcgugcccgucgccgugcacaccgccaugaaggacggucagcuguaccucaccgggggcguguggucccuggacggcagcgacagcauccaggagaccaugcaggccaccauccaugugcccgcccagcacgaggacggccccgaggacgacccccagcuggucggcaucaccgccaggaacaucccgagggggccucagcuggccgcucaaaaccuaggcaucagccuggccaaccuccugcucagcaagggcgccaagaauauccuggacgucgccaggcagcugaacgacgcgcau

SEQ ID NO: 27 - RNA, 1083 nt, Artificial Sequence
  PBGD-CO019
augagcggcaacgggaacgccgccgccaccgccgaggagaacagccccaagaugagggugauccgggucgguaccaggaagagccagcuggcccgaauccagaccgauagcgugguggccacgcugaaggccagcuaccccggacugcaguucgagauaaucgcgaugagcacaacgggggacaagauccuggacaccgcccucuccaagaucggcgagaaaagccucuucaccaaagagcuggagcaugcccuggagaagaacgagguagaccucguaguccauagccugaaggaccugcccaccgugcugccccccggauucaccaucggcgccaucuguaagcgcgagaacccccacgacgccguggucuuccaccccaaguucgucggaaagacacuggagacccugcccgaaaagagcguggugggcaccagcagccugaggagggccgcccagcugcagcgcaaguucccccaccuagaauucaggagcauccggggcaacuuaaacaccaggcugaggaagcuggaugagcagcaggaauucagcgccaucauccucgccacggccgggcugcagaggaugggcuggcacaaccgggugggccagauccugcauccggaagagugcauguacgccgugggccagggagcccugggcguggagguccgggccaaggaucaagauauccuggaucuggugggggugcugcacgaccccgagacccugcugcgcugcaucgccgagagggccuuucugcgccaucuggaggggggcugcagcgugcccguggcggugcauaccgccaugaaggacggccagcucuaucugaccggcggggucuggagccuggacgggagcgacagcauccaggagaccaugcaggcgaccauccacgugcccgcccagcacgaggacggccccgaagaugacccccagcugguugggaucaccgcgaggaacauccccaggggcccccagcuagccgcccagaaccuuggcaucucccuggccaaccugcuacucagcaagggugccaagaauauccuggaugucgccaggcagcugaacgacgcccau

SEQ ID NO: 28 - RNA, 1083 nt, Artificial Sequence
  PBGD-CO020
auguccggcaacggcaacgccgccgccaccgccgaggaaaauagccccaagaugcgggugauccgggugggaacacgaaagucccagcucgcccggauccagaccgacagcgugguggccacccugaaggccagcuacccuggccugcaguucgagaucaucgccaugagcaccaccggcgacaagauccuggauacggcccugagcaagaucggggagaaaucccucuucaccaaggaacuggagcacgcccuggagaagaacgagguggaccuggugguccacucccugaaggaccugcccacagugcucccacccggcuucaccaucggcgccaucugcaaacgcgagaacccccacgacgccguggucuuucaccccaaguucguggguaagacccuggagacccugcccgaaaagagcguggugggcaccuccagccugaggcgggccgcccagcugcagaggaaauuuccccaccuggaguuccggagcaucaggggcaaccucaacaccaggcugaggaagcuggacgagcagcaggaauuuagcgcgaucauccuggccaccgccggccugcagaggaugggguggcacaacagggugggacaaauccugcaucccgaggagugcauguacgccgugggccaaggagcucugggcguggaagugagggccaaggaccaggacauccuggaccucgugggcguacugcacgaccccgagacccugcugcggugcauugccgagcgggccuuccuccgucaccucgagggcggcuguuccgugcccguggccgugcauacggccaugaaggauggacagcuguaucugacgggcggcguguggucacuggacgggucggacuccauccaggagaccaugcaggccaccauccacgugcccgcccagcacgaggacggcccagaagacgacccccagcucgucgggauaaccgcccgcaauaucccuaggggcccccagcuggccgcccagaaccucgggaucagccuggccaaccuccugcuguccaagggcgccaagaacauacuggacgucgcccggcagcugaacgaugcccau

SEQ ID NO: 29 - RNA, 1083 nt, Artificial Sequence
  PBGD-CO021
augagcggcaacgggaacgccgccgcaaccgccgaggagaacucaccaaagaugagggugauccgagugggcaccaggaagucgcagcuggccaggauccagaccgacagcgugguggcgacccucaaggccuccuaccccggccugcaguucgagauaaucgccauguccaccaccggcgacaagauccuggauaccgcccucagcaagaucggcgaaaagagccuguucaccaaggagcucgagcacgcucuggagaagaacgagguggaccuggucgugcacucccugaaagaccugcccaccgugcugcccccgggcuucaccauaggggccaucugcaagcgggagaacccccacgacgccgugguguuccauccgaaguucgugggcaagacccuggagacccugcccgagaagagcguggugggcacgagcagccuaagaagggccgcacagcuccagaggaaguucccccaccucgaguuccgcagcaucagaggcaaccugaacaccaggcugcggaagcucgacgagcagcaggaguuuagcgccaucauccucgccaccgccggccugcagaggaugggauggcauaaccggguggggcagauccugcaccccgaggaguguauguacgccguggggcagggggcccugggcguggaggugcgggccaaggaucaggacauccucgaccuggugggcgugcuucacgaucccgagacccuucugcggugcaucgccgagcgggccuuucugaggcaucuggagggcggguguagugugccaguggcaguucacaccgccaugaaggacggccagcuguaccugaccggugggguuuggagccuggacggguccgacagcauccaggagaccaugcaggccacgauccaugugcccgcucagcaugaggacggaccagaagacgacccgcagcuggugggcaucacggcccggaacauacccagggggccccagcuggcggcccagaaccugggcaucagccuggccaaccugcugcugagcaagggcgccaagaacauccuggauguggcgcggcagcugaaugaugcccac

SEQ ID NO: 30 - RNA, 1083 nt, Artificial Sequence
  PBGD-CO022
augucgggcaacggcaacgcggccgccaccgcggaggagaauagccccaagaugcgggugaucagggugggcaccaggaagagccagcuggccaggauccagaccgacagugugguggccacccugaaggccagcuacccagggcugcaguucgagaucauugccaugucuaccaccggcgacaagauccucgacaccgcccugagcaaaaucggggagaagagccuguuuaccaaagagcuggagcacgcccuggagaagaaugagguggaccuggucgugcacucccugaaggaccugcccaccgugcugccacccggcuucaccaucggcgccaucuguaagagggagaauccccacgacgcaguuguguuccaccccaaguucgugggcaagacccuggagacccugcccgagaagagcguggugggcacgucgagccugcgacgggccgcucagcugcagcggaaauucccccaccucgaguuccggucuauuaggggcaaccucaacacccgccucaggaaacuggacgagcagcaggaguucucggccaucauccucgccaccgccggacugcaaaggaugggguggcacaaccgcgugggacagauccugcaucccgaggagugcauguacgccgugggccagggcgcgcugggaguggaggucagggcuaaagaccaggacauacucgaccucgugggcgugcugcacgacccggagacccugcugcggugcauagccgagcgggccuuccuuaggcaccuggagggcggcugcuccgugcccguggccgugcacaccgccaugaaggacggccaacuguaccugaccggcgggguguggucccuggacggcucagacagcauacaggagaccaugcaagcgaccauccacgugcccgcccagcacgaggacggccccgaggaugacccccagcugguggggaucacagcccgcaacauccccaggggcccccagcuggccgcccagaacuugggcauuagccuggcaaaccuccugcuguccaagggagccaaaaauauccuggacguggccaggcagcugaacgacgcccau

SEQ ID NO: 31 - RNA, 1083 nt, Artificial Sequence
  PBGD-CO023
augagcggcaacggcaacgccgcggccaccgcggaggagaacagccccaagaugagggugaucagggugggcaccaggaagucccaacuggcuaggauccagaccgacagcgugguggccacccugaaagcauccuaccccggccuccaguucgagauaaucgccaugagcaccacaggcgacaagauccuggacaccgcccugagcaagaucggcgagaagucgcuguuuaccaaggagcuggagcacgcgcuggagaaaaacgagguggaccuggucgugcacagccugaaggaucugcccacagugcuccccccaggcuucaccaucggagccaucugcaagagggagaauccccacgacgcggugguguuucaucccaaguucguggggaagacccuggagacccugccggagaagagcgugguggggaccagcagccugaggcgggccgcccagcugcagaggaaauucccccaucuggaguucagaagcaucaggggcaaccugaacaccaggcugaggaagcucgacgagcagcaggaauucagcgccaucauccucgccacggccgggcugcagaggaugggcuggcauaacaggguggggcagauccuccaccccgaagagugcauguacgccgugggccagggcgcccucggcguggaggugagggccaaggaccaggacauccuggacuuggugggcguccugcaugaccccgagacccugcugcggugcaucgccgagcgggccuuccucaggcaccuggagggcggcugcagcgugcccguggccguacacaccgccaugaaagauggccagcuguaccugaccggcggcguguggagccuggacggcuccgacagcauccaggagaccaugcaggccaccauccaugugcccgcccagcacgaggacgggccagaggacgauccccagcuugugggaaucaccgccaggaacaucccuaggggcccacagcuggccgcccaaaaucucgggauaagccuggcuaaccugcugcugagcaagggcgcgaagaacauccuggacguggcgcgacagcugaacgacgcccau

SEQ ID NO: 32 - RNA, 1083 nt, Artificial Sequence
  PBGD-CO024
augagcggcaacggcaacgcggcggccacggccgaggagaacagccccaaaaugaggguuaucagggugggcacccgcaagucacagcuggccaggauccagacagauuccgugguggccaccuugaaggccuccuaccccggccugcaguucgagaucauagccaugucaacgaccggggacaagauccucgacaccgcccugagcaagaucggggagaagucacuguucacaaaggaacuggaacacgcccuugagaagaacgagguugaccuggugguccacucccugaaggaccugccaaccgugcugccgccgggcuucaccaucggggccaucugcaagcgggagaacccccacgacgccgucguguuccacccgaaauucguggggaaaacccucgagacccugcccgagaagagcguggugggcacguccagccugcggagggccgcccagcugcagcggaaguucccccaccuggaguucagguccauccgggggaaccugaauacgaggcugaggaagcuggacgaacagcaggaguucagcgccaucauccuggcgaccgccggccugcagcggaugggcuggcacaaucgggugggccagauccugcacccggaggagugcauguacgccguggggcagggcgcccucggcgucgaggugcgggccaaggaccaggauauccuggaccugguaggaguccugcacgaucccgaaacccugcuccgguguauagccgagcgugccuuccugaggcaucuggaaggcggaugcuccguccccguggccgugcacaccgcaaugaaagacggccagcuguaccugaccggcggcgucuggagccuggacggcucagacagcauccaagagaccaugcaggccaccauccacgucccugcccagcacgaggacggccccgaagacgacccgcagcuggugggcaucacagccaggaacaucccccggggcccgcagcuggccgcccagaaucugggaauuagccuggccaaccuccugcugagcaagggagccaagaacauccuggacguggcccggcagcugaacgacgcccac

SEQ ID NO: 33 - RNA, 1083 nt, Artificial Sequence
  PBGD-CO025
augagcggcaacggcaacgcggccgccaccgccgaagagaacagccccaagaugagggugaucagggugggcacgaggaagagccagcuggccaggauccagaccgacagcgugguggcgacccugaaggccucuuacccuggccugcaguuugagaucaucgccaugagcaccaccggggauaagauccucgacaccgcccuguccaagauuggagaaaaaucgcuguucaccaaggaacuggagcacgcccuggagaagaacgagguagaccugguggugcauagccucaaggaucugccaaccgugcugccccccggguuuaccaucggcgccauaugcaagagggagaacccccacgacgcggugguguuccaccccaaguucgugggcaaaacccucgagacgcugcccgagaagagcgucguuggcaccuccagccugaggcgggccgcccagcugcagaggaaguucccccaccucgaguucagaagcaucaggggcaaccugaacaccaggcugaggaagcuggacgagcagcaggaguucagcgccaucauccuggccaccgccggccugcagaggaugggauggcacaauagggugggccagauccugcaccccgaggagugcauguacgccgucggacagggcgcgcugggcguggaggucagggcgaaggaccaggacauccuggaccuggucgggguccugcacgacccggagacccugcugaggugcaucgccgagcgggccuuccuccggcaccuggagggcgguugcagcgugccaguggccgugcacaccgccaugaaggaugggcagcuguaucugaccggcggaguguggagccucgacgguagcgacuccauccaggaaaccaugcaggccacuauccacgugcccgcccagcacgaggauggccccgaggacgauccccagcuggucgggauuacggcccggaacauccccaggggcccgcagcucgccgcacagaaccucggcaucucccuggccaaccugcugcucuccaagggcgccaagaacauccucgacguggcccggcaacugaacgacgcccac

SEQ ID NO: 34 - RNA, 87 nt, Artificial Sequence
  miR-142
gacagugcagucacccauaaaguagaaagcacuacuaacagcacuggaggguguaguguuuccuacuuuauggaugaguguacugug

SEQ ID NO: 35 - RNA, 23 nt, Artificial Sequence
  miR 142-3p sequence
uguaguguuuccuacuuuaugga

SEQ ID NO: 36 - RNA, 23 nt, Artificial Sequence
  miR 142-3p binding site
uccauaaaguaggaaacacuaca

SEQ ID NO: 37 - RNA, 21 nt, Artificial Sequence
  miR 142-5p sequence
cauaaaguagaaagcacuacu

SEQ ID NO: 38 - RNA, 21 nt, Artificial Sequence
  miR-142-5p binding site
aguagugcuuucuacuuuaug

SEQ ID NO: 39 - RNA, 47 nt, Artificial Sequence
  5'UTR-001 (Upstream UTR)
gggaaauaagagagaaaagaagaguaagaagaaauauaagagccacc

SEQ ID NO: 40 - RNA, 47 nt, Artificial Sequence
  5'UTR-002 (Upstream UTR)
gggagaucagagagaaaagaagaguaagaagaaauauaagagccacc

SEQ ID NO: 41 - RNA, 145 nt, Artificial Sequence
  5'UTR-003 (Upstream UTR)
ggaauaaaagucucaacacaacauauacaaaacaaacgaaucucaagcaaucaagcauucuacuucuauugcagcaauuuaaaucauuucuuuuaaagcaaaagcaauuuucugaaaauuuucaccauuuacgaacgauagcaac

SEQ ID NO: 42 - RNA, 42 nt, Artificial Sequence
  5'UTR-004 (Upstream UTR)
gggagacaagcuuggcauuccgguacuguugguaaagccacc

SEQ ID NO: 43 - RNA, 47 nt, Artificial Sequence; identical to SEQ ID NO: 40
  5'UTR-005 (Upstream UTR)

SEQ ID NO: 44 - RNA, 145 nt, Artificial Sequence; identical to SEQ ID NO: 41
  5'UTR-006 (Upstream UTR)

SEQ ID NO: 45 - RNA, 42 nt, Artificial Sequence; identical to SEQ ID NO: 42
  5'UTR-007 (Upstream UTR)

SEQ ID NO: 46 - RNA, 47 nt, Artificial Sequence
  5'UTR-008 (Upstream UTR)
gggaauuaacagagaaaagaagaguaagaagaaauauaagagccacc

SEQ ID NO: 47 - RNA, 47 nt, Artificial Sequence
  5'UTR-009 (Upstream UTR)
gggaaauuagacagaaaagaagaguaagaagaaauauaagagccacc

SEQ ID NO: 48 - RNA, 47 nt, Artificial Sequence
  5'UTR-010 (Upstream UTR)
gggaaauaagagaguaaagaacaguaagaagaaauauaagagccacc

SEQ ID NO: 49 - RNA, 47 nt, Artificial Sequence
  5'UTR-011 (Upstream UTR)
gggaaaaaagagagaaaagaagacuaagaagaaauauaagagccacc

SEQ ID NO: 50 - RNA, 47 nt, Artificial Sequence
  5'UTR-012 (Upstream UTR)
gggaaauaagagagaaaagaagaguaagaagauauauaagagccacc

SEQ ID NO: 51 - RNA, 47 nt, Artificial Sequence
  5'UTR-013 (Upstream UTR)
gggaaauaagagacaaaacaagaguaagaagaaauauaagagccacc

SEQ ID NO: 52 - RNA, 47 nt, Artificial Sequence
  5'UTR-014 (Upstream UTR)
gggaaauuagagaguaaagaacaguaaguagaauuaaaagagccacc

SEQ ID NO: 53 - RNA, 47 nt, Artificial Sequence
  5'UTR-015 (Upstream UTR)
gggaaauaagagagaauagaagaguaagaagaaauauaagagccacc

SEQ ID NO: 54 - RNA, 47 nt, Artificial Sequence
  5'UTR-016 (Upstream UTR)
gggaaauaagagagaaaagaagaguaagaagaaaauuaagagccacc

SEQ ID NO: 55 - RNA, 47 nt, Artificial Sequence
  5'UTR-017 (Upstream UTR)
gggaaauaagagagaaaagaagaguaagaagaaauuuaagagccacc

SEQ ID NO: 56 - RNA, 92 nt, Artificial Sequence
  5'UTR-018 (Upstream UTR)
ucaagcuuuuggacccucguacagaagcuaauacgacucacuauagggaaauaagagagaaaagaagaguaagaagaaauauaagagccacc

SEQ ID NO: 57 - RNA, 142 nt, Artificial Sequence
  142-3p 3'UTR (UTR including miR142-3p binding site)
ugauaauaguccauaaaguaggaaacacuacagcuggagccucgguggccaugcuucuugccccuugggccuccccccagccccuccuccccuuccugcacccguacccccguggucuuugaauaaagucugagugggcggc

SEQ ID NO: 58 - RNA, 142 nt, Artificial Sequence
  142-3p 3'UTR (UTR including miR142-3p binding site)
ugauaauaggcuggagccucgguggcuccauaaaguaggaaacacuacacaugcuucuugccccuugggccuccccccagccccuccuccccuuccugcacccguacccccguggucuuugaauaaagucugagugggcggc

SEQ ID NO: 59 - RNA, 142 nt, Artificial Sequence
  142-3p 3'UTR (UTR including miR142-3p binding site)
ugauaauaggcuggagccucgguggccaugcuucuugccccuuccauaaaguaggaaacacuacaugggccuccccccagccccuccuccccuuccugcacccguacccccguggucuuugaauaaagucugagugggcggc

SEQ ID NO: 60 - RNA, 142 nt, Artificial Sequence
  142-3p 3'UTR (UTR including miR142-3p binding site)
ugauaauaggcuggagccucgguggccaugcuucuugccccuugggccuccccccaguccauaaaguaggaaacacuacaccccuccuccccuuccugcacccguacccccguggucuuugaauaaagucugagugggcggc

SEQ ID NO: 61 - RNA, 142 nt, Artificial Sequence
  142-3p 3'UTR (UTR including miR142-3p binding site)
ugauaauaggcuggagccucgguggccaugcuucuugccccuugggccuccccccagccccuccuccccuucuccauaaaguaggaaacacuacacugcacccguacccccguggucuuugaauaaagucugagugggcggc

SEQ ID NO: 62 - RNA, 142 nt, Artificial Sequence
  142-3p 3'UTR (UTR including miR142-3p binding site)
ugauaauaggcuggagccucgguggccaugcuucuugccccuugggccuccccccagccccuccuccccuuccugcacccguacccccuccauaaaguaggaaacacuacaguggucuuugaauaaagucugagugggcggc

SEQ ID NO: 63 - RNA, 142 nt, Artificial Sequence
  142-3p 3'UTR (UTR including miR142-3p binding site)
ugauaauaggcuggagccucgguggccaugcuucuugccccuugggccuccccccagccccuccuccccuuccugcacccguacccccguggucuuugaauaaaguuccauaaaguaggaaacacuacacugagugggcggc

SEQ ID NO: 64 - RNA, 371 nt, Artificial Sequence
  3'UTR-001 (Creatine Kinase UTR)
gcgccugcccaccugccaccgacugcuggaacccagccagugggagggccuggcccaccagaguccugcucccucacuccucgccccgcccccugucccagagucccaccugggggcucucuccacccuucucagaguuccaguuucaaccagaguuccaaccaaugggcuccauccucuggauucuggccaaugaaauaucucccuggcaggguccucuucuuuucccagagcuccaccccaaccaggagcucuaguuaauggagagcucccagcacacucggagcuugugcuuugucuccacgcaaagcgauaaauaaaagcauugguggccuuuggucuuugaauaaagccugaguaggaagucuaga

SEQ ID NO: 65 - RNA, 568 nt, Artificial Sequence
  3'UTR-002 (Myoglobin UTR)
gccccugccgcucccacccccacccaucugggccccggguucaagagagagcggggucugaucucguguagccauauagaguuugcuucugagugucugcuuuguuuaguagaggugggcaggaggagcugaggggcuggggcugggguguugaaguuggcuuugcaugcccagcgaugcgccucccugugggaugucaucacccugggaaccgggaguggcccuuggcucacuguguucugcaugguuuggaucugaauuaauuguccuuucuucuaaaucccaaccgaacuucuuccaaccuccaaacuggcuguaaccccaaauccaagccauuaacuacaccugacaguagcaauugucugauuaaucacuggccccuugaagacagcagaaugucccuuugcaaugaggaggagaucugggcugggcgggccagcuggggaagcauuugacuaucuggaacuugugugugccuccucagguauggcagugacucaccugguuuuaauaaaacaaccugcaacaucucauggucuuugaauaaagccugaguaggaagucuaga

SEQ ID NO: 66 - RNA, 289 nt, Artificial Sequence
  3'UTR-003 (alpha-actin UTR)
acacacuccaccuccagcacgcgacuucucaggacgacgaaucuucucaaugggggggcggcugagcuccagccaccccgcagucacuuucuuuguaacaacuuccguugcugccaucguaaacugacacaguguuuauaacguguacauacauuaacuuauuaccucauuuuguuauuuuucgaaacaaagcccuguggaagaaaauggaaaacuugaagaagcauuaaagucauucuguuaagcugcguaaauggucuuugaauaaagccugaguaggaagucuaga

SEQ ID NO: 67 - RNA, 379 nt, Artificial Sequence
  3'UTR-004 (Albumin UTR)
caucacauuuaaaagcaucucagccuaccaugagaauaagagaaagaaaaugaagaucaaaagcuuauucaucuguuuuucuuuuucguugguguaaagccaacacccugucuaaaaaacauaaauuucuuuaaucauuuugccucuuuucucugugcuucaauuaauaaaaaauggaaagaaucuaauagagugguacagcacuguuauuuuucaaagauguguugcuauccugaaaauucuguagguucuguggaaguuccaguguucucucuuauuccacuucgguagaggauuucuaguuucuugugggcuaauuaaauaaaucauuaauacucuucuaauggucuuugaauaaagccugaguaggaagucuaga

SEQ ID NO: 68 - RNA, 118 nt, Artificial Sequence
  3'UTR-005 (alpha-globin UTR)
gcugccuucugcggggcuugccuucuggccaugcccuucuucucucccuugcaccuguaccucuuggucuuugaauaaagccugaguaggaaggcggccgcucgagcaugcaucuaga

SEQ ID NO: 69 - RNA, 908 nt, Artificial Sequence
  3'UTR-006 (G-CSF UTR)
gccaagcccuccccaucccauguauuuaucucuauuuaauauuuaugucuauuuaagccucauauuuaaagacagggaagagcagaacggagccccaggccucuguguccuucccugcauuucugaguuucauucuccugccuguagcagugagaaaaagcuccuguccucccauccccuggacugggagguagauagguaaauaccaaguauuuauuacuaugacugcuccccagcccuggcucugcaaugggcacugggaugagccgcugugagccccugguccugaggguccccaccugggacccuugagaguaucaggucucccacgugggagacaagaaaucccuguuuaauauuuaaacagcaguguuccccaucuggguccuugcaccccucacucuggccucagccgacugcacagcggccccugcauccccuuggcugugaggccccuggacaagcagagguggccagagcugggaggcauggcccuggggucccacgaauuugcuggggaaucucguuuuucuucuuaagacuuuugggacaugguuugacucccgaacaucaccgacgcgucuccuguuuuucuggguggccucgggacaccugcccugcccccacgagggucaggacugugacucuuuuuagggccaggcaggugccuggacauuugccuugcuggacggggacuggggaugugggagggagcagacaggaggaaucaugucaggccugugugugaaaggaagcuccacugucacccuccaccucuucaccccccacucaccaguguccccuccacugucacauuguaacugaacuucaggauaauaaaguguuugccuccauggucuuugaauaaagccugaguaggaaggcggccgcucgagcaugcaucuaga

SEQ ID NO: 70 - RNA, 835 nt, Artificial Sequence
  3'UTR-007 (Col1a2; collagen, type I, alpha 2 UTR)
acucaaucuaaauuaaaaaagaaagaaauuugaaaaaacuuucucuuugccauuucuucuucuucuuuuuuaacugaaagcugaauccuuccauuucuucugcacaucuacuugcuuaaauugugggcaaaagagaaaaagaaggauugaucagagcauugugcaauacaguuucauuaacuccuucccccgcucccccaaaaauuugaauuuuuuuuucaacacucuuacaccuguuauggaaaaugucaaccuuuguaagaaaaccaaaauaaaaauugaaaaauaaaaaccauaaacauuugcaccacuuguggcuuuugaauaucuuccacagagggaaguuuaaaacccaaacuuccaaagguuuaaacuaccucaaaacacuuucccaugagugugauccacauuguuaggugcugaccuagacagagaugaacugagguccuuguuuuguuuuguucauaauacaaaggugcuaauuaauaguauuucagauacuugaagaauguugauggugcuagaagaauuugagaagaaauacuccuguauugaguuguaucgugugguguauuuuuuaaaaaauuugauuuagcauucauauuuuccaucuuauucccaauuaaaaguaugcagauuauuugcccaaaucuucuucagauucagcauuuguucuuugccagucucauuuucaucuucuuccaugguuccacagaagcuuuguuucuugggcaagcagaaaaauuaaauuguaccuauuuuguauaugugagauguuuaaauaaauugugaaaaaaaugaaauaaagcauguuugguuuuccaaaagaacauau

SEQ ID NO: 71 - RNA, 297 nt, Artificial Sequence
  3'UTR-008 (Col6a2; collagen, type VI, alpha 2 UTR)
cgccgccgcccgggccccgcagucgagggucgugagcccaccccguccauggugcuaagcgggcccgggucccacacggccagcaccgcugcucacucggacgacgcccugggccugcaccucuccagcuccucccacgggguccccguagccccggcccccgcccagccccaggucuccccaggcccuccgcaggcugcccggccucccucccccugcagccaucccaaggcuccugaccuaccuggccccugagcucuggagcaagcccugacccaauaaaggcuuugaacccau

SEQ ID NO: 72 - RNA, 602 nt, Artificial Sequence
  3'UTR-009 (RPN1; ribophorin I UTR)
ggggcuagagcccucuccgcacagcguggagacggggcaaggagggggguuauuaggauuggugguuuuguuuugcuuuguuuaaagccgugggaaaauggcacaacuuuaccucugugggagaugcaacacugagagccaaggggugggaguugggauaauuuuuauauaaaagaaguuuuuccacuuugaauugcuaaaaguggcauuuuuccuaugugcagucacuccucucauuucuaaaauagggacguggccaggcacgguggcucaugccuguaaucccagcacuuugggaggccgaggcaggcggcucacgaggucaggagaucgagacuauccuggcuaacacgguaaaacccugucucuacuaaaaguacaaaaaauuagcugggcgugguggugggcaccuguagucccagcuacucgggaggcugaggcaggagaaaggcaugaauccaagaggcagagcuugcagugagcugagaucacgccauugcacuccagccugggcaacaguguuaagacucugucucaaauauaaauaaauaaauaaauaaauaaauaaauaaauaaaaauaaagcgagauguugcccucaaa

SEQ ID NO: 73 - RNA, 785 nt, Artificial Sequence
  3'UTR-010 (LRP1; low density lipoprotein receptor-related protein 1 UTR)
ggcccugccccgucggacugcccccagaaagccuccugcccccugccagugaaguccuucagugagccccuccccagccagcccuucccuggccccgccggauguauaaauguaaaaaugaaggaauuacauuuuauaugugagcgagcaagccggcaagcgagcacaguauuauuucuccauccccucccugccugcuccuuggcacccccaugcugccuucagggagacaggcagggagggcuuggggcugcaccuccuacccucccaccagaacgcaccccacugggagagcugguggugcagccuuccccucccuguauaagacacuuugccaaggcucuccccucucgccccaucccugcuugcccgcucccacagcuuccugagggcuaauucugggaagggagaguucuuugcugccccugucuggaagacguggcucugggugagguaggcgggaaaggauggaguguuuuaguucuugggggaggccaccccaaaccccagccccaacuccaggggcaccuaugagauggccaugcucaaccccccucccagacaggcccucccugucuccagggcccccaccgagguucccagggcuggagacuuccucugguaaacauuccuccagccuccccuccccuggggacgccaaggaggugggccacacccaggaagggaaagcgggcagccccguuuuggggacgugaacguuuuaauaauuuuugcugaauuccuuuacaacuaaauaacacagauauuguuauaaauaaaauugu

SEQ ID NO: 74 - RNA, 3001 nt, Artificial Sequence
  3'UTR-011 (Nnt1; cardiotrophin-like cytokine factor 1 UTR)
auauuaaggaucaagcuguuagcuaauaaugccaccucugcaguuuugggaacaggcaaauaaaguaucaguauacauggugauguacaucuguagcaaagcucuuggagaaaaugaagacugaagaaagcaaagcaaaaacuguauagagagauuuuucaaaagcaguaaucccucaauuuuaaaaaaggauugaaaauucuaaaugucuuucugugcauauuuuuuguguuaggaaucaaaaguauuuuauaaaaggagaaagaacagccucauuuuagauguaguccuguuggauuuuuuaugccuccucaguaaccagaaauguuuuaaaaaacuaaguguuuaggauuucaagacaacauuauacauggcucugaaauaucugacacaauguaaacauugcaggcaccugcauuuuauguuuuuuuuuucaacaaaugugacuaauuugaaacuuuuaugaacuucugagcuguccccuugcaauucaaccgcaguuugaauuaaucauaucaaaucaguuuuaauuuuuuaaauuguacuucagagucuauauuucaagggcacauuuucucacuacuauuuuaauacauuaaaggacuaaauaaucuuucagagaugcuggaaacaaaucauuugcuuuauauguuucauuagaauaccaaugaaacauacaacuugaaaauuaguaauaguauuuuugaagaucccauuucuaauuggagaucucuuuaauuucgaucaacuuauaauguguaguacuauauuaagugcacuugaguggaauucaacauuugacuaauaaaaugaguucaucauguuggcaagugauguggcaauuaucucuggugacaaaagaguaaaaucaaauauuucugccuguuacaaauaucaaggaagaccugcuacuaugaaauagaugacauuaaucugucuucacuguuuauaauacggauggauuuuuuuucaaaucaguguguguuuugaggucuuauguaauugaugacauuugagagaaaugguggcuuuuuuuagcuaccucuuuguucauuuaagcaccaguaaagaucaugucuuuuuauagaaguguagauuuucuuugugacuuugcuaucgugccuaaagcucuaaauauaggugaaugugugaugaauacucagauuauuugucucucuauauaauuaguuugguacuaaguuucucaaaaaauuauuaacacaugaaagacaaucucuaaaccagaaaaagaaguaguacaaauuuuguuacuguaaugcucgcguuuagugaguuuaaaacacacaguaucuuuugguuuuauaaucaguuucuauuuugcugugccugagauuaagaucuguguaugugugugugugugugugugcguuuguguguuaaagcagaaaagacuuuuuuaaaaguuuuaagugauaaaugcaauuuguuaauugaucuuagaucacuaguaaacucagggcugaauuauaccauguauauucuauuagaagaaaguaaacaccaucuuuauuccugcccuuuuucuucucucaaaguaguuguaguuauaucuagaaagaagcaauuuugauuucuugaaaagguaguuccugcacucaguuuaaacuaaaaauaaucauacuuggauuuuauuuauuuuugucauaguaaaaauuuuaauuuauauauauuuuuauuuaguauuaucuuauucuuugcuauuugccaauccuuugucaucaauuguguuaaaugaauugaaaauucaugcccuguucauuuuauuuuacuuuauugguuaggauauuuaaaggauuuuuguauauauaauuucuuaaauuaauauuccaaaagguuaguggacuuagauuauaaauuauggcaaaaaucuaaaaacaacaaaaaugauuuuuauacauucuauuucauuauuccucuuuuuccaauaagucauacaauugguagauaugacuuauuuuauuuuuguauuauucacuauaucuuuaugauauuuaaguauaaauaauuaaaaaaauuuauuguaccuuauagucugucaccaaaaaaaaaaaauuaucuguagguagugaaaugcuaauguugauuugucuuuaagggcuuguuaacuauccuuuauuuucucauuugucuuaaauuaggaguuuguguuuaaauuacucaucuaagcaaaaaauguauauaaaucccauuacuggguauauacccaaaggauuauaaaucaugcugcuauaaagacacaugcacacguauguuuauugcagcacuauucacaauagcaaagacuuggaaccaacccaaauguccaucaaugauagacuugauuaagaaaaugugcacauauacaccauggaauacuaugcagccauaaaaaaggaugaguucauguccuuuguagggacauggauaaagcuggaaaccaucauucugagcaaacuauugcaaggacagaaaaccaaacacugcauguucucacucauaggugggaauugaacaaugagaacacuuggacacaagguggggaacaccacacaccagggccugucaugggguggggggaguggggagggauagcauuaggagauauaccuaauguaaaugaugaguuaaugggugcagcacaccaacauggcacauguauacauauguagcaaaccugcacguugugcacauguacccuagaacuuaaaguauaauuaaaaaaaaaaagaaaacagaagcuauuuauaaagaaguuauuugcugaaauaaaugugaucuuucccauuaaaaaaauaaagaaauuuugggguaaaaaaacacaauauauuguauucuugaaaaauucuaagagaguggaugugaaguguucucaccacaaaagugauaacuaauugagguaaugcacauauuaauuagaaagauuuugucauuccacaauguauauauacuuaaaaauauguuauacacaauaaauacauacauuaaaaaauaaguaaaugua

SEQ ID NO: 75 - RNA, 1037 nt, Artificial Sequence
  3'UTR-012 (Col6a1; collagen, type VI, alpha 1 UTR)
cccacccugcacgccggcaccaaacccuguccucccaccccuccccacucaucacuaaacagaguaaaaugugaugcgaauuuucccgaccaaccugauucgcuagauuuuuuuuaaggaaaagcuuggaaagccaggacacaacgcugcugccugcuuugugcaggguccuccggggcucagcccugaguuggcaucaccugcgcagggcccucuggggcucagcccugagcuagugucaccugcacagggcccucugaggcucagcccugagcuggcgucaccugugcagggcccucuggggcucagcccugagcuggccucaccuggguuccccaccccgggcucuccugcccugcccuccugcccgcccucccuccugccugcgcagcuccuucccuaggcaccucugugcugcaucccaccagccugagcaagacgcccucucggggccugugccgcacuagccucccucuccucuguccccauagcugguuuuucccaccaauccucaccuaacaguuacuuuacaauuaaacucaaagcaagcucuucuccucagcuuggggcagccauuggccucugucucguuuugggaaaccaaggucaggaggccguugcagacauaaaucucggcgacucggccccgucuccugaggguccugcuggugaccggccuggaccuuggcccuacagcccuggaggccgcugcugaccagcacugaccccgaccucagagaguacucgcaggggcgcuggcugcacucaagacccucgagauuaacggugcuaaccccgucugcuccucccucccgcagagacuggggccuggacuggacaugagagccccuuggugccacagagggcugugucuuacuagaaacaacgcaaaccucuccuuccucagaauagugauguguucgacguuuuaucaaaggcccccuuucuauguucauguuaguuuugcuccuucuguguuuuuuucugaaccauauccauguugcugacuuuuccaaauaaagguuuucacuccucuc

SEQ ID NO: 76 - RNA, 577 nt, Artificial Sequence
  3'UTR-013 (Calr; calreticulin UTR)
agaggccugccuccagggcuggacugaggccugagcgcuccugccgcagagcuggccgcgccaaauaaugucucugugagacucgagaacuuucauuuuuuuccaggcugguucggauuugggguggauuuugguuuuguuccccuccuccacucucccccacccccuccccgcccuuuuuuuuuuuuuuuuuuaaacugguauuuuaucuuugauucuccuucagcccucaccccugguucucaucuuucuugaucaacaucuuuucuugccucuguccccuucucucaucucuuagcuccccuccaaccuggggggcagugguguggagaagccacaggccugagauuucaucugcucuccuuccuggagcccagaggagggcagcagaaggggguggugucuccaaccccccagcacugaggaagaacggggcucuucucauuucaccccucccuuucuccccugcccccaggacugggccacuucuggguggggcagugggucccagauuggcucacacugagaauguaagaacuacaaacaaaauuucuauuaaauuaaauuuugugucucc

SEQ ID NO: 77 - RNA, 2212 nt, Artificial Sequence
  3'UTR-014 (Col1a1; collagen, type I, alpha 1 UTR)
cucccuccaucccaaccuggcucccucccacccaaccaacuuuccccccaacccggaaacagacaagcaacccaaacugaacccccucaaaagccaaaaaaugggagacaauuucacauggacuuuggaaaauauuuuuuuccuuugcauucaucucucaaacuuaguuuuuaucuuugaccaaccgaacaugaccaaaaaccaaaagugcauucaaccuuaccaaaaaaaaaaaaaaaaaaagaauaaauaaauaacuuuuuaaaaaaggaagcuugguccacuugcuugaagacccaugcggggguaagucccuuucugcccguugggcuuaugaaaccccaaugcugcccuuucugcuccuuucuccacaccccccuuggggccuccccuccacuccuucccaaaucugucuccccagaagacacaggaaacaauguauugucugcccagcaaucaaaggcaaugcucaaacacccaaguggcccccacccucagcccgcuccugcccgcccagcacccccaggcccugggggaccugggguucucagacugccaaagaagccuugccaucuggcgcucccauggcucuugcaacaucuccccuucguuuuugagggggucaugccgggggagccaccagccccucacuggguucggaggagagucaggaagggccacgacaaagcagaaacaucggauuuggggaacgcgugucaaucccuugugccgcagggcugggcgggagagacuguucuguuccuuguguaacuguguugcugaaagacuaccucguucuugucuugaugugucaccggggcaacugccugggggcggggaugggggcaggguggaagcggcuccccauuuuauaccaaaggugcuacaucuaugugaugggugggguggggagggaaucacuggugcuauagaaauugagaugcccccccaggccagcaaauguuccuuuuuguucaaagucuauuuuuauuccuugauauuuuucuuuuuuuuuuuuuuuuuuuguggauggggacuugugaauuuuucuaaaggugcuauuuaacaugggaggagagcgugugcggcuccagcccagcccgcugcucacuuuccacccucucuccaccugccucuggcuucucaggccucugcucuccgaccucucuccucugaaacccuccuccacagcugcagcccauccucccggcucccuccuagucuguccugcguccucuguccccggguuucagagacaacuucccaaagcacaaagcaguuuuucccccuaggggugggaggaagcaaaagacucuguaccuauuuuguauguguauaauaauuugagauguuuuuaauuauuuugauugcuggaauaaagcauguggaaaugacccaaacauaauccgcaguggccuccuaauuuccuucuuuggaguugggggagggguagacauggggaaggggcuuuggggugaugggcuugccuuccauuccugcccuuucccuccccacuauucucuucuagaucccuccauaaccccacuccccuuucucucacccuucuuauaccgcaaaccuuucuacuuccucuuucauuuucuauucuugcaauuuccuugcaccuuuuccaaauccucuucuccccugcaauaccauacaggcaauccacgugcacaacacacacacacacucuucacaucugggguuguccaaaccucauacccacuccccuucaagcccauccacucuccacccccuggaugcccugcacuugguggcggugggaugcucauggauacugggagggugaggggaguggaacccgugaggaggaccugggggccucuccuugaacugacaugaagggucaucuggccucugcucccuucucacccacgcugaccuccugccgaaggagcaacgcaacaggagaggggucugcugagccuggcgagggucugggagggaccaggaggaaggcgugcucccugcucgcuguccuggcccugggggagugagggagacagacaccugggagagcuguggggaaggcacucgcaccgugcucuugggaaggaaggagaccuggcccugcucaccacggacugggugccucgaccuccugaauccccagaacacaaccccccugggcugggguggucuggggaaccaucgugcccccgccucccgccuacuccuuuuuaagcuu

SEQ ID NO: 78 - RNA, 729 nt, Artificial Sequence
  3'UTR-015 (Plod1; procollagen-lysine, 2-oxoglutarate 5-dioxygenase 1 UTR)
uuggccaggccugacccucuuggaccuuucuucuuugccgacaaccacugcccagcagccucugggaccucggggucccagggaacccaguccagccuccuggcuguugacuucccauugcucuuggagccaccaaucaaagagauucaaagagauuccugcaggccagaggcggaacacaccuuuauggcuggggcucuccgugguguucuggacccagccccuggagacaccauucacuuuuacugcuuuguagugacucgugcucuccaaccugucuuccugaaaaaccaaggcccccuucccccaccucuuccauggggugagacuugagcagaacaggggcuuccccaaguugcccagaaagacugucugggugagaagccauggccagagcuucucccaggcacagguguugcaccagggacuucugcuucaaguuuugggguaaagacaccuggaucagacuccaagggcugcccugagucugggacuucugccuccauggcuggucaugagagcaaaccguaguccccuggagacagcgacuccagagaaccucuugggagacagaagaggcaucugugcacagcucgaucuucuacuugccuguggggaggggagugacagguccacacaccacacugggucacccuguccuggaugccucugaagagagggacagaccgucagaaacuggagaguuucuauuaaaggucauuuaaacca

SEQ ID NO: 79 - RNA, 847 nt, Artificial Sequence
  3'UTR-016 (Nucb1; nucleobindin 1 UTR)
uccuccgggaccccagcccucaggauuccugaugcuccaaggcgacugaugggcgcuggaugaaguggcacagucagcuucccugggggcuggugucauguugggcuccuggggcgggggcacggccuggcauuucacgcauugcugccaccccagguccaccugucuccacuuucacagccuccaagucuguggcucuucccuucuguccuccgaggggcuugccuucucucguguccagugaggugcucagugaucggcuuaacuuagagaagcccgcccccuccccuucuccgucugucccaagagggucugcucugagccugcguuccuagguggcucggccucagcugccuggguuguggccgcccuagcauccuguaugcccacagcuacuggaauccccgcugcugcuccgggccaagcuucugguugauuaaugagggcaugggguggucccucaagaccuuccccuaccuuuuguggaaccagugaugccucaaagacaguguccccuccacagcugggugccaggggcaggggauccucaguauagccggugaacccugauaccaggagccugggccucccugaaccccuggcuuccagccaucucaucgccagccuccuccuggaccucuuggcccccagccccuuccccacacagccccagaagggucccagagcugaccccacuccaggaccuaggcccagccccucagccucaucuggagccccugaagaccagucccacccaccuuucuggccucaucugacacugcuccgcauccugcuguguguccuguuccauguuccgguuccauccaaauacacuuucuggaacaaa

SEQ ID NO: 80 - RNA, 110 nt, Artificial Sequence
  3'UTR-017 (alpha-globin)
gcuggagccucgguggccaugcuucuugccccuugggccuccccccagccccuccuccccuuccugcacccguacccccguggucuuugaauaaagucugagugggcggc

SEQ ID NO: 81 - RNA, 119 nt, Artificial Sequence
  3'UTR-018
ugauaauaggcuggagccucgguggccaugcuucuugccccuugggccuccccccagccccuccuccccuuccugcacccguacccccguggucuuugaauaaagucugagugggcggc

SEQ ID NO: 82 - DNA, 18 bp, Artificial Sequence
  Syn5 promoter
attgggcacccgtaaggg

SEQ ID NO: 83 - DNA, 92 bp, Artificial Sequence
  5'UTR of mRNA encoding human PBGD
tcaagcttttggaccctcgtacagaagctaatacgactcactatagggaaataagagagaaaagaagagtaagaagaaatataagagccacc

SEQ ID NO: 84 - DNA, 119 bp, Artificial Sequence
  3'UTR of mRNA encoding human PBGD
tgataataggctggagcctcggtggccatgcttcttgccccttgggcctccccccagcccctcctccccttcctgcacccgtacccccgtggtctttgaataaagtctgagtgggcggc

SEQ ID NO: 85 - protein, 19 aa, Artificial Sequence
  human specific peptide
ASYPGLQFEIIAMSTTGDK

SEQ ID NO: 86 - RNA, 1650 nt, Artificial Sequence
  PBGD-CO27
auggaagaugcgaagaacaucaagaagggaccugccccguuuuacccuuuggaggacgguacagcaggagaacagcuccacaaggcgaugaaacgcuacgcccugguccccggaacgauugcguuuaccgaugcacauauugagguagacaucacauacgcagaauacuucgaaaugucggugaggcuggcggaagcgaugaagagauauggucuuaacacuaaucaccgcaucgugguguguucggagaacucauugcaguuuuucaugccgguccuuggagcacuuuucaucggggucgcagucgcgccagcgaacgacaucuacaaugagcgggaacucuugaauagcaugggaaucucccagccgacggucguguuugucuccaaaaaggggcugcagaaaauccucaacgugcagaagaagcuccccauuauucaaaagaucaucauuauggauagcaagacagauuaccaaggguuccagucgauguauaccuuugugacaucgcauuugccgccaggguuuaacgaguaugacuucguccccgagucauuugacagagauaaaaccaucgcgcugauuaugaauuccucggguagcaccgguuugccaaaggggguggcguugccccaccgcacugcuugugugcgguucucgcacgcuagggauccuaucuuugguaaucagaucauucccgacacagcaauccuguccgugguaccuuuucaucacgguuuuggcauguucacgacucucggcuauuugauuugcgguuucagggucguacuuauguaucgguucgaggaagaacuguuuuugagauccuugcaagauuacaagauccagucggcccuccuugugccaacgcuuuucucauucuuugcgaaaucgacacuuauugauaaguaugaccuuuccaaucugcaugagauugccucagggggagcgccgcuuagcaaggaagucggggaggcaguggccaagcgcuuccaccuucccggaauucggcagggauacgggcucacggagacaacauccgcgauccuuaucacgcccgagggugacgauaagccgggagccgucggaaaagugguccccuucuuugaagccaaggucguagaccucgacacgggaaaaacccucggagugaaccagaggggcgagcucugcgugagagggccgaugaucaugucagguuacgugaauaacccugaagcgacgaaugcgcugaucgacaaggaugggugguugcauucgggagacauugccuauugggaugaggaugagcacuucuuuaucguagaucgacuuaagagcuugaucaaauacaaaggcuaucagguagcgccugccgagcucgagucaauccugcuccagcaccccaacauuuucgacgccggaguggccggguugcccgaugacgacgcgggugagcugccagcggccgugguaguccucgaacaugggaaaacaaugaccgaaaaggagaucguggacuacguagcaucacaagugacgacugcgaagaaacugaggggagggguagucuuuguggacgaggucccgaaaggcuugacugggaagcuugacgcucgcaaaauccgggaaauccugauuaaggcaaagaaaggcgggaaaaucgcuguc

SEQ ID NO: 87 - RNA, 1083 nt, Artificial Sequence
  PBGD-CO26
augucugguaacggcaaugcggcugcaacggcggaagaaaacagcccaaagaugagagugauucgcguggguacccgcaagagccagcuugcucgcauacagacggacagugugguggcaacauugaaagccucguacccuggccugcaguuugaaaucauugcuauguccaccacaggggacaagauucuugauacugcacucucuaagauuggagagaaaagccuguuuaccaaggagcuugaacaugcccuggagaagaaugaaguggaccugguuguucacuccuugaaggaccugcccacugugcuuccuccuggcuucaccaucggagccaucugcaagcgggaaaacccucaugaugcuguugucuuucacccaaaauuuguugggaagacccuagaaacccugccagagaagaguguggugggaaccagcucccugcgaagagcagcccagcugcagagaaaguucccgcaucuggaguucaggaguauucggggaaaccucaacacccggcuucggaagcuggacgagcagcaggaguucagugccaucauccuggcaacagcuggccugcagcgcaugggcuggcacaaccggguggggcagauccugcacccugaggaaugcauguaugcugugggccagggggccuugggcguggaagugcgagccaaggaccaggacaucuuggaucuggugggugugcugcacgaucccgagacucugcuucgcugcaucgcugaaagggccuuccugaggcaccuggaaggaggcugcagugugccaguagccgugcauacagcuaugaaggaugggcaacuguaccugacuggaggagucuggagccuagacggcucagauagcauacaagagaccaugcaggcuaccauccaugucccugcccagcaugaagauggcccugaggaugacccacaguugguaggcaucacugcucguaacauuccacgagggccccaguuggcugcccagaacuugggcaucagccuggccaacuuguugcugagcaaaggagccaaaaacauccuggauguugcacggcagcuuaacgaugcccau

SEQ ID NO: 88 - RNA, 1083 nt, Artificial Sequence
  PBGD-CO28
augaguggcaacggaaacgccgccgcuacagcagaggagaacuccccgaagaugcgcgugauuaggguaggcaccagaaagucucagcuggccagaauccaaaccgauagcguuguggccacauugaaggcuagcuaucccggccugcaguucgagaucaucgccaugagcaccaccggcgacaagauacucgacaccgcucugaguaaaaucggcgagaagagccuguuuaccaaggagcuggagcacgcccuggaaaagaacgaaguggaccugguggugcauagucugaaagaccuucccaccguccuuccaccaggcuucacuaucggcgccaucugcaagagggagaauccucacgaugccgucguguuucaucccaaguucgugggcaagaccuuagaaacccugccagagaaaagcgucguugggaccuccucccugcgacgggccgcccagcugcagagaaaguucccccacuuggaauucagauccaucagagggaaucugaauacucgccugagaaagcuggacgagcagcaggaguuuagcgcuaucauccuggccacggcugguuugcagagaaugggcuggcacaaccgggugggacagauccugcaccccgaggagugcauguaugcaguaggccagggggcccuggggguggaggucagagccaaagaucaggacauccuggaccuggucggcgugcugcacgaucccgaaacacugcugcgguguaucgccgagagggcuuuccuccggcacuuagagggcggcugcuccguccccguggccguucacacugccaugaaagacgggcagcuguaccugacgggcggcguguggucccuggacggcucagacuccauucaggagaccaugcaagcuaccauccacgucccugcccaacacgaagauggccccgaggacgacccccagcuggugggcaucaccgccaggaauaucccaagaggcccccaguuggccgcccagaaccugggcaucagucuggccaaccugcugcugaguaagggcgccaaaaacauccuggacguggcucggcagcugaaugacgcccac

SEQ ID NO: 89 - RNA, 1083 nt, Artificial Sequence
  PBGD-CO30
augagcggcaacggcaacgccgcagccaccgccgaggaaaacagccccaagaugcgggugaucagagugggcacccggaagagccagcuggcccggauccagaccgacagcgugguggccacccugaaggccuccuaccccggccugcaguucgagaucauugccaugagcaccaccggcgacaagauccuggacaccgcccugagcaagaucggcgagaagagccuguucacaaaagagcuggaacacgcccuggaaaagaacgagguggaccugguggugcacagccugaaggaccugcccaccgugcugcccccuggcuucaccaucggcgccaucugcaagagagagaacccccacgacgccgugguguuccacccuaaguucgugggcaagacacuggaaacccugcccgagaaguccguggugggcaccagcagccugcggagagccgcccagcugcagcggaaguucccccaccuggaauuucggagcauccggggcaaccugaacacccggcugcggaagcuggacgagcagcaggaauuuuccgcuaucauccuggccacagccggacugcagcggaugggcuggcacaacagagugggccagauccugcaccccgaggaaugcauguacgccgugggccagggagcccugggcguggaagugcgggccaaggaccaggacauccuggaucuggugggcgugcugcaugaccccgagacacugcugcgguguaucgccgagcgggccuuccugcggcaccuggaaggcggcugcagcgugcccguggccgugcacaccgccaugaaggacggacagcuguaccugacaggcggcguguggagccuggacggcagcgacagcauccaggagaccaugcaggccaccauccacgugcccgcccagcacgaggacggccccgaggacgacccucagcuggucggcaucaccgcccggaacauccccagaggcccccagcuggccgcccagaaccugggcaucagccuggccaaccugcugcuguccaagggcgccaagaacauccuggacguggcccggcagcugaacgacgcccac

SEQ ID NO: 90 - RNA, 1083 nt, Artificial Sequence
  PBGD-CO31
augagcggcaacggcaacgccgccgcuaccgccgaagagaacagcccaaagaugcgcgugaucagggucggcacgcgcaagucccagcucgcccggauccaaaccgauagcgugguggccacgcucaaggcgagcuauccgggcuuacaguucgagaucaucgccaugagcaccaccggcgauaagauacuggacaccgcccuguccaagaucggcgaaaagagccuguucaccaaggaacuggagcacgcgcuggagaagaacgagguggaccugguggugcacagccugaaggaccugccgaccgugcugccgccgggauucaccaucggcgccaucugcaagagggagaauccgcacgaugccgugguguuccacccaaaguucgugggcaagaccuuggaaacccugccagagaagucuguggucggcaccuccagccugcggcgagccgcccagcugcagcgaaaguucccgcaccuggaguucagguccauccgcggaaaucugaacaccaggcugcgcaagcucgacgagcagcaggaguucuccgccaucauccuggccaccgcaggccuccaaagaaugggcuggcauaaccgagucggccagauccuccacccggaggagugcauguacgcagugggccaaggcgcccugggcgucgaggugcgugccaaggaccaggacauccuggaccuggugggcgugcuccacgauccagagacacugcugagaugcaucgcggagcgcgccuuccugcgccaucuggagggaggcugcuccgucccgguggccguacauaccgccaugaaggacggucagcuguaccucaccggcggcguauggucccucgacgguagcgacagcauacaggagacgaugcaggccaccauccacgugccggcgcagcacgaggauggaccagaggacgacccgcagcugguggguaucaccgccaggaauaucccgcggggaccucagcuggccgcccagaaccugggcaucucccucgccaaccuccugcugagcaagggcgccaagaacauccuggacguggccaggcagcucaacgaugcccau

SEQ ID NO: 91 - RNA, 1083 nt, Artificial Sequence
  PBGD-CO32
augagcggcaacggcaacgccgccgccaccgccgaggaaaacagcccgaagaugcgggugaucagggugggcaccaggaagucccagcucgcccggauccagaccgacagcguggucgccaccuugaaggccuccuacccgggccuccaguucgagaucaucgccauguccacaaccggcgacaagauccuggauaccgcccucagcaagaucggcgagaagucccuguucaccaaggagcuggagcacgcccuggagaagaaugagguggaccugguggugcacagccugaaggaccugccuaccgugcugccaccaggcuucacaaucggcgccaucugcaagagagagaacccgcacgacgccgugguguuccauccgaaguucgugggcaagacccuggaaacccugccggagaaguccguagugggaaccucaagccugaggcgcgccgcccagcuccagaggaaguucccucaccuggaauuccgguccaucaggggcaaccugaacacgcgccugcggaagcucgacgagcagcaggaguucuccgccaucauccuggccacagccggccuucagcgcaugggcuggcacaacagggugggccagauccugcacccggaagaaugcauguacgccgugggccaaggcgcccucggcguggaagugcgugccaaggaccaggacauccuggaccuggugggcgugcugcacgacccugagacgcugcucaggugcaucgccgaacgcgcguuccugcggcaccuggagggaggcugcagcgucccgguggccguccacaccgccaugaaggacggccagcucuaccugacuggcggcguguggagccuggacggcagcgacagcauucaggaaaccaugcaggccaccauccacgugccugcccagcacgaggacggcccggaggacgacccucaacuggugggcauuacugcgcgaaacaucccgcgcggaccucagcuggccgcccagaaccugggcaucagccuggccaaccugcuccuguccaagggcgccaagaacauccucgacguggccaggcagcugaacgacgcgcac

SEQ ID NO: 92 - RNA, 1083 nt, Artificial Sequence
  PBGD-CO33
augagcggcaacggaaacgccgccgcgaccgcggaggagaacucgccuaagaugagagugauaaggguaggcacccggaagucucaacucgccaggauccagaccgacagcgugguggccacccucaaggccagcuauccaggacuccaguucgaaaucaucgccauguccaccacaggcgauaagauccuggacaccgcccuguccaagaucggcgagaagucccucuucaccaaggaacuggagcacgcccuggagaagaacgaggucgaucuggucgugcacagccugaaggaucugccuaccgugcucccgccgggcuucaccaucggcgccaucugcaagagggagaauccucacgacgccgugguguuccacccgaaguucgugggcaagacccuggagacacugccagaaaagucgguggugggcaccagcagccugcggcgggcggcccagcugcagcggaaguucccacaccuggaguucagguccauccguggcaaucugaacacccggcugcguaagcuggacgagcagcaggaauucagcgcgaucauccuggcaaccgccggucugcaaaggaugggcuggcacaacagggugggccagauccugcacccugaggagugcauguacgccgugggccagggagcccugggcguggaagugcgggccaaggaccaggacauccuggaccuggugggugugcuccacgacccugaaacccugcugcggugcaucgccgaaagggccuuccugaggcaccucgagggcggcugcagcgugccggucgccgugcacaccgccaugaaggacggccagcuguaccugaccggaggaguguggagccuggacggcuccgacuccauccaggagacuaugcaggccaccauucaugugccggcccagcaugaggacgguccggaggacgauccacagcuggucggcaucaccgcgcggaacaucccaagaggcccgcaacuggccgcucagaaccugggcauaucccuggccaaccugcuccugagcaagggcgccaagaacauccuggacguggccaggcagcugaaugacgcccac

SEQ ID NO: 93 - RNA, 1083 nt, Artificial Sequence
  PBGD-CO34
auguccggcaacggcaacgccgccgcuaccgccgaggagaacuccccuaagaugcgggucaucagggugggcacccgaaagucccaacuugcccggauccagaccgacuccgucguggccacccucaaggcuagcuauccaggccuccaguucgaaaucaucgccaugagcaccaccggcgacaagauucuggacaccgcccuguccaagaucggcgagaagagucuguucacgaaggagcucgagcacgcccuggaaaagaacgagguggaccugguggugcauucccugaaggaccugccaaccgugcugccgccgggcuucacuauaggagccaucugcaagcgggagaacccgcacgacgcggugguguuccauccgaaguucgugggcaagacucuggaaacccugccggagaaguccguggugggaacuagcucccugcggcgggccgcccagcugcagaggaaguucccgcaccuggaguucaggagcauacgcggcaaccugaacacccgccugcguaagcucgacgagcagcaggaauucagugccaucauccuggccacggcgggccugcagcggaugggcuggcacaacagggugggccagauccuccacccggaggaauguauguacgccgugggccagggcgcacugggcguggagguccgcgccaaggaccaagacauccuggaccuggucggcgugcugcacgacccugaaacccugcugaggugcauugccgagagagccuuccugaggcaucuggagggcggcugcagcgugccuguggccgugcacacagccaugaaggacggucagcuguaccugaccggcggcguguggagccuggacggcagcgacuccauccaggagacaaugcaggccaccauccacgucccggcccaacacgaggacggaccugaggacgauccucagcuggugggcaucaccgccaggaacaucccucggggcccgcagcuggccgcccagaaccugggcaucucccucgccaaccugcugcuguccaagggcgccaagaacauccucgacguggccagacagcugaacgacgcccac

SEQ ID NO: 94 - RNA, 1083 nt, Artificial Sequence
  PBGD-CO35
augagcggcaacggcaacgccgccgccaccgccgaggagaacagcccgaagaugagggugauaagggugggcacacggaagucccagcucgcccgcauccaaaccgacuccgugguggccacccucaaggccagcuacccgggccuccaauucgagaucaucgccaugagcaccaccggcgacaagauccuggacaccgcccugucuaagauaggcgaaaagagccuguucaccaaggagcuggagcaugcccuggagaagaacgagguggaccuggugguccacagucucaaggaccugccaaccgugcugccgccaggcuucaccaucggcgccaucugcaagcgugagaacccgcacgaugcugugguguuccacccuaaguucgugggaaagacccuggagacgcugccggaaaagagcguggucggcaccuccagccugcggagggccgcccaacuccagaggaaguucccgcaccuggaguucaggagcauccgcggcaaccugaacaccaggcugcgaaagcuggacgagcagcaggaauucucggccaucauccucgccaccgccggcuugcaaagaaugggcuggcauaaucgcgugggccagauccugcacccugaggagugcauguacgccgugggccagggugcucugggaguggaggugcgggccaaggaccaggauauccuggaccuggucggcgugcuucaugacccggagacgcuccugaggugcaucgccgagcgggccuuccugagacaccuggagggcggcugcuccgugccaguggccgugcacaccgccaugaaggacggacagcuguaccugaccggcggcguguggagccuggacggaagcgacagcauccaagaaaccaugcaggcgaccauucacgucccugcccagcacgaggauggaccagaggacgacccgcagcuggugggcaucaccgcccgcaacaucccuagaggcccacagcuggccgcccagaaucugggcaucagccuggccaaccugcugcugucuaagggagccaagaacauccuggacguggccaggcagcugaacgacgcccau

SEQ ID NO: 95 - RNA, 1083 nt, Artificial Sequence
  PBGD-CO36
auguccggcaacggcaacgccgcagccaccgccgaggagaauuccccgaagaugcgggugauccgggugggcaccagaaagagccagcucgcccgcauccaaaccgacuccgugguggccacccucaaggccuccuacccaggcuugcaguucgaaaucaucgccaugagcaccaccggcgacaagauccuggacaccgcccugagcaagauuggcgagaagucccuguucaccaaggagcuggagcaugcucuggagaagaacgagguggaccucguggugcacucccugaaggaccugccgacugugcugccgccuggcuucacgaucggcgccauaugcaagcgggaaaacccacacgacgccguggucuuccacccaaaguucgugggcaagacccuggaaacccugccggaaaagagcguggucggcacaagcucccugaggagagccgcccaacugcaaaggaaguucccucaccucgaguucagguccauccggggcaaccugaacaccaggcugagaaagcucgacgaacagcaggaguucagcgccaucauccuggccacggccggccugcagaggaugggauggcauaacagggugggccagauccugcacccggaggagugcauguacgccgugggccagggagcccucggcguggaggucagggccaaggaucaggauauccuggaccuggugggcgugcugcacgauccugagacgcugcugaggugcaucgccgagcgggccuuccugcggcaccuagagggcggaugcagcgugccggucgcgguccacaccgcgaugaaggacggccagcuguaccugaccggcggcguguggucccuggacggcagcgauucaauccaggagacgaugcaggccaccauccacgugccagcccagcacgaggauggcccggaggacgacccgcagcuggugggcauuacagccaggaacaucccucggggcccgcagcuggccgcccagaaucugggcaucagccuggcgaaccugcugcucagcaagggagcgaagaacauccuggacguggcccgccagcugaacgaugcccac

SEQ ID NO: 96 - RNA, 1083 nt, Artificial Sequence
  PBGD-CO37
augagcggcaacggcaacgccgccgccaccgccgaggagaacagcccaaagaugcgggugaucagggugggcacccgcaagagccaacucgccagaauccagaccgacagcgugguggccaccuugaaggccagcuacccgggccuccaguucgagaucaucgcuauguccaccaccggcgacaagauccuggacaccgcgcuguccaagaucggcgaaaagagccuguucaccaaggaacuggagcacgcccucgagaagaacgagguggaccugguggugcacucccugaaggaccugccgacgguccugccgccgggcuucaccaucggcgccaucugcaagcgggaaaacccgcacgacgcugugguguuccacccaaaguucgugggcaagacccuggaaacccugccagaaaagagcguggugggcaccagcagccucaggagagccgcccagcugcagaggaaguucccgcaccuggaguucaggagcaucaggggcaaccugaacaccaggcugcguaagcuggacgagcagcaggaguucuccgccaucauccucgccacagccggccuccagaggauggguuggcacaacagggugggccagauccugcacccggaagagugcauguacgcagugggccagggcgcccuuggcguggaagugcgagccaaggaucaggauauccuggaccuggugggcgugcugcacgacccggaaacucugcugcggugcaucgccgaaagggccuuccugcgccaccucgaaggcggcuguagcgugccgguggccgugcacaccgccaugaaggacggccagcuguaccugaccggcggcguguggagccucgacggcagcgacagcauccaggagacaaugcaggccaccauccacgugccggcccagcaugaggauggcccggaggacgacccucagcuggugggcaucaccgcccgcaacaucccaagaggaccgcaacuggccgcccagaaccugggcaucucccuggccaaccugcuccugagcaagggcgcgaagaacauccucgacgucgcacggcagcugaacgacgcccac

SEQ ID NO: 97 - RNA, 1083 nt, Artificial Sequence
  PBGD-CO38
augagcggcaacggcaacgccgccgcgacggccgaggaaaauagcccgaagaugcgggugaucagggugggcaccaggaagucccagcucgccaggauccagaccgacagcgugguggccacccucaaggccuccuacccgggccuccaauucgagaucaucgccauguccaccaccggcgacaagauccucgacaccgcccugagcaagaucggcgaaaagucgcuguucaccaaggagcuggagcacgcccucgagaagaacgagguggaccugguagugcacucccuaaaggaccugccgaccgugcugccgccgggcuucacgaucggcgccaucugcaagcgcgagaacccgcaugaugccgucguuuuccacccuaaguucgugggcaagacccuggagacgcugccggagaagucgguggugggaaccagcagccugaggagggccgcacaacugcagaggaaguucccgcaucuggaguuccgcagcauucgaggcaaccugaacacgcgccugagaaagcucgaugaacagcaggaguucagcgccaucauucuggccacugccggacugcagcggaugggcuggcacaacagagugggccagauccugcauccggaagaguguauguacgccgugggccagggugcccugggcguggaggugcgggccaaggaccaggauauacuggaucuggucggcgugcuccacgacccagaaacacuccugaggugcaucgcugagagagccuuccuccggcaccucgagggcggcuguuccgugccgguggccguccauaccgccaugaaggacggucagcuguaccugaccggaggcguuuggucccuggacggcagcgacagcauccaggaaaccaugcaggccaccauccacgugccggcgcagcacgaggacggcccggaagacgacccgcagcuggucggcaucacggccagaaacaucccgcggggcccgcagcuggcggcccagaaccugggaaucucccuggccaaccugcugcugagcaagggcgcgaagaacauccuggacguggccaggcagcugaacgaugcccac

SEQ ID NO: 98 - RNA, 1083 nt, Artificial Sequence
  PBGD-CO39
augagcgguaacggcaacgccgccgccaccgccgaggagaacuccccgaagaugcgcgugauucgggucggcacaagaaagucucaacucgcccgaauccaaacggacagcgugguggccacccucaaggcgagcuacccgggccuccaguucgaaaucaucgccaugagcaccaccggcgacaagauccuggacaccgcccugucgaagauuggcgaaaagucccuguucaccaaggagcuggagcacgcccuggagaagaacgaagucgaccuggucgugcacagccugaaggaccugccgaccguucugccgccgggcuucaccaucggagccaucugcaagcgggagaauccgcacgacgccguggucuuccacccaaaguucgugggaaagacccucgagacacugccggagaaguccguggugggaaccuccucccugcggagggccgcccaacugcagcggaaguucccacaccuggaauuccgguccaucagaggcaaccucaacaccaggcugaggaagcucgaugagcagcaggaguucagcgccaucauccuggccacagccggacugcagcgcaugggcuggcauaacagagugggccagauccuccacccggaggagugcauguacgccgugggacaaggcgcgcugggcguggaaguucgggccaaggaccaggauauccuggaccuggugggcgugcuccacgacccagagacgcugcugcggugcaucgccgagcgcgccuuccugcggcaccucgagggcggcugcagcgugccggucgcugugcacacagccaugaaggacggccagcuguaccugaccggcggcguguggagucuggacggcagcgacuccauccaggagacuaugcaagccaccauccaugugccggcccaacaugaggacggcccggaggacgacccgcaacuggugggcaucaccgcccggaacaucccgaggggcccgcagcuggccgcccagaaccugggcauuagccuggccaaccugcuccugagcaagggcgcuaagaacauccuggacgucgccagacagcugaacgacgcccac

SEQ ID NO: 99 - RNA, 1083 nt, Artificial Sequence
  PBGD-CO40A
augagcggcaacggcaacgccgccgccaccgccgaggagaacagccccaagaugcgggugauccgggugggcacccguaagagccagcuggcccggauccagaccgacagcgugguggccacccugaaggccagcuaccccggccugcaguucgagaucaucgccaugagcaccaccggcgacaagauccuggacaccgcccugagcaagaucggcgagaagucccuguucaccaaggagcuggagcacgcccuggagaagaacgagguggaccugguggugcacagccugaaggaccugcccaccgugcugccuccaggcuucaccaucggcgccaucugcaagcgggagaacccccacgacgccgugguguuccaccccaaguucgugggcaagacccuggaaacccugccugagaaguccgucguaggaaccagcagccugcggcgggccgcccagcugcagcggaaguucccccaccuggaguuccggagcauccggggcaaccugaacacccggcugcggaagcuggacgagcagcaggaguucagcgccaucauccuggcuaccgccggucugcaacgaaugggcuggcacaauagggugggccagauccugcaccccgaggagugcauguacgcggugggacagggcgcccugggcguggaggugcgggccaaggaccaggacauccuugaucuggugggcgugcugcacgaccccgagacgcugcugcggugcaucgccgagcgggccuuccugcggcauuuggagggcggaugcagcgugcccguggccgugcacaccgccaugaaggacggccagcuguaccugaccggcggcguguggagccuggacggcagcgacagcauccaggaaaccaugcaggccaccauccacgugccugcucagcacgaagacggcccagaggacgacccccagcugguaggcaucaccgcccggaacaucccccggggcccucagcucgccgcacagaaccuuggaaucagccuggccaaccugcuguugucaaagggcgccaagaauauccucgacguggcccggcagcugaacgacgcccac

SEQ ID NO: 100 - RNA, 1083 nt, Artificial Sequence
  PBGD-CO41A
augagcggcaacggcaacgccgccgccaccgccgaggagaacagccccaagaugcgggugauccgggugggcaccagaaagagccagcuggcccggauccagaccgacagcgugguggccacccugaaggccagcuaccccggccugcaguucgagaucaucgccaugagcaccaccggcgacaagauccuggacaccgcccugagcaagaucggcgagaagagucuguucaccaaggagcuggagcacgcccuggagaagaacgagguggaccugguggugcacagccugaaggaccugcccaccgugcugccgccuggcuucaccaucggcgccaucugcaagcgggagaacccccacgacgccgugguguuccaccccaaguucgugggcaagacucuggaaacccugccugagaaguccguggucggaacaagcagccugcggcgggccgcccagcugcagcggaaguucccccaccuggaguuccggagcauccggggcaaccugaacacccggcugcggaagcuggacgagcagcaggaguucagcgccaucauccuggccacagccggccuucagaggaugggcuggcacaaucggguaggccagauccugcaccccgaggagugcauguacgcgguaggucagggcgcccugggcguggaggugcgggccaaggaccaggacaucuuagaucugguuggcgugcugcacgaccccgaaacacugcugcggugcaucgccgagcgggccuuccugcggcaccucgagggcggcugcagugugcccguggccgugcacaccgccaugaaggacggccagcuguaccugaccggcggcguguggagccuggacggcagcgacagcauccaggagacaaugcaggccaccauccacgugccagcucagcacgaagacggaccagaggacgacccccaguuagugggaaucaccgcccggaacaucccccggggcccucagcucgcggcccagaaccugggcaucagccuggccaaccugcugcugucuaagggcgccaagaacauccuagacguggcccggcagcugaacgacgcccac

SEQ ID NO: 101 - RNA, 1083 nt, Artificial Sequence
  PBGD-CO42A
augagcggcaacggcaacgccgccgccaccgccgaggagaacagccccaagaugcgggugauccgggugggcaccaggaagucacagcuggcccggauccagaccgacagcgugguggccacccugaaggccagcuaccccggccugcaguucgagaucaucgccaugagcaccaccggcgacaagauccuggacaccgcccugagcaagaucggcgagaagucccuguucaccaaggagcuggagcacgcccuggagaagaacgagguggaccugguggugcacagccugaaggaccugcccaccgugcugccgccaggcuucaccaucggcgccaucugcaagcgggagaacccccacgacgccgugguguuccaccccaaguucgugggcaagacccuugaaacccugccagagaagucuguggucggcaccagcagccugcggcgggccgcccagcugcagcggaaguucccccaccuggaguuccggagcauccggggcaaccugaacacccggcugcggaagcuggacgagcagcaggaguucagcgccaucauccuggccaccgcuggccuacagcggaugggcuggcacaauagaguuggucagauccugcaccccgaggagugcauguacgccgucggccagggcgcccugggcguggaggugcgggccaaggaccaggacauacuagaccucgugggcgugcugcacgaccccgaaaccuugcugcggugcaucgccgagcgggccuuccugcggcaccuggaaggcgguugcagcgugcccguggccgugcacaccgccaugaaggacggccagcuguaccugaccggcggcguguggagccuggacggcagcgacagcauccaggagacaaugcaggccaccauccacgugccggcccaacacgaggacggaccugaggacgacccccagcuugugggaaucaccgcccggaacaucccccggggcccucaacuggcagcccagaacuuaggcauaagccuggccaaccugcugcuguccaagggcgccaagaacauccucgauguggcccggcagcugaacgacgcccac

SEQ ID NO: 102 - RNA, 1083 nt, Artificial Sequence
  PBGD-CO43A
augagcggcaacggcaacgccgccgccaccgccgaggagaacagccccaagaugcgggugauccgggugggcacccgcaagagucagcuggcccggauccagaccgacagcgugguggccacccugaaggccagcuaccccggccugcaguucgagaucaucgccaugagcaccaccggcgacaagauccuggacaccgcccugagcaagaucggcgagaagagucuguucaccaaggagcuggagcacgcccuggagaagaacgagguggaccugguggugcacagccugaaggaccugcccaccgugcugccaccuggcuucaccaucggcgccaucugcaagcgggagaacccccacgacgccgugguguuccaccccaaguucgugggcaagacacuggaaacccugccggagaaguccgugguaggcaccagcagccugcggcgggccgcccagcugcagcggaaguucccccaccuggaguuccggagcauccggggcaaccugaacacccggcugcggaagcuggacgagcagcaggaguucagcgccaucauccuggcaacagccggcuuacagcguaugggcuggcacaacagggugggacagauccugcaccccgaggagugcauguacgcugugggccagggcgcccugggcguggaggugcgggccaaggaccaggacaucuuagaucucgucggcgugcugcacgaccccgaaaccuugcugcggugcaucgccgagcgggccuuccugcggcaucuugagggcggaugcuccgugcccguggccgugcacaccgccaugaaggacggccagcuguaccugaccggcggcguguggagccuggacggcagcgacagcauccaggagacuaugcaggccaccauccacgugccagcccagcacgaagacggcccagaggacgacccccagcuggugggaaucaccgcccggaacaucccccggggcccucaacuggccgcacagaaccuaggcaucagccuggccaaccugcugcucagcaagggcgccaagaauaucuuggacguggcccggcagcugaacgacgcccac

SEQ ID NO: 103 - RNA, 1083 nt, Artificial Sequence
  PBGD-CO44A
augagcggcaacggcaacgccgccgccaccgccgaggagaacagccccaagaugcgggugauccgggugggcaccagaaagagccagcuggcccggauccagaccgacagcgugguggccacccugaaggccagcuaccccggccugcaguucgagaucaucgccaugagcaccaccggcgacaagauccuggacaccgcccugagcaagaucggcgagaagucucuguucaccaaggagcuggagcacgcccuggagaagaacgagguggaccugguggugcacagccugaaggaccugcccaccgugcugccuccuggcuucaccaucggcgccaucugcaagcgggagaacccccacgacgccgugguguuccaccccaaguucgugggcaagacccuugagacucugccagagaagucuguagugggaaccagcagccugcggcgggccgcccagcugcagcggaaguucccccaccuggaguuccggagcauccggggcaaccugaacacccggcugcggaagcuggacgagcagcaggaguucagcgccaucauccuggccacggccggauuacagagaaugggcuggcacaaccgagugggacagauccugcaccccgaggagugcauguaugccguuggccaaggcgcccugggcguggaggugcgggccaaggaccaggacauccucgaucucgugggcgugcugcacgaccccgagacuuugcugcggugcaucgccgagcgggccuuccugcggcaccuagagggcggcugcucggugcccguggccgugcacaccgccaugaaggacggccagcuguaccugaccggcggcguguggagccuggacggcagcgacagcauccaggagacaaugcaggccaccauccacgugccagcccagcacgaggauggcccugaagacgacccccagcuggugggcaucaccgcccggaacaucccccggggcccacaauuggccgcucagaacuuaggcauuagccuggccaaccugcugcugucuaagggcgccaagaacauacuggacguggcccggcagcugaacgacgcccac

SEQ ID NO: 104 - RNA, 1083 nt, Artificial Sequence
  PBGD-CO45A
augagcggcaacggcaacgccgccgccaccgccgaggagaacagccccaagaugcgggugauccgggugggcacccggaagagccagcuggcccggauccagaccgacagcgugguggccacccugaaggccagcuaccccggccugcaguucgagaucaucgccaugagcaccaccggcgacaagauccuggacaccgcccugagcaagaucggcgagaagagccuguucaccaaggagcuggagcacgcccuggagaagaacgagguggaccugguggugcacagccugaaggaccugcccaccgugcugccccccggcuucaccaucggcgccaucugcaagcgggagaacccccacgacgccgugguguuccaccccaaguucgugggcaagacccuggagacccugcccgagaagagcguggugggcaccagcagccugcggcgggccgcccagcugcagcggaaguucccccaccuggaguuccggagcauccggggcaaccugaacacccggcugcggaagcuggacgagcagcaggaguucagcgccaucauccuggccaccgccggccugcagcggaugggcuggcacaaccgggugggccagauccugcaccccgaggagugcauguacgccgugggccagggcgcccugggcguggaggugcgggccaaggaccaggacauccuggaccuggugggcgugcugcacgaccccgagacccugcugcggugcaucgccgagcgggccuuccugcggcaccuggagggcggcugcagcgugcccguggccgugcacaccgccaugaaggacggccagcuguaccugaccggcggcguguggagccuggacggcagcgacagcauccaggagaccaugcaggccaccauccacgugcccgcccagcacgaggacggccccgaggacgacccccagcuggugggcaucaccgcccggaacaucccccggggcccccagcuggccgcccagaaccugggcaucagccuggccaaccugcugcugagcaagggcgccaagaacauccuggacguggcccggcagcugaacgacgcccac

SEQ ID NO: 105 - RNA, 1083 nt, Artificial Sequence
  PBGD-CO46A
augagcggcaacggcaacgccgccgccaccgccgaggagaacagccccaagaugcgggugauccgggugggcacccggaagagccagcuggcgaggauccagacggacagcgugguggcgacgcugaaggcgagcuacccggggcugcaguucgagaucaucgcgaugagcacgacgggggacaagauccuggacacggcgcugagcaagaucggggagaagagccuguucacgaaggagcuggagcacgcgcuggagaagaacgagguggaccugguggugcacagccugaaggaccugccgacggugcugccgccgggguucacgaucggggcgaucugcaagagggagaacccgcacgacgcggugguguuccacccgaaguucguggggaagacgcuggagacgcugccggagaagagcgugguggggacgagcagccugaggagggcggcgcagcugcagaggaaguucccgcaccuggaguucaggagcaucagggggaaccugaacacgaggcugaggaagcuggacgagcagcaggaguucagcgcgaucauccuggcgacggcggggcugcagaggaugggguggcacaacaggguggggcagauccugcacccggaggagugcauguacgcgguggggcagggggcgcuggggguggaggugagggcgaaggaccaggacauccuggaccuggugggggugcugcacgacccggagacgcugcugaggugcaucgcggagagggcguuccugaggcaccuggagggggggugcagcgugccgguggcggugcacacggcgaugaaggacgggcagcuguaccugacgggggggguguggagccuggacgggagcgacagcauccaggagacgaugcaggcgacgauccacgugccggcgcagcacgaggacgggccggaggacgacccgcagcugguggggaucacggcgaggaacaucccgagggggccgcagcuggcggcgcagaaccuggggaucagccuggcgaaccugcugcugagcaagggggcgaagaacauccuggacguggcgaggcagcugaacgacgcgcac

SEQ ID NO: 106 - RNA, 1083 nt, Artificial Sequence
  PBGD-CO47A
augagcggcaacggcaacgccgccgccaccgccgaggagaacagccccaagaugcgggugauccgggugggcacccggaagagccagcuggcccgcauccagaccgacuccgucgucgccacccucaaggccuccuaccccggccuccaguucgagaucaucgccauguccaccaccggcgacaagauccucgacaccgcccucuccaagaucggcgagaagucccucuucaccaaggagcucgagcacgcccucgagaagaacgaggucgaccucgucguccacucccucaaggaccuccccaccguccucccccccggcuucaccaucggcgccaucugcaagcgcgagaacccccacgacgccgucgucuuccaccccaaguucgucggcaagacccucgagacccuccccgagaaguccgucgucggcaccuccucccuccgccgcgccgcccagcuccagcgcaaguucccccaccucgaguuccgcuccauccgcggcaaccucaacacccgccuccgcaagcucgacgagcagcaggaguucuccgccaucauccucgccaccgccggccuccagcgcaugggcuggcacaaccgcgucggccagauccuccaccccgaggagugcauguacgccgucggccagggcgcccucggcgucgagguccgcgccaaggaccaggacauccucgaccucgucggcguccuccacgaccccgagacccuccuccgcugcaucgccgagcgcgccuuccuccgccaccucgagggcggcugcuccguccccgucgccguccacaccgccaugaaggacggccagcucuaccucaccggcggcgucuggucccucgacggcuccgacuccauccaggagaccaugcaggccaccauccacguccccgcccagcacgaggacggccccgaggacgacccccagcucgucggcaucaccgcccgcaacaucccccgcggcccccagcucgccgcccagaaccucggcaucucccucgccaaccuccuccucuccaagggcgccaagaacauccucgacgucgcccgccagcucaacgacgcccac

SEQ ID NO: 107 - RNA, 1083 nt, Artificial Sequence
  PBGD-CO40B
augagcggcaacggcaacgccgccgccaccgccgaggagaacagccccaagaugcgggugauccgggugggcacccguaagagccagcuggcccggauccagaccgacagcgugguggccacccugaaggccagcuaccccggccugcaguucgagaucaucgccaugagcaccaccggcgacaagauccuggacaccgcccugagcaagaucggcgagaagucccuguucaccaaggagcuggagcacgcccuggagaagaacgagguggaccugguggugcacagccugaaggaccugcccaccgugcugccuccaggcuucaccaucggcgccaucugcaagcgggagaacccucacgacgccgugguguuccaccccaaguucgugggcaagacccuggaaacccugccugagaaguccgucguaggaaccagcagccugcggcgggccgcccagcugcagcggaaguucccacaccuggaguuccggagcauccggggcaaccugaacacccggcugcggaagcuggacgagcagcaggaguucagcgccaucauccuggcuaccgccggucugcaacgaaugggcuggcacaauagggugggccagauccugcaccccgaggagugcauguacgcggugggacagggcgcccugggcguggaggugcgggccaaggaccaggacauccuugaucuggugggcgugcugcacgaccccgagacgcugcugcggugcaucgccgagcgggccuuccugcggcauuuggagggcggaugcagcgugcccguggccgugcacaccgccaugaaggacggccagcuguaccugaccggcggcguguggagccuggacggcagcgacagcauccaggaaaccaugcaggccaccauccacgugccugcucagcacgaagacggcccagaggacgacccucagcugguaggcaucaccgcccggaacaucccucggggcccucagcucgccgcacagaaccuuggaaucagccuggccaaccugcuguugucaaagggcgccaagaauauccucgacguggcccggcagcugaacgacgcccac

SEQ ID NO: 108 - RNA, 1083 nt, Artificial Sequence
  PBGD-CO41B
augagcggcaacggcaacgccgccgccaccgccgaggagaacagccccaagaugcgggugauccgggugggcaccagaaagagccagcuggcccggauccagaccgacagcgugguggccacccugaaggccagcuaccccggccugcaguucgagaucaucgccaugagcaccaccggcgacaagauccuggacaccgcccugagcaagaucggcgagaagagucuguucaccaaggagcuggagcacgcccuggagaagaacgagguggaccugguggugcacagccugaaggaccugcccaccgugcugccgccuggcuucaccaucggcgccaucugcaagcgggagaacccgcacgacgccgugguguuccaccccaaguucgugggcaagacucuggaaacccugccugagaaguccguggucggaacaagcagccugcggcgggccgcccagcugcagcggaaguucccacaccuggaguuccggagcauccggggcaaccugaacacccggcugcggaagcuggacgagcagcaggaguucagcgccaucauccuggccacagccggccuucagaggaugggcuggcacaaucggguaggccagauccugcaccccgaggagugcauguacgcgguaggucagggcgcccugggcguggaggugcgggccaaggaccaggacaucuuagaucugguuggcgugcugcacgaccccgaaacacugcugcggugcaucgccgagcgggccuuccugcggcaccucgagggcggcugcagugugcccguggccgugcacaccgccaugaaggacggccagcuguaccugaccggcggcguguggagccuggacggcagcgacagcauccaggagacaaugcaggccaccauccacgugccagcucagcacgaagacggaccagaggacgacccacaguuagugggaaucaccgcccggaacaucccgcggggcccucagcucgcggcccagaaccugggcaucagccuggccaaccugcugcugucuaagggcgccaagaacauccuagacguggcccggcagcugaacgacgcccac

SEQ ID NO: 109 - RNA, 1083 nt, Artificial Sequence
  PBGD-CO42B
augagcggcaacggcaacgccgccgccaccgccgaggagaacagccccaagaugcgggugauccgggugggcaccaggaagucacagcuggcccggauccagaccgacagcgugguggccacccugaaggccagcuaccccggccugcaguucgagaucaucgccaugagcaccaccggcgacaagauccuggacaccgcccugagcaagaucggcgagaagucccuguucaccaaggagcuggagcacgcccuggagaagaacgagguggaccugguggugcacagccugaaggaccugcccaccgugcugccgccaggcuucaccaucggcgccaucugcaagcgggagaacccgcacgacgccgugguguuccaccccaaguucgugggcaagacccuugaaacccugccagagaagucuguggucggcaccagcagccugcggcgggccgcccagcugcagcggaaguucccgcaccuggaguuccggagcauccggggcaaccugaacacccggcugcggaagcuggacgagcagcaggaguucagcgccaucauccuggccaccgcuggccuacagcggaugggcuggcacaauagaguuggucagauccugcaccccgaggagugcauguacgccgucggccagggcgcccugggcguggaggugcgggccaaggaccaggacauacuagaccucgugggcgugcugcacgaccccgaaaccuugcugcggugcaucgccgagcgggccuuccugcggcaccuggaaggcgguugcagcgugcccguggccgugcacaccgccaugaaggacggccagcuguaccugaccggcggcguguggagccuggacggcagcgacagcauccaggagacaaugcaggccaccauccacgugccggcccaacacgaggacggaccugaggacgacccacagcuugugggaaucaccgcccggaacaucccacggggcccucaacuggcagcccagaacuuaggcauaagccuggccaaccugcugcuguccaagggcgccaagaacauccucgauguggcccggcagcugaacgacgcccac

SEQ ID NO: 110 - RNA, 1083 nt, Artificial Sequence
  PBGD-CO43B
augagcggcaacggcaacgccgccgccaccgccgaggagaacagccccaagaugcgggugauccgggugggcacccgcaagagucagcuggcccggauccagaccgacagcgugguggccacccugaaggccagcuaccccggccugcaguucgagaucaucgccaugagcaccaccggcgacaagauccuggacaccgcccugagcaagaucggcgagaagagucuguucaccaaggagcuggagcacgcccuggagaagaacgagguggaccugguggugcacagccugaaggaccugcccaccgugcugccaccuggcuucaccaucggcgccaucugcaagcgggagaacccacacgacgccgugguguuccaccccaaguucgugggcaagacacuggaaacccugccggagaaguccgugguaggcaccagcagccugcggcgggccgcccagcugcagcggaaguucccgcaccuggaguuccggagcauccggggcaaccugaacacccggcugcggaagcuggacgagcagcaggaguucagcgccaucauccuggcaacagccggcuuacagcguaugggcuggcacaacagggugggacagauccugcaccccgaggagugcauguacgcugugggccagggcgcccugggcguggaggugcgggccaaggaccaggacaucuuagaucucgucggcgugcugcacgaccccgaaaccuugcugcggugcaucgccgagcgggccuuccugcggcaucuugagggcggaugcuccgugcccguggccgugcacaccgccaugaaggacggccagcuguaccugaccggcggcguguggagccuggacggcagcgacagcauccaggagacuaugcaggccaccauccacgugccagcccagcacgaagacggcccagaggacgacccacagcuggugggaaucaccgcccggaacaucccgcggggcccucaacuggccgcacagaaccuaggcaucagccuggccaaccugcugcucagcaagggcgccaagaauaucuuggacguggcccggcagcugaacgacgcccac

SEQ ID NO: 111 - RNA, 1083 nt, Artificial Sequence
  PBGD-CO44B
augagcggcaacggcaacgccgccgccaccgccgaggagaacagccccaagaugcgggugauccgggugggcaccagaaagagccagcuggcccggauccagaccgacagcgugguggccacccugaaggccagcuaccccggccugcaguucgagaucaucgccaugagcaccaccggcgacaagauccuggacaccgcccugagcaagaucggcgagaagucucuguucaccaaggagcuggagcacgcccuggagaagaacgagguggaccugguggugcacagccugaaggaccugcccaccgugcugccuccuggcuucaccaucggcgccaucugcaagcgggagaacccacacgacgccgugguguuccaccccaaguucgugggcaagacccuugagacucugccagagaagucuguagugggaaccagcagccugcggcgggccgcccagcugcagcggaaguucccucaccuggaguuccggagcauccggggcaaccugaacacccggcugcggaagcuggacgagcagcaggaguucagcgccaucauccuggccacggccggauuacagagaaugggcuggcacaaccgagugggacagauccugcaccccgaggagugcauguaugccguuggccaaggcgcccugggcguggaggugcgggccaaggaccaggacauccucgaucucgugggcgugcugcacgaccccgagacuuugcugcggugcaucgccgagcgggccuuccugcggcaccuagagggcggcugcucggugcccguggccgugcacaccgccaugaaggacggccagcuguaccugaccggcggcguguggagccuggacggcagcgacagcauccaggagacaaugcaggccaccauccacgugccagcccagcacgaggauggcccugaagacgacccacagcuggugggcaucaccgcccggaacaucccgcggggcccacaauuggccgcucagaacuuaggcauuagccuggccaaccugcugcugucuaagggcgccaagaacauacuggacguggcccggcagcugaacgacgcccac

SEQ ID NO: 112 - RNA, 1083 nt, Artificial Sequence
  PBGD-CO45B
augagcggcaacggcaacgccgccgccaccgccgaggagaacagccccaagaugcgggugauccgggugggcacccggaagagccagcuggcccggauccagaccgacagcgugguggccacccugaaggccagcuaccccggccugcaguucgagaucaucgccaugagcaccaccggcgacaagauccuggacaccgcccugagcaagaucggcgagaagagccuguucaccaaggagcuggagcacgcccuggagaagaacgagguggaccugguggugcacagccugaaggaccugcccaccgugcugccgcccggcuucaccaucggcgccaucugcaagcgggagaacccgcacgacgccgugguguuccaccccaaguucgugggcaagacccuggagacccugcccgagaagagcguggugggcaccagcagccugcggcgggccgcccagcugcagcggaaguucccucaccuggaguuccggagcauccggggcaaccugaacacccggcugcggaagcuggacgagcagcaggaguucagcgccaucauccuggccaccgccggccugcagcggaugggcuggcacaaccgggugggccagauccugcaccccgaggagugcauguacgccgugggccagggcgcccugggcguggaggugcgggccaaggaccaggacauccuggaccuggugggcgugcugcacgaccccgagacccugcugcggugcaucgccgagcgggccuuccugcggcaccuggagggcggcugcagcgugcccguggccgugcacaccgccaugaaggacggccagcuguaccugaccggcggcguguggagccuggacggcagcgacagcauccaggagaccaugcaggccaccauccacgugcccgcccagcacgaggacggccccgaggacgacccucagcuggugggcaucaccgcccggaacaucccacggggcccucagcuggccgcccagaaccugggcaucagccuggccaaccugcugcugagcaagggcgccaagaacauccuggacguggcccggcagcugaacgacgcccac

SEQ ID NO: 113 - RNA, 1083 nt, Artificial Sequence
  PBGD-CO46B
augagcggcaacggcaacgccgccgccaccgccgaggagaacagccccaagaugcgggugauccgggugggcacccggaagagccagcuggcgaggauccagacggacagcgugguggcgacgcugaaggcgagcuacccggggcugcaguucgagaucaucgcgaugagcacgacgggcgacaagauccuggacacggcgcugagcaagaucggggagaagagccuguucacgaaggagcuggagcacgcgcuggagaagaacgagguggaccugguggugcacagccugaaggaccugccgacggugcugccgccgggguucacgaucggggcgaucugcaagagggagaacccgcacgacgcggugguguuccacccgaaguucguggggaagacgcuggagacgcugccggagaagagcgugguggggacgagcagccugaggagggcggcgcagcugcagaggaaguucccgcaccuggaguucaggagcaucagggguaaccugaacacgaggcugaggaagcuggacgagcagcaggaguucagcgcgaucauccuggcgacggcggggcugcagaggaugggguggcacaacaggguggggcagauccugcacccggaggagugcauguacgcgguggggcagggcgcgcugggcguggaggugagggcgaaggaccaggacauccuggaccuggugggcgugcugcacgacccggagacgcugcugaggugcaucgcggagagggcguuccugaggcaccuggagggcgggugcagcgugccgguggcggugcacacggcgaugaaggacgggcagcuguaccugacgggagggguguggagccuggacgggagcgacagcauccaggagacgaugcaggcgacgauccacgugccggcgcagcacgaggacgggccggaggacgacccgcagcugguggggaucacggcgaggaacaucccgagggguccgcagcuggcggcgcagaaccuggggaucagccuggcgaaccugcugcugagcaagggagcgaagaacauccuggacguggcgaggcagcugaacgacgcgcac

SEQ ID NO: 114 - RNA, 1083 nt, Artificial Sequence
  PBGD-CO47B
augagcggcaacggcaacgccgccgccaccgccgaggagaacagccccaagaugcgggugauccgggugggcacccggaagagccagcuggcccgcauccagaccgacuccgucgucgccacccucaaggccuccuaccccggccuccaguucgagaucaucgccauguccaccaccggcgacaagauccucgacaccgcccucuccaagaucggcgagaagucccucuucaccaaggagcucgagcacgcccucgagaagaacgaggucgaccucgucguccacucccucaaggaccuccccaccguccucccacccggcuucaccaucggcgccaucugcaagcgcgagaacccucacgacgccgucgucuuccaccccaaguucgucggcaagacccucgagacccuccccgagaaguccgucgucggcaccuccucccuccgccgcgccgcccagcuccagcgcaaguucccacaccucgaguuccgcuccauccgcggcaaccucaacacccgccuccgcaagcucgacgagcagcaggaguucuccgccaucauccucgccaccgccggccuccagcgcaugggcuggcacaaccgcgucggccagauccuccaccccgaggagugcauguacgccgucggccagggcgcccucggcgucgagguccgcgccaaggaccaggacauccucgaccucgucggcguccuccacgaccccgagacccuccuccgcugcaucgccgagcgcgccuuccuccgccaccucgagggcggcugcuccguccccgucgccguccacaccgccaugaaggacggccagcucuaccucaccggcggcgucuggucccucgacggcuccgacuccauccaggagaccaugcaggccaccauccacguccccgcccagcacgaggacggccccgaggacgacccucagcucgucggcaucaccgcccgcaacaucccgcgcggcccucagcucgccgcccagaaccucggcaucucccucgccaaccuccuccucuccaagggcgccaagaacauccucgacgucgcccgccagcucaacgacgcccac

SEQ ID NO: 115 - RNA, 1083 nt, Artificial Sequence
  CONSTRUCT #29
auguccggaaacggaaacgccgccgcuaccgccgaggaaaauagcccgaagaugagagugauccggguggguaccaggaagucccagcucgccaggauccaaacggacucggugguggccacccucaaggcuagcuacccgggccugcaauucgagaucauugcuauguccaccaccggcgacaagauccuggauacggcccuguccaagaucggcgaaaagagccucuucaccaaggagcuggaacacgcgcucgagaagaacgagguggaccuggucguccacagccucaaggaccugccuacggugcugccgccgggauucaccaucggcgccaucuguaagcgggagaauccgcacgacgccgugguguuccacccuaaguucgugggcaagacccucgagacacugccggaaaaguccgucgugggcaccuccucccugagaagggccgcucagcuccagagaaaguucccgcaccuggaauucaggagcauccggggcaaccugaauacccggcuucgcaagcuggacgagcagcaggaguucagcgccaucauccuggccaccgccggccugcagcggaugggcuggcacaaccgggugggccagauccugcacccggaggagugcauguaugccgugggucagggagcccugggcguggagguccgggccaaggaccaggacauccuggaccucgugggcgugcuccacgacccugaaacccuccugaggugcaucgccgagagggccuuccuccggcaccuggagggcggcuguuccgucccuguggccgugcauaccgccaugaaggacggacagcuguaccugaccggcggcguguggucccuggacggcuccgacagcauccaggaaaccaugcaggccacuauccacgugccggcccagcacgaagacggcccagaggaugacccgcaacuggucggcauuaccgccaggaacauaccaaggggcccgcagcuggccgcccagaaccugggcaucucccuggccaaccugcugcuguccaagggagccaagaacauucuggacguggccaggcagcucaaugaugcccac

SEQ ID NO: 116 - RNA, 1083 nt, Artificial Sequence
  CONSTRUCT #30
augagcggcaacggcaacgccgccgccaccgcagaggagaauagcccgaagaugagggugauccgagugggcaccaggaagucccagcuugcgcgaauucagaccgacagcgugguggccacccucaaggccuccuacccgggacuccaguucgagaucaucgccaugagcaccacgggagacaagauccuggacaccgcccuguccaagaucggcgaaaagagccucuucaccaaggagcuggagcacgcccuggagaagaacgaggucgaucugguggugcacagccugaaggaccugccgaccguccugccgccgggauucaccaucggugccaucuguaagcgggagaacccgcacgacgccgugguguuccacccgaaguucgucggcaagacccuggaaacccugccggagaaguccguggugggcaccagcagccugaggcgggccgcccagcugcagcggaaguucccgcaccuggaauucaggagcauccggggcaaccugaacacccggcugcggaagcuggacgagcagcaggaguucagcgccaucauccuggccaccgcaggccuccagcgcaugggauggcacaacaggguaggccaaauccugcacccggaggaguguauguacgccgugggccagggagcccugggcguggaggugagagccaaggaccaggacauccuagaccuggucggcgugcugcacgacccggagacacugcugagaugcaucgcggagagagccuuccugcgacaccuggagggcggcugcuccgugccgguggccgugcacaccgccaugaaggacggccagcuguaucugaccggcggcguguggagccuggacggcagcgacuccauccaagaaaccaugcaggcuaccauccacgugccggcccagcacgaggauggaccagaggacgauccucaacuggugggcaucacugccaggaacaucccaagaggcccgcagcuggccgcccagaaccugggcaucagccuggccaaccugcugcuguccaagggcgccaagaacauucucgauguggccaggcagcugaacgaugcccac

SEQ ID NO: 117 - RNA, 1083 nt, Artificial Sequence
  CONSTRUCT #31
augucgggaaacggcaacgccgccgccacggccgaggagaacagcccgaagaugagagugauuagggugggcacccggaagucccaacucgcgcggauccagaccgacuccgugguggccacccucaaggccagcuacccgggccuccaguucgagauuaucgccauguccaccacaggcgacaagauccucgacaccgcacucucgaagaucggcgagaagucccuguucaccaaggaacuggagcacgcccuggagaagaacgagguggaccugguggugcacucccugaaggaccugccgaccgugcucccaccaggcuucaccaucggcgcaaucuguaagcgcgagaauccgcacgacgccgugguguuccacccaaaguucgugggcaagacccucgaaacccucccggaaaagagcgugguggguaccagcucccugcggagagcugcccagcugcagagaaaguucccgcaucuggaauucaggagcaucaggggaaaucugaauaccagacugcgcaagcuggacgagcagcaggaguucagcgccaucauccuggccaccgccggccugcagcggaugggcuggcacaacagggugggccagauacugcauccggaggaguguauguacgccgugggccagggcgcccucggcguggaggugagagccaaggaccaagacauccuggaccuagugggcgugcugcaugacccugaaacccugcucaggugcaucgccgagagggccuuccugcggcaccuggagggcggcugcagcgugccgguggccguccacaccgccaugaaggacggccagcuguaccugaccggcggcgucuggagccuggacggauccgacagcauccaggaaaccaugcaggccaccauccacgugccggcccagcacgaggacggcccugaggacgacccucagcuggugggcaucaccgcuaggaacaucccaaggggcccgcagcuggccgcccagaaccucggcaucagccuggccaaccugcugcuguccaagggcgccaagaauauccuggacguggccaggcagcugaacgacgcccac

SEQ ID NO: 118 - RNA, 1294 nt, Artificial Sequence
  CONSTRUCT #1
gggaaauaagagagaaaagaagaguaagaagaaauauaagagccaccaugagcggcaacggcaacgccgcagccaccgccgaggaaaacagccccaagaugcgggugaucagagugggcacccggaagagccagcuggcccggauccagaccgacagcgugguggccacccugaaggccuccuaccccggccugcaguucgagaucauugccaugagcaccaccggcgacaagauccuggacaccgcccugagcaagaucggcgagaagagccuguucacaaaagagcuggaacacgcccuggaaaagaacgagguggaccugguggugcacagccugaaggaccugcccaccgugcugcccccuggcuucaccaucggcgccaucugcaagagagagaacccccacgacgccgugguguuccacccuaaguucgugggcaagacacuggaaacccugcccgagaaguccguggugggcaccagcagccugcggagagccgcccagcugcagcggaaguucccccaccuggaauuucggagcauccggggcaaccugaacacccggcugcggaagcuggacgagcagcaggaauuuuccgcuaucauccuggccacagccggacugcagcggaugggcuggcacaacagagugggccagauccugcaccccgaggaaugcauguacgccgugggccagggagcccugggcguggaagugcgggccaaggaccaggacauccuggaucuggugggcgugcugcaugaccccgagacacugcugcgguguaucgccgagcgggccuuccugcggcaccuggaaggcggcugcagcgugcccguggccgugcacaccgccaugaaggacggacagcuguaccugacaggcggcguguggagccuggacggcagcgacagcauccaggagaccaugcaggccaccauccacgugcccgcccagcacgaggacggccccgaggacgacccucagcuggucggcaucaccgcccggaacauccccagaggcccccagcuggccgcccagaaccugggcaucagccuggccaaccugcugcuguccaagggcgccaagaacauccuggacguggcccggcagcugaacgacgcccacugauaauaguccauaaaguaggaaacacuacagcuggagccucgguggccaugcuucuugccccuugggccuccccccagccccuccuccccuuccugcacccguaccccccgcauuauuacucacgguacgaguggucuuugaauaaagucugagugggcggc

SEQ ID NO: 119 - RNA, 1294 nt, Artificial Sequence
  CONSTRUCT #2
gggaaauaagagagaaaagaagaguaagaagaaauauaagagccaccaugagcggcaacggcaacgccgccgcuaccgccgaagagaacagcccaaagaugcgcgugaucagggucggcacgcgcaagucccagcucgcccggauccaaaccgauagcgugguggccacgcucaaggcgagcuauccgggcuuacaguucgagaucaucgccaugagcaccaccggcgauaagauacuggacaccgcccuguccaagaucggcgaaaagagccuguucaccaaggaacuggagcacgcgcuggagaagaacgagguggaccugguggugcacagccugaaggaccugccgaccgugcugccgccgggauucaccaucggcgccaucugcaagagggagaauccgcacgaugccgugguguuccacccaaaguucgugggcaagaccuuggaaacccugccagagaagucuguggucggcaccuccagccugcggcgagccgcccagcugcagcgaaaguucccgcaccuggaguucagguccauccgcggaaaucugaacaccaggcugcgcaagcucgacgagcagcaggaguucuccgccaucauccuggccaccgcaggccuccaaagaaugggcuggcauaaccgagucggccagauccuccacccggaggagugcauguacgcagugggccaaggcgcccugggcgucgaggugcgugccaaggaccaggacauccuggaccuggugggcgugcuccacgauccagagacacugcugagaugcaucgcggagcgcgccuuccugcgccaucuggagggaggcugcuccgucccgguggccguacauaccgccaugaaggacggucagcuguaccucaccggcggcguauggucccucgacgguagcgacagcauacaggagacgaugcaggccaccauccacgugccggcgcagcacgaggauggaccagaggacgacccgcagcugguggguaucaccgccaggaauaucccgcggggaccucagcuggccgcccagaaccugggcaucucccucgccaaccuccugcugagcaagggcgccaagaacauccuggacguggccaggcagcucaacgaugcccauugauaauaguccauaaaguaggaaacacuacagcuggagccucgguggccaugcuucuugccccuugggccuccccccagccccuccuccccuuccugcacccguaccccccgcauuauuacucacgguacgaguggucuuugaauaaagucugagugggcggc

SEQ ID NO: 120 - RNA, 1294 nt, Artificial Sequence
  CONSTRUCT #3
gggaaauaagagagaaaagaagaguaagaagaaauauaagagccaccaugagcggcaacggcaacgccgccgccaccgccgaggaaaacagcccgaagaugcgggugaucagggugggcaccaggaagucccagcucgcccggauccagaccgacagcguggucgccaccuugaaggccuccuacccgggccuccaguucgagaucaucgccauguccacaaccggcgacaagauccuggauaccgcccucagcaagaucggcgagaagucccuguucaccaaggagcuggagcacgcccuggagaagaaugagguggaccugguggugcacagccugaaggaccugccuaccgugcugccaccaggcuucacaaucggcgccaucugcaagagagagaacccgcacgacgccgugguguuccauccgaaguucgugggcaagacccuggaaacccugccggagaaguccguagugggaaccucaagccugaggcgcgccgcccagcuccagaggaaguucccucaccuggaauuccgguccaucaggggcaaccugaacacgcgccugcggaagcucgacgagcagcaggaguucuccgccaucauccuggccacagccggccuucagcgcaugggcuggcacaacagggugggccagauccugcacccggaagaaugcauguacgccgugggccaaggcgcccucggcguggaagugcgugccaaggaccaggacauccuggaccuggugggcgugcugcacgacccugagacgcugcucaggugcaucgccgaacgcgcguuccugcggcaccuggagggaggcugcagcgucccgguggccguccacaccgccaugaaggacggccagcucuaccugacuggcggcguguggagccuggacggcagcgacagcauucaggaaaccaugcaggccaccauccacgugccugcccagcacgaggacggcccggaggacgacccucaacuggugggcauuacugcgcgaaacaucccgcgcggaccucagcuggccgcccagaaccugggcaucagccuggccaaccugcuccuguccaagggcgccaagaacauccucgacguggccaggcagcugaacgacgcgcacugauaauaguccauaaaguaggaaacacuacagcuggagccucgguggccaugcuucuugccccuugggccuccccccagccccuccuccccuuccugcacccguaccccccgcauuauuacucacgguacgaguggucuuugaauaaagucugagugggcggc

SEQ ID NO: 121 - RNA, 1294 nt, Artificial Sequence
  CONSTRUCT #4
gggaaauaagagagaaaagaagaguaagaagaaauauaagagccaccaugagcggcaacggaaacgccgccgcgaccgcggaggagaacucgccuaagaugagagugauaaggguaggcacccggaagucucaacucgccaggauccagaccgacagcgugguggccacccucaaggccagcuauccaggacuccaguucgaaaucaucgccauguccaccacaggcgauaagauccuggacaccgcccuguccaagaucggcgagaagucccucuucaccaaggaacuggagcacgcccuggagaagaacgaggucgaucuggucgugcacagccugaaggaucugccuaccgugcucccgccgggcuucaccaucggcgccaucugcaagagggagaauccucacgacgccgugguguuccacccgaaguucgugggcaagacccuggagacacugccagaaaagucgguggugggcaccagcagccugcggcgggcggcccagcugcagcggaaguucccacaccuggaguucagguccauccguggcaaucugaacacccggcugcguaagcuggacgagcagcaggaauucagcgcgaucauccuggcaaccgccggucugcaaaggaugggcuggcacaacagggugggccagauccugcacccugaggagugcauguacgccgugggccagggagcccugggcguggaagugcgggccaaggaccaggacauccuggaccuggugggugugcuccacgacccugaaacccugcugcggugcaucgccgaaagggccuuccugaggcaccucgagggcggcugcagcgugccggucgccgugcacaccgccaugaaggacggccagcuguaccugaccggaggaguguggagccuggacggcuccgacuccauccaggagacuaugcaggccaccauucaugugccggcccagcaugaggacgguccggaggacgauccacagcuggucggcaucaccgcgcggaacaucccaagaggcccgcaacuggccgcucagaaccugggcauaucccuggccaaccugcuccugagcaagggcgccaagaacauccuggacguggccaggcagcugaaugacgcccacugauaauaguccauaaaguaggaaacacuacagcuggagccucgguggccaugcuucuugccccuugggccuccccccagccccuccuccccuuccugcacccguaccccccgcauuauuacucacgguacgaguggucuuugaauaaagucugagugggcggc

SEQ ID NO: 122 - RNA, 1294 nt, Artificial Sequence
  CONSTRUCT #5
gggaaauaagagagaaaagaagaguaagaagaaauauaagagccaccauguccggcaacggcaacgccgccgcuaccgccgaggagaacuccccuaagaugcgggucaucagggugggcacccgaaagucccaacuugcccggauccagaccgacuccgucguggccacccucaaggcuagcuauccaggccuccaguucgaaaucaucgccaugagcaccaccggcgacaagauucuggacaccgcccuguccaagaucggcgagaagagucuguucacgaaggagcucgagcacgcccuggaaaagaacgagguggaccugguggugcauucccugaaggaccugccaaccgugcugccgccgggcuucacuauaggagccaucugcaagcgggagaacccgcacgacgcggugguguuccauccgaaguucgugggcaagacucuggaaacccugccggagaaguccguggugggaacuagcucccugcggcgggccgcccagcugcagaggaaguucccgcaccuggaguucaggagcauacgcggcaaccugaacacccgccugcguaagcucgacgagcagcaggaauucagugccaucauccuggccacggcgggccugcagcggaugggcuggcacaacagggugggccagauccuccacccggaggaauguauguacgccgugggccagggcgcacugggcguggagguccgcgccaaggaccaagacauccuggaccuggucggcgugcugcacgacccugaaacccugcugaggugcauugccgagagagccuuccugaggcaucuggagggcggcugcagcgugccuguggccgugcacacagccaugaaggacggucagcuguaccugaccggcggcguguggagccuggacggcagcgacuccauccaggagacaaugcaggccaccauccacgucccggcccaacacgaggacggaccugaggacgauccucagcuggugggcaucaccgccaggaacaucccucggggcccgcagcuggccgcccagaaccugggcaucucccucgccaaccugcugcuguccaagggcgccaagaacauccucgacguggccagacagcugaacgacgcccacugauaauaguccauaaaguaggaaacacuacagcuggagccucgguggccaugcuucuugccccuugggccuccccccagccccuccuccccuuccugcacccguaccccccgcauuauuacucacgguacgaguggucuuugaauaaagucugagugggcggc

SEQ ID NO: 123 - RNA, 1294 nt, Artificial Sequence
  CONSTRUCT #6
gggaaauaagagagaaaagaagaguaagaagaaauauaagagccaccaugagcggcaacggcaacgccgccgccaccgccgaggagaacagcccgaagaugagggugauaagggugggcacacggaagucccagcucgcccgcauccaaaccgacuccgugguggccacccucaaggccagcuacccgggccuccaauucgagaucaucgccaugagcaccaccggcgacaagauccuggacaccgcccugucuaagauaggcgaaaagagccuguucaccaaggagcuggagcaugcccuggagaagaacgagguggaccuggugguccacagucucaaggaccugccaaccgugcugccgccaggcuucaccaucggcgccaucugcaagcgugagaacccgcacgaugcugugguguuccacccuaaguucgugggaaagacccuggagacgcugccggaaaagagcguggucggcaccuccagccugcggagggccgcccaacuccagaggaaguucccgcaccuggaguucaggagcauccgcggcaaccugaacaccaggcugcgaaagcuggacgagcagcaggaauucucggccaucauccucgccaccgccggcuugcaaagaaugggcuggcauaaucgcgugggccagauccugcacccugaggagugcauguacgccgugggccagggugcucugggaguggaggugcgggccaaggaccaggauauccuggaccuggucggcgugcuucaugacccggagacgcuccugaggugcaucgccgagcgggccuuccugagacaccuggagggcggcugcuccgugccaguggccgugcacaccgccaugaaggacggacagcuguaccugaccggcggcguguggagccuggacggaagcgacagcauccaagaaaccaugcaggcgaccauucacgucccugcccagcacgaggauggaccagaggacgacccgcagcuggugggcaucaccgcccgcaacaucccuagaggcccacagcuggccgcccagaaucugggcaucagccuggccaaccugcugcugucuaagggagccaagaacauccuggacguggccaggcagcugaacgacgcccauugauaauaguccauaaaguaggaaacacuacagcuggagccucgguggccaugcuucuugccccuugggccuccccccagccccuccuccccuuccugcacccguaccccccgcauuauuacucacgguacgaguggucuuugaauaaagucugagugggcggc

SEQ ID NO: 124 - RNA, 1294 nt, Artificial Sequence
  CONSTRUCT #7
gggaaauaagagagaaaagaagaguaagaagaaauauaagagccaccauguccggcaacggcaacgccgcagccaccgccgaggagaauuccccgaagaugcgggugauccgggugggcaccagaaagagccagcucgcccgcauccaaaccgacuccgugguggccacccucaaggccuccuacccaggcuugcaguucgaaaucaucgccaugagcaccaccggcgacaagauccuggacaccgcccugagcaagauuggcgagaagucccuguucaccaaggagcuggagcaugcucuggagaagaacgagguggaccucguggugcacucccugaaggaccugccgacugugcugccgccuggcuucacgaucggcgccauaugcaagcgggaaaacccacacgacgccguggucuuccacccaaaguucgugggcaagacccuggaaacccugccggaaaagagcguggucggcacaagcucccugaggagagccgcccaacugcaaaggaaguucccucaccucgaguucagguccauccggggcaaccugaacaccaggcugagaaagcucgacgaacagcaggaguucagcgccaucauccuggccacggccggccugcagaggaugggauggcauaacagggugggccagauccugcacccggaggagugcauguacgccgugggccagggagcccucggcguggaggucagggccaaggaucaggauauccuggaccuggugggcgugcugcacgauccugagacgcugcugaggugcaucgccgagcgggccuuccugcggcaccuagagggcggaugcagcgugccggucgcgguccacaccgcgaugaaggacggccagcuguaccugaccggcggcguguggucccuggacggcagcgauucaauccaggagacgaugcaggccaccauccacgugccagcccagcacgaggauggcccggaggacgacccgcagcuggugggcauuacagccaggaacaucccucggggcccgcagcuggccgcccagaaucugggcaucagccuggcgaaccugcugcucagcaagggagcgaagaacauccuggacguggcccgccagcugaacgaugcccacugauaauaguccauaaaguaggaaacacuacagcuggagccucgguggccaugcuucuugccccuugggccuccccccagccccuccuccccuuccugcacccguaccccccgcauuauuacucacgguacgaguggucuuugaauaaagucugagugggcggc

SEQ ID NO: 125 - RNA, 1294 nt, Artificial Sequence
  CONSTRUCT #8
gggaaauaagagagaaaagaagaguaagaagaaauauaagagccaccaugagcggcaacggcaacgccgccgccaccgccgaggagaacagcccaaagaugcgggugaucagggugggcacccgcaagagccaacucgccagaauccagaccgacagcgugguggccaccuugaaggccagcuacccgggccuccaguucgagaucaucgcuauguccaccaccggcgacaagauccuggacaccgcgcuguccaagaucggcgaaaagagccuguucaccaaggaacuggagcacgcccucgagaagaacgagguggaccugguggugcacucccugaaggaccugccgacgguccugccgccgggcuucaccaucggcgccaucugcaagcgggaaaacccgcacgacgcugugguguuccacccaaaguucgugggcaagacccuggaaacccugccagaaaagagcguggugggcaccagcagccucaggagagccgcccagcugcagaggaaguucccgcaccuggaguucaggagcaucaggggcaaccugaacaccaggcugcguaagcuggacgagcagcaggaguucuccgccaucauccucgccacagccggccuccagaggauggguuggcacaacagggugggccagauccugcacccggaagagugcauguacgcagugggccagggcgcccuuggcguggaagugcgagccaaggaucaggauauccuggaccuggugggcgugcugcacgacccggaaacucugcugcggugcaucgccgaaagggccuuccugcgccaccucgaaggcggcuguagcgugccgguggccgugcacaccgccaugaaggacggccagcuguaccugaccggcggcguguggagccucgacggcagcgacagcauccaggagacaaugcaggccaccauccacgugccggcccagcaugaggauggcccggaggacgacccucagcuggugggcaucaccgcccgcaacaucccaagaggaccgcaacuggccgcccagaaccugggcaucucccuggccaaccugcuccugagcaagggcgcgaagaacauccucgacgucgcacggcagcugaacgacgcccacugauaauaguccauaaaguaggaaacacuacagcuggagccucgguggccaugcuucuugccccuugggccuccccccagccccuccuccccuuccugcacccguaccccccgcauuauuacucacgguacgaguggucuuugaauaaagucugagugggcggc

SEQ ID NO: 126 - RNA, 1294 nt, Artificial Sequence
  CONSTRUCT #9
gggaaauaagagagaaaagaagaguaagaagaaauauaagagccaccaugagcggcaacggcaacgccgccgcgacggccgaggaaaauagcccgaagaugcgggugaucagggugggcaccaggaagucccagcucgccaggauccagaccgacagcgugguggccacccucaaggccuccuacccgggccuccaauucgagaucaucgccauguccaccaccggcgacaagauccucgacaccgcccugagcaagaucggcgaaaagucgcuguucaccaaggagcuggagcacgcccucgagaagaacgagguggaccugguagugcacucccuaaaggaccugccgaccgugcugccgccgggcuucacgaucggcgccaucugcaagcgcgagaacccgcaugaugccgucguuuuccacccuaaguucgugggcaagacccuggagacgcugccggagaagucgguggugggaaccagcagccugaggagggccgcacaacugcagaggaaguucccgcaucuggaguuccgcagcauucgaggcaaccugaacacgcgccugagaaagcucgaugaacagcaggaguucagcgccaucauucuggccacugccggacugcagcggaugggcuggcacaacagagugggccagauccugcauccggaagaguguauguacgccgugggccagggugcccugggcguggaggugcgggccaaggaccaggauauacuggaucuggucggcgugcuccacgacccagaaacacuccugaggugcaucgcugagagagccuuccuccggcaccucgagggcggcuguuccgugccgguggccguccauaccgccaugaaggacggucagcuguaccugaccggaggcguuuggucccuggacggcagcgacagcauccaggaaaccaugcaggccaccauccacgugccggcgcagcacgaggacggcccggaagacgacccgcagcuggucggcaucacggccagaaacaucccgcggggcccgcagcuggcggcccagaaccugggaaucucccuggccaaccugcugcugagcaagggcgcgaagaacauccuggacguggccaggcagcugaacgaugcccacugauaauaguccauaaaguaggaaacacuacagcuggagccucgguggccaugcuucuugccccuugggccuccccccagccccuccuccccuuccugcacccguaccccccgcauuauuacucacgguacgaguggucuuugaauaaagucugagugggcggc

SEQ ID NO: 127 - RNA, 1294 nt, Artificial Sequence
  CONSTRUCT #10
gggaaauaagagagaaaagaagaguaagaagaaauauaagagccaccaugagcgguaacggcaacgccgccgccaccgccgaggagaacuccccgaagaugcgcgugauucgggucggcacaagaaagucucaacucgcccgaauccaaacggacagcgugguggccacccucaaggcgagcuacccgggccuccaguucgaaaucaucgccaugagcaccaccggcgacaagauccuggacaccgcccugucgaagauuggcgaaaagucccuguucaccaaggagcuggagcacgcccuggagaagaacgaagucgaccuggucgugcacagccugaaggaccugccgaccguucugccgccgggcuucaccaucggagccaucugcaagcgggagaauccgcacgacgccguggucuuccacccaaaguucgugggaaagacccucgagacacugccggagaaguccguggugggaaccuccucccugcggagggccgcccaacugcagcggaaguucccacaccuggaauuccgguccaucagaggcaaccucaacaccaggcugaggaagcucgaugagcagcaggaguucagcgccaucauccuggccacagccggacugcagcgcaugggcuggcauaacagagugggccagauccuccacccggaggagugcauguacgccgugggacaaggcgcgcugggcguggaaguucgggccaaggaccaggauauccuggaccuggugggcgugcuccacgacccagagacgcugcugcggugcaucgccgagcgcgccuuccugcggcaccucgagggcggcugcagcgugccggucgcugugcacacagccaugaaggacggccagcuguaccugaccggcggcguguggagucuggacggcagcgacuccauccaggagacuaugcaagccaccauccaugugccggcccaacaugaggacggcccggaggacgacccgcaacuggugggcaucaccgcccggaacaucccgaggggcccgcagcuggccgcccagaaccugggcauuagccuggccaaccugcuccugagcaagggcgcuaagaacauccuggacgucgccagacagcugaacgacgcccacugauaauaguccauaaaguaggaaacacuacagcuggagccucgguggccaugcuucuugccccuugggccuccccccagccccuccuccccuuccugcacccguaccccccgcauuauuacucacgguacgaguggucuuugaauaaagucugagugggcggc

SEQ ID NO: 128 - RNA, 1294 nt, Artificial Sequence
  CONSTRUCT #11
gggaaauaagagagaaaagaagaguaagaagaaauauaagagccaccaugagcggcaacggcaacgccgccgccaccgccgaggagaacagccccaagaugcgggugauccgggugggcacccguaagagccagcuggcccggauccagaccgacagcgugguggccacccugaaggccagcuaccccggccugcaguucgagaucaucgccaugagcaccaccggcgacaagauccuggacaccgcccugagcaagaucggcgagaagucccuguucaccaaggagcuggagcacgcccuggagaagaacgagguggaccugguggugcacagccugaaggaccugcccaccgugcugccuccaggcuucaccaucggcgccaucugcaagcgggagaacccccacgacgccgugguguuccaccccaaguucgugggcaagacccuggaaacccugccugagaaguccgucguaggaaccagcagccugcggcgggccgcccagcugcagcggaaguucccccaccuggaguuccggagcauccggggcaaccugaacacccggcugcggaagcuggacgagcagcaggaguucagcgccaucauccuggcuaccgccggucugcaacgaaugggcuggcacaauagggugggccagauccugcaccccgaggagugcauguacgcggugggacagggcgcccugggcguggaggugcgggccaaggaccaggacauccuugaucuggugggcgugcugcacgaccccgagacgcugcugcggugcaucgccgagcgggccuuccugcggcauuuggagggcggaugcagcgugcccguggccgugcacaccgccaugaaggacggccagcuguaccugaccggcggcguguggagccuggacggcagcgacagcauccaggaaaccaugcaggccaccauccacgugccugcucagcacgaagacggcccagaggacgacccccagcugguaggcaucaccgcccggaacaucccccggggcccucagcucgccgcacagaaccuuggaaucagccuggccaaccugcuguugucaaagggcgccaagaauauccucgacguggcccggcagcugaacgacgcccacugauaauaguccauaaaguaggaaacacuacagcuggagccucgguggccaugcuucuugccccuugggccuccccccagccccuccuccccuuccugcacccguaccccccgcauuauuacucacgguacgaguggucuuugaauaaagucugagugggcggc

SEQ ID NO: 129 - RNA, 1294 nt, Artificial Sequence
  CONSTRUCT #12
gggaaauaagagagaaaagaagaguaagaagaaauauaagagccaccaugagcggcaacggcaacgccgccgccaccgccgaggagaacagccccaagaugcgggugauccgggugggcaccagaaagagccagcuggcccggauccagaccgacagcgugguggccacccugaaggccagcuaccccggccugcaguucgagaucaucgccaugagcaccaccggcgacaagauccuggacaccgcccugagcaagaucggcgagaagagucuguucaccaaggagcuggagcacgcccuggagaagaacgagguggaccugguggugcacagccugaaggaccugcccaccgugcugccgccuggcuucaccaucggcgccaucugcaagcgggagaacccccacgacgccgugguguuccaccccaaguucgugggcaagacucuggaaacccugccugagaaguccguggucggaacaagcagccugcggcgggccgcccagcugcagcggaaguucccccaccuggaguuccggagcauccggggcaaccugaacacccggcugcggaagcuggacgagcagcaggaguucagcgccaucauccuggccacagccggccuucagaggaugggcuggcacaaucggguaggccagauccugcaccccgaggagugcauguacgcgguaggucagggcgcccugggcguggaggugcgggccaaggaccaggacaucuuagaucugguuggcgugcugcacgaccccgaaacacugcugcggugcaucgccgagcgggccuuccugcggcaccucgagggcggcugcagugugcccguggccgugcacaccgccaugaaggacggccagcuguaccugaccggcggcguguggagccuggacggcagcgacagcauccaggagacaaugcaggccaccauccacgugccagcucagcacgaagacggaccagaggacgacccccaguuagugggaaucaccgcccggaacaucccccggggcccucagcucgcggcccagaaccugggcaucagccuggccaaccugcugcugucuaagggcgccaagaacauccuagacguggcccggcagcugaacgacgcccacugauaauaguccauaaaguaggaaacacuacagcuggagccucgguggccaugcuucuugccccuugggccuccccccagccccuccuccccuuccugcacccguaccccccgcauuauuacucacgguacgaguggucuuugaauaaagucugagugggcggc

SEQ ID NO: 130 - RNA, 1294 nt, Artificial Sequence
  CONSTRUCT #13
gggaaauaagagagaaaagaagaguaagaagaaauauaagagccaccaugagcggcaacggcaacgccgccgccaccgccgaggagaacagccccaagaugcgggugauccgggugggcaccaggaagucacagcuggcccggauccagaccgacagcgugguggccacccugaaggccagcuaccccggccugcaguucgagaucaucgccaugagcaccaccggcgacaagauccuggacaccgcccugagcaagaucggcgagaagucccuguucaccaaggagcuggagcacgcccuggagaagaacgagguggaccugguggugcacagccugaaggaccugcccaccgugcugccgccaggcuucaccaucggcgccaucugcaagcgggagaacccccacgacgccgugguguuccaccccaaguucgugggcaagacccuugaaacccugccagagaagucuguggucggcaccagcagccugcggcgggccgcccagcugcagcggaaguucccccaccuggaguuccggagcauccggggcaaccugaacacccggcugcggaagcuggacgagcagcaggaguucagcgccaucauccuggccaccgcuggccuacagcggaugggcuggcacaauagaguuggucagauccugcaccccgaggagugcauguacgccgucggccagggcgcccugggcguggaggugcgggccaaggaccaggacauacuagaccucgugggcgugcugcacgaccccgaaaccuugcugcggugcaucgccgagcgggccuuccugcggcaccuggaaggcgguugcagcgugcccguggccgugcacaccgccaugaaggacggccagcuguaccugaccggcggcguguggagccuggacggcagcgacagcauccaggagacaaugcaggccaccauccacgugccggcccaacacgaggacggaccugaggacgacccccagcuugugggaaucaccgcccggaacaucccccggggcccucaacuggcagcccagaacuuaggcauaagccuggccaaccugcugcuguccaagggcgccaagaacauccucgauguggcccggcagcugaacgacgcccacugauaauaguccauaaaguaggaaacacuacagcuggagccucgguggccaugcuucuugccccuugggccuccccccagccccuccuccccuuccugcacccguaccccccgcauuauuacucacgguacgaguggucuuugaauaaagucugagugggcggc

SEQ ID NO: 131 - RNA, 1294 nt, Artificial Sequence
  CONSTRUCT #14
gggaaauaagagagaaaagaagaguaagaagaaauauaagagccaccaugagcggcaacggcaacgccgccgccaccgccgaggagaacagccccaagaugcgggugauccgggugggcacccgcaagagucagcuggcccggauccagaccgacagcgugguggccacccugaaggccagcuaccccggccugcaguucgagaucaucgccaugagcaccaccggcgacaagauccuggacaccgcccugagcaagaucggcgagaagagucuguucaccaaggagcuggagcacgcccuggagaagaacgagguggaccugguggugcacagccugaaggaccugcccaccgugcugccaccuggcuucaccaucggcgccaucugcaagcgggagaacccccacgacgccgugguguuccaccccaaguucgugggcaagacacuggaaacccugccggagaaguccgugguaggcaccagcagccugcggcgggccgcccagcugcagcggaaguucccccaccuggaguuccggagcauccggggcaaccugaacacccggcugcggaagcuggacgagcagcaggaguucagcgccaucauccuggcaacagccggcuuacagcguaugggcuggcacaacagggugggacagauccugcaccccgaggagugcauguacgcugugggccagggcgcccugggcguggaggugcgggccaaggaccaggacaucuuagaucucgucggcgugcugcacgaccccgaaaccuugcugcggugcaucgccgagcgggccuuccugcggcaucuugagggcggaugcuccgugcccguggccgugcacaccgccaugaaggacggccagcuguaccugaccggcggcguguggagccuggacggcagcgacagcauccaggagacuaugcaggccaccauccacgugccagcccagcacgaagacggcccagaggacgacccccagcuggugggaaucaccgcccggaacaucccccggggcccucaacuggccgcacagaaccuaggcaucagccuggccaaccugcugcucagcaagggcgccaagaauaucuuggacguggcccggcagcugaacgacgcccacugauaauaguccauaaaguaggaaacacuacagcuggagccucgguggccaugcuucuugccccuugggccuccccccagccccuccuccccuuccugcacccguaccccccgcauuauuacucacgguacgaguggucuuugaauaaagucugagugggcggc

SEQ ID NO: 132 - RNA, 1294 nt, Artificial Sequence
  CONSTRUCT #15
gggaaauaagagagaaaagaagaguaagaagaaauauaagagccaccaugaguggcaacggaaacgccgccgcuacagcagaggagaacuccccgaagaugcgcgugauuaggguaggcaccagaaagucucagcuggccagaauccaaaccgauagcguuguggccacauugaaggcuagcuaucccggccugcaguucgagaucaucgccaugagcaccaccggcgacaagauacucgacaccgcucugaguaaaaucggcgagaagagccuguuuaccaaggagcuggagcacgcccuggaaaagaacgaaguggaccugguggugcauagucugaaagaccuucccaccguccuuccaccaggcuucacuaucggcgccaucugcaagagggagaauccucacgaugccgucguguuucaucccaaguucgugggcaagaccuuagaaacccugccagagaaaagcgucguugggaccuccucccugcgacgggccgcccagcugcagagaaaguucccccacuuggaauucagauccaucagagggaaucugaauacucgccugagaaagcuggacgagcagcaggaguuuagcgcuaucauccuggccacggcugguuugcagagaaugggcuggcacaaccgggugggacagauccugcaccccgaggagugcauguaugcaguaggccagggggcccuggggguggaggucagagccaaagaucaggacauccuggaccuggucggcgugcugcacgaucccgaaacacugcugcgguguaucgccgagagggcuuuccuccggcacuuagagggcggcugcuccguccccguggccguucacacugccaugaaagacgggcagcuguaccugacgggcggcguguggucccuggacggcucagacuccauucaggagaccaugcaagcuaccauccacgucccugcccaacacgaagauggccccgaggacgacccccagcuggugggcaucaccgccaggaauaucccaagaggcccccaguuggccgcccagaaccugggcaucagucuggccaaccugcugcugaguaagggcgccaaaaacauccuggacguggcucggcagcugaaugacgcccacugauaauaguccauaaaguaggaaacacuacagcuggagccucgguggccaugcuucuugccccuugggccuccccccagccccuccuccccuuccugcacccguaccccccgcauuauuacucacgguacgaguggucuuugaauaaagucugagugggcggc

SEQ ID NO: 133 - RNA, 1294 nt, Artificial Sequence
  CONSTRUCT #16
gggaaauaagagagaaaagaagaguaagaagaaauauaagagccaccaugagcggcaacggcaacgccgccgccaccgccgaggagaacagccccaagaugcgggugauccgggugggcacccggaagagccagcuggcccggauccagaccgacagcgugguggccacccugaaggccagcuaccccggccugcaguucgagaucaucgccaugagcaccaccggcgacaagauccuggacaccgcccugagcaagaucggcgagaagagccuguucaccaaggagcuggagcacgcccuggagaagaacgagguggaccugguggugcacagccugaaggaccugcccaccgugcugccccccggcuucaccaucggcgccaucugcaagcgggagaacccccacgacgccgugguguuccaccccaaguucgugggcaagacccuggagacccugcccgagaagagcguggugggcaccagcagccugcggcgggccgcccagcugcagcggaaguucccccaccuggaguuccggagcauccggggcaaccugaacacccggcugcggaagcuggacgagcagcaggaguucagcgccaucauccuggccaccgccggccugcagcggaugggcuggcacaaccgggugggccagauccugcaccccgaggagugcauguacgccgugggccagggcgcccugggcguggaggugcgggccaaggaccaggacauccuggaccuggugggcgugcugcacgaccccgagacccugcugcggugcaucgccgagcgggccuuccugcggcaccuggagggcggcugcagcgugcccguggccgugcacaccgccaugaaggacggccagcuguaccugaccggcggcguguggagccuggacggcagcgacagcauccaggagaccaugcaggccaccauccacgugcccgcccagcacgaggacggccccgaggacgacccccagcuggugggcaucaccgcccggaacaucccccggggcccccagcuggccgcccagaaccugggcaucagccuggccaaccugcugcugagcaagggcgccaagaacauccuggacguggcccggcagcugaacgacgcccacugauaauaguccauaaaguaggaaacacuacagcuggagccucgguggccaugcuucuugccccuugggccuccccccagccccuccuccccuuccugcacccguaccccccgcauuauuacucacgguacgaguggucuuugaauaaagucugagugggcggc

SEQ ID NO: 134 - RNA, 1294 nt, Artificial Sequence
  CONSTRUCT #16
gggaaauaagagagaaaagaagaguaagaagaaauauaagagccaccaugagcggcaacggcaacgccgccgccaccgccgaggagaacagccccaagaugcgggugauccgggugggcacccggaagagccagcuggcgaggauccagacggacagcgugguggcgacgcugaaggcgagcuacccggggcugcaguucgagaucaucgcgaugagcacgacgggggacaagauccuggacacggcgcugagcaagaucggggagaagagccuguucacgaaggagcuggagcacgcgcuggagaagaacgagguggaccugguggugcacagccugaaggaccugccgacggugcugccgccgggguucacgaucggggcgaucugcaagagggagaacccgcacgacgcggugguguuccacccgaaguucguggggaagacgcuggagacgcugccggagaagagcgugguggggacgagcagccugaggagggcggcgcagcugcagaggaaguucccgcaccuggaguucaggagcaucagggggaaccugaacacgaggcugaggaagcuggacgagcagcaggaguucagcgcgaucauccuggcgacggcggggcugcagaggaugggguggcacaacaggguggggcagauccugcacccggaggagugcauguacgcgguggggcagggggcgcuggggguggaggugagggcgaaggaccaggacauccuggaccuggugggggugcugcacgacccggagacgcugcugaggugcaucgcggagagggcguuccugaggcaccuggagggggggugcagcgugccgguggcggugcacacggcgaugaaggacgggcagcuguaccugacgggggggguguggagccuggacgggagcgacagcauccaggagacgaugcaggcgacgauccacgugccggcgcagcacgaggacgggccggaggacgacccgcagcugguggggaucacggcgaggaacaucccgagggggccgcagcuggcggcgcagaaccuggggaucagccuggcgaaccugcugcugagcaagggggcgaagaacauccuggacguggcgaggcagcugaacgacgcgcacugauaauaguccauaaaguaggaaacacuacagcuggagccucgguggccaugcuucuugccccuugggccuccccccagccccuccuccccuuccugcacccguaccccccgcauuauuacucacgguacgaguggucuuugaauaaagucugagugggcggc

SEQ ID NO: 135 - RNA, 1294 nt, Artificial Sequence
  CONSTRUCT #17
gggaaauaagagagaaaagaagaguaagaagaaauauaagagccaccaugagcggcaacggcaacgccgccgccaccgccgaggagaacagccccaagaugcgggugauccgggugggcacccggaagagccagcuggcccgcauccagaccgacuccgucgucgccacccucaaggccuccuaccccggccuccaguucgagaucaucgccauguccaccaccggcgacaagauccucgacaccgcccucuccaagaucggcgagaagucccucuucaccaaggagcucgagcacgcccucgagaagaacgaggucgaccucgucguccacucccucaaggaccuccccaccguccucccccccggcuucaccaucggcgccaucugcaagcgcgagaacccccacgacgccgucgucuuccaccccaaguucgucggcaagacccucgagacccuccccgagaaguccgucgucggcaccuccucccuccgccgcgccgcccagcuccagcgcaaguucccccaccucgaguuccgcuccauccgcggcaaccucaacacccgccuccgcaagcucgacgagcagcaggaguucuccgccaucauccucgccaccgccggccuccagcgcaugggcuggcacaaccgcgucggccagauccuccaccccgaggagugcauguacgccgucggccagggcgcccucggcgucgagguccgcgccaaggaccaggacauccucgaccucgucggcguccuccacgaccccgagacccuccuccgcugcaucgccgagcgcgccuuccuccgccaccucgagggcggcugcuccguccccgucgccguccacaccgccaugaaggacggccagcucuaccucaccggcggcgucuggucccucgacggcuccgacuccauccaggagaccaugcaggccaccauccacguccccgcccagcacgaggacggccccgaggacgacccccagcucgucggcaucaccgcccgcaacaucccccgcggcccccagcucgccgcccagaaccucggcaucucccucgccaaccuccuccucuccaagggcgccaagaacauccucgacgucgcccgccagcucaacgacgcccacugauaauaguccauaaaguaggaaacacuacagcuggagccucgguggccaugcuucuugccccuugggccuccccccagccccuccuccccuuccugcacccguaccccccgcauuauuacucacgguacgaguggucuuugaauaaagucugagugggcggc

SEQ ID NO: 136 - RNA, 1294 nt, Artificial Sequence
  CONSTRUCT #18
gggaaauaagagagaaaagaagaguaagaagaaauauaagagccaccaugagcggcaacggcaacgccgccgccaccgccgaggagaacagccccaagaugcgggugauccgggugggcacccguaagagccagcuggcccggauccagaccgacagcgugguggccacccugaaggccagcuaccccggccugcaguucgagaucaucgccaugagcaccaccggcgacaagauccuggacaccgcccugagcaagaucggcgagaagucccuguucaccaaggagcuggagcacgcccuggagaagaacgagguggaccugguggugcacagccugaaggaccugcccaccgugcugccuccaggcuucaccaucggcgccaucugcaagcgggagaacccucacgacgccgugguguuccaccccaaguucgugggcaagacccuggaaacccugccugagaaguccgucguaggaaccagcagccugcggcgggccgcccagcugcagcggaaguucccacaccuggaguuccggagcauccggggcaaccugaacacccggcugcggaagcuggacgagcagcaggaguucagcgccaucauccuggcuaccgccggucugcaacgaaugggcuggcacaauagggugggccagauccugcaccccgaggagugcauguacgcggugggacagggcgcccugggcguggaggugcgggccaaggaccaggacauccuugaucuggugggcgugcugcacgaccccgagacgcugcugcggugcaucgccgagcgggccuuccugcggcauuuggagggcggaugcagcgugcccguggccgugcacaccgccaugaaggacggccagcuguaccugaccggcggcguguggagccuggacggcagcgacagcauccaggaaaccaugcaggccaccauccacgugccugcucagcacgaagacggcccagaggacgacccucagcugguaggcaucaccgcccggaacaucccucggggcccucagcucgccgcacagaaccuuggaaucagccuggccaaccugcuguugucaaagggcgccaagaauauccucgacguggcccggcagcugaacgacgcccacugauaauaguccauaaaguaggaaacacuacagcuggagccucgguggccaugcuucuugccccuugggccuccccccagccccuccuccccuuccugcacccguaccccccgcauuauuacucacgguacgaguggucuuugaauaaagucugagugggcggc

SEQ ID NO: 137 - RNA, 1294 nt, Artificial Sequence
  CONSTRUCT #19
gggaaauaagagagaaaagaagaguaagaagaaauauaagagccaccaugagcggcaacggcaacgccgccgccaccgccgaggagaacagccccaagaugcgggugauccgggugggcaccagaaagagccagcuggcccggauccagaccgacagcgugguggccacccugaaggccagcuaccccggccugcaguucgagaucaucgccaugagcaccaccggcgacaagauccuggacaccgcccugagcaagaucggcgagaagagucuguucaccaaggagcuggagcacgcccuggagaagaacgagguggaccugguggugcacagccugaaggaccugcccaccgugcugccgccuggcuucaccaucggcgccaucugcaagcgggagaacccgcacgacgccgugguguuccaccccaaguucgugggcaagacucuggaaacccugccugagaaguccguggucggaacaagcagccugcggcgggccgcccagcugcagcggaaguucccacaccuggaguuccggagcauccggggcaaccugaacacccggcugcggaagcuggacgagcagcaggaguucagcgccaucauccuggccacagccggccuucagaggaugggcuggcacaaucggguaggccagauccugcaccccgaggagugcauguacgcgguaggucagggcgcccugggcguggaggugcgggccaaggaccaggacaucuuagaucugguuggcgugcugcacgaccccgaaacacugcugcggugcaucgccgagcgggccuuccugcggcaccucgagggcggcugcagugugcccguggccgugcacaccgccaugaaggacggccagcuguaccugaccggcggcguguggagccuggacggcagcgacagcauccaggagacaaugcaggccaccauccacgugccagcucagcacgaagacggaccagaggacgacccacaguuagugggaaucaccgcccggaacaucccgcggggcccucagcucgcggcccagaaccugggcaucagccuggccaaccugcugcugucuaagggcgccaagaacauccuagacguggcccggcagcugaacgacgcccacugauaauaguccauaaaguaggaaacacuacagcuggagccucgguggccaugcuucuugccccuugggccuccccccagccccuccuccccuuccugcacccguaccccccgcauuauuacucacgguacgaguggucuuugaauaaagucugagugggcggc

SEQ ID NO: 138 - RNA, 1294 nt, Artificial Sequence
  CONSTRUCT #20
gggaaauaagagagaaaagaagaguaagaagaaauauaagagccaccaugagcggcaacggcaacgccgccgccaccgccgaggagaacagccccaagaugcgggugauccgggugggcaccaggaagucacagcuggcccggauccagaccgacagcgugguggccacccugaaggccagcuaccccggccugcaguucgagaucaucgccaugagcaccaccggcgacaagauccuggacaccgcccugagcaagaucggcgagaagucccuguucaccaaggagcuggagcacgcccuggagaagaacgagguggaccugguggugcacagccugaaggaccugcccaccgugcugccgccaggcuucaccaucggcgccaucugcaagcgggagaacccgcacgacgccgugguguuccaccccaaguucgugggcaagacccuugaaacccugccagagaagucuguggucggcaccagcagccugcggcgggccgcccagcugcagcggaaguucccgcaccuggaguuccggagcauccggggcaaccugaacacccggcugcggaagcuggacgagcagcaggaguucagcgccaucauccuggccaccgcuggccuacagcggaugggcuggcacaauagaguuggucagauccugcaccccgaggagugcauguacgccgucggccagggcgcccugggcguggaggugcgggccaaggaccaggacauacuagaccucgugggcgugcugcacgaccccgaaaccuugcugcggugcaucgccgagcgggccuuccugcggcaccuggaaggcgguugcagcgugcccguggccgugcacaccgccaugaaggacggccagcuguaccugaccggcggcguguggagccuggacggcagcgacagcauccaggagacaaugcaggccaccauccacgugccggcccaacacgaggacggaccugaggacgacccacagcuugugggaaucaccgcccggaacaucccacggggcccucaacuggcagcccagaacuuaggcauaagccuggccaaccugcugcuguccaagggcgccaagaacauccucgauguggcccggcagcugaacgacgcccacugauaauaguccauaaaguaggaaacacuacagcuggagccucgguggccaugcuucuugccccuugggccuccccccagccccuccuccccuuccugcacccguaccccccgcauuauuacucacgguacgaguggucuuugaauaaagucugagugggcggc

SEQ ID NO: 139 - RNA, 1294 nt, Artificial Sequence
  CONSTRUCT #21
gggaaauaagagagaaaagaagaguaagaagaaauauaagagccaccaugagcggcaacggcaacgccgccgccaccgccgaggagaacagccccaagaugcgggugauccgggugggcacccgcaagagucagcuggcccggauccagaccgacagcgugguggccacccugaaggccagcuaccccggccugcaguucgagaucaucgccaugagcaccaccggcgacaagauccuggacaccgcccugagcaagaucggcgagaagagucuguucaccaaggagcuggagcacgcccuggagaagaacgagguggaccugguggugcacagccugaaggaccugcccaccgugcugccaccuggcuucaccaucggcgccaucugcaagcgggagaacccacacgacgccgugguguuccaccccaaguucgugggcaagacacuggaaacccugccggagaaguccgugguaggcaccagcagccugcggcgggccgcccagcugcagcggaaguucccgcaccuggaguuccggagcauccggggcaaccugaacacccggcugcggaagcuggacgagcagcaggaguucagcgccaucauccuggcaacagccggcuuacagcguaugggcuggcacaacagggugggacagauccugcaccccgaggagugcauguacgcugugggccagggcgcccugggcguggaggugcgggccaaggaccaggacaucuuagaucucgucggcgugcugcacgaccccgaaaccuugcugcggugcaucgccgagcgggccuuccugcggcaucuugagggcggaugcuccgugcccguggccgugcacaccgccaugaaggacggccagcuguaccugaccggcggcguguggagccuggacggcagcgacagcauccaggagacuaugcaggccaccauccacgugccagcccagcacgaagacggcccagaggacgacccacagcuggugggaaucaccgcccggaacaucccgcggggcccucaacuggccgcacagaaccuaggcaucagccuggccaaccugcugcucagcaagggcgccaagaauaucuuggacguggcccggcagcugaacgacgcccacugauaauaguccauaaaguaggaaacacuacagcuggagccucgguggccaugcuucuugccccuugggccuccccccagccccuccuccccuuccugcacccguaccccccgcauuauuacucacgguacgaguggucuuugaauaaagucugagugggcggc

SEQ ID NO: 140 - RNA, 1294 nt, Artificial Sequence
  CONSTRUCT #22
gggaaauaagagagaaaagaagaguaagaagaaauauaagagccaccaugagcggcaacggcaacgccgccgccaccgccgaggagaacagccccaagaugcgggugauccgggugggcaccagaaagagccagcuggcccggauccagaccgacagcgugguggccacccugaaggccagcuaccccggccugcaguucgagaucaucgccaugagcaccaccggcgacaagauccuggacaccgcccugagcaagaucggcgagaagucucuguucaccaaggagcuggagcacgcccuggagaagaacgagguggaccugguggugcacagccugaaggaccugcccaccgugcugccuccuggcuucaccaucggcgccaucugcaagcgggagaacccacacgacgccgugguguuccaccccaaguucgugggcaagacccuugagacucugccagagaagucuguagugggaaccagcagccugcggcgggccgcccagcugcagcggaaguucccucaccuggaguuccggagcauccggggcaaccugaacacccggcugcggaagcuggacgagcagcaggaguucagcgccaucauccuggccacggccggauuacagagaaugggcuggcacaaccgagugggacagauccugcaccccgaggagugcauguaugccguuggccaaggcgcccugggcguggaggugcgggccaaggaccaggacauccucgaucucgugggcgugcugcacgaccccgagacuuugcugcggugcaucgccgagcgggccuuccugcggcaccuagagggcggcugcucggugcccguggccgugcacaccgccaugaaggacggccagcuguaccugaccggcggcguguggagccuggacggcagcgacagcauccaggagacaaugcaggccaccauccacgugccagcccagcacgaggauggcccugaagacgacccacagcuggugggcaucaccgcccggaacaucccgcggggcccacaauuggccgcucagaacuuaggcauuagccuggccaaccugcugcugucuaagggcgccaagaacauacuggacguggcccggcagcugaacgacgcccacugauaauaguccauaaaguaggaaacacuacagcuggagccucgguggccaugcuucuugccccuugggccuccccccagccccuccuccccuuccugcacccguaccccccgcauuauuacucacgguacgaguggucuuugaauaaagucugagugggcggc

SEQ ID NO: 141 - RNA, 1294 nt, Artificial Sequence
  CONSTRUCT #24
gggaaauaagagagaaaagaagaguaagaagaaauauaagagccaccaugagcggcaacggcaacgccgccgccaccgccgaggagaacagccccaagaugcgggugauccgggugggcacccggaagagccagcuggcccggauccagaccgacagcgugguggccacccugaaggccagcuaccccggccugcaguucgagaucaucgccaugagcaccaccggcgacaagauccuggacaccgcccugagcaagaucggcgagaagagccuguucaccaaggagcuggagcacgcccuggagaagaacgagguggaccugguggugcacagccugaaggaccugcccaccgugcugccgcccggcuucaccaucggcgccaucugcaagcgggagaacccgcacgacgccgugguguuccaccccaaguucgugggcaagacccuggagacccugcccgagaagagcguggugggcaccagcagccugcggcgggccgcccagcugcagcggaaguucccucaccuggaguuccggagcauccggggcaaccugaacacccggcugcggaagcuggacgagcagcaggaguucagcgccaucauccuggccaccgccggccugcagcggaugggcuggcacaaccgggugggccagauccugcaccccgaggagugcauguacgccgugggccagggcgcccugggcguggaggugcgggccaaggaccaggacauccuggaccuggugggcgugcugcacgaccccgagacccugcugcggugcaucgccgagcgggccuuccugcggcaccuggagggcggcugcagcgugcccguggccgugcacaccgccaugaaggacggccagcuguaccugaccggcggcguguggagccuggacggcagcgacagcauccaggagaccaugcaggccaccauccacgugcccgcccagcacgaggacggccccgaggacgacccucagcuggugggcaucaccgcccggaacaucccacggggcccucagcuggccgcccagaaccugggcaucagccuggccaaccugcugcugagcaagggcgccaagaacauccuggacguggcccggcagcugaacgacgcccacugauaauaguccauaaaguaggaaacacuacagcuggagccucgguggccaugcuucuugccccuugggccuccccccagccccuccuccccuuccugcacccguaccccccgcauuauuacucacgguacgaguggucuuugaauaaagucugagugggcggc

SEQ ID NO: 142 - RNA, 1294 nt, Artificial Sequence
  CONSTRUCT #23
gggaaauaagagagaaaagaagaguaagaagaaauauaagagccaccaugagcggcaacggcaacgccgccgccaccgccgaggagaacagccccaagaugcgggugauccgggugggcacccggaagagccagcuggcgaggauccagacggacagcgugguggcgacgcugaaggcgagcuacccggggcugcaguucgagaucaucgcgaugagcacgacgggcgacaagauccuggacacggcgcugagcaagaucggggagaagagccuguucacgaaggagcuggagcacgcgcuggagaagaacgagguggaccugguggugcacagccugaaggaccugccgacggugcugccgccgggguucacgaucggggcgaucugcaagagggagaacccgcacgacgcggugguguuccacccgaaguucguggggaagacgcuggagacgcugccggagaagagcgugguggggacgagcagccugaggagggcggcgcagcugcagaggaaguucccgcaccuggaguucaggagcaucagggguaaccugaacacgaggcugaggaagcuggacgagcagcaggaguucagcgcgaucauccuggcgacggcggggcugcagaggaugggguggcacaacaggguggggcagauccugcacccggaggagugcauguacgcgguggggcagggcgcgcugggcguggaggugagggcgaaggaccaggacauccuggaccuggugggcgugcugcacgacccggagacgcugcugaggugcaucgcggagagggcguuccugaggcaccuggagggcgggugcagcgugccgguggcggugcacacggcgaugaaggacgggcagcuguaccugacgggagggguguggagccuggacgggagcgacagcauccaggagacgaugcaggcgacgauccacgugccggcgcagcacgaggacgggccggaggacgacccgcagcugguggggaucacggcgaggaacaucccgagggguccgcagcuggcggcgcagaaccuggggaucagccuggcgaaccugcugcugagcaagggagcgaagaacauccuggacguggcgaggcagcugaacgacgcgcacugauaauaguccauaaaguaggaaacacuacagcuggagccucgguggccaugcuucuugccccuugggccuccccccagccccuccuccccuuccugcacccguaccccccgcauuauuacucacgguacgaguggucuuugaauaaagucugagugggcggc

SEQ ID NO: 143 - RNA, 1294 nt, Artificial Sequence
  CONSTRUCT #24
gggaaauaagagagaaaagaagaguaagaagaaauauaagagccaccaugagcggcaacggcaacgccgccgccaccgccgaggagaacagccccaagaugcgggugauccgggugggcacccggaagagccagcuggcccgcauccagaccgacuccgucgucgccacccucaaggccuccuaccccggccuccaguucgagaucaucgccauguccaccaccggcgacaagauccucgacaccgcccucuccaagaucggcgagaagucccucuucaccaaggagcucgagcacgcccucgagaagaacgaggucgaccucgucguccacucccucaaggaccuccccaccguccucccacccggcuucaccaucggcgccaucugcaagcgcgagaacccucacgacgccgucgucuuccaccccaaguucgucggcaagacccucgagacccuccccgagaaguccgucgucggcaccuccucccuccgccgcgccgcccagcuccagcgcaaguucccacaccucgaguuccgcuccauccgcggcaaccucaacacccgccuccgcaagcucgacgagcagcaggaguucuccgccaucauccucgccaccgccggccuccagcgcaugggcuggcacaaccgcgucggccagauccuccaccccgaggagugcauguacgccgucggccagggcgcccucggcgucgagguccgcgccaaggaccaggacauccucgaccucgucggcguccuccacgaccccgagacccuccuccgcugcaucgccgagcgcgccuuccuccgccaccucgagggcggcugcuccguccccgucgccguccacaccgccaugaaggacggccagcucuaccucaccggcggcgucuggucccucgacggcuccgacuccauccaggagaccaugcaggccaccauccacguccccgcccagcacgaggacggccccgaggacgacccucagcucgucggcaucaccgcccgcaacaucccgcgcggcccucagcucgccgcccagaaccucggcaucucccucgccaaccuccuccucuccaagggcgccaagaacauccucgacgucgcccgccagcucaacgacgcccacugauaauaguccauaaaguaggaaacacuacagcuggagccucgguggccaugcuucuugccccuugggccuccccccagccccuccuccccuuccugcacccguaccccccgcauuauuacucacgguacgaguggucuuugaauaaagucugagugggcggc

SEQ ID NO: 144 - RNA, 1294 nt, Artificial Sequence
  CONSTRUCT #27
gggaaauaagagagaaaagaagaguaagaagaaauauaagagccaccaugagcggcaacggcaacgccgccgccaccgccgaggagaacagccccaagaugcgggugauccgggugggcacccggaagagccagcuggcccggauccagaccgacagcgugguggccacccugaaggccagcuaccccggccugcaguucgagaucaucgccaugagcaccaccggcgacaagauccuggacaccgcccugagcaagaucggcgagaagagccuguucaccaaggagcuggagcacgcccuggagaagaacgagguggaccugguggugcacagccugaaggaccugcccaccgugcugccgcccggcuucaccaucggcgccaucugcaagcgggagaacccgcacgacgccgugguguuccaccccaaguucgugggcaagacccuggagacccugcccgagaagagcguggugggcaccagcagccugcggcgggccgcccagcugcagcggaaguucccucaccuggaguuccggagcauccggggcaaccugaacacccggcugcggaagcuggacgagcagcaggaguucagcgccaucauccuggccaccgccggccugcagcggaugggcuggcacaaccgggugggccagauccugcaccccgaggagugcauguacgccgugggccagggcgcccugggcguggaggugcgggccaaggaccaggacauccuggaccuggugggcgugcugcacgaccccgagacccugcugcggugcaucgccgagcgggccuuccugcggcaccuggagggcggcugcagcgugcccguggccgugcacaccgccaugaaggacggccagcuguaccugaccggcggcguguggagccuggacggcagcgacagcauccaggagaccaugcaggccaccauccacgugcccgcccagcacgaggacggccccgaggacgacccucagcuggugggcaucaccgcccggaacaucccacggggcccucagcuggccgcccagaaccugggcaucagccuggccaaccugcugcugagcaagggcgccaagaacauccuggacguggcccggcagcugaacgacgcccacugauaauaguccauaaaguaggaaacacuacagcuggagccucgguggccuagcuucuugccccuugggccuccccccagccccuccuccccuuccugcacccguaccccccgcauuauuacucacgguacgaguggucuuugaauaaagucugagugggcggc

SEQ ID NO: 145 - RNA, 1272 nt, Artificial Sequence
  CONSTRUCT #28
gggaaauaagagagaaaagaagaguaagaagaaauauaagagccaccaugagcggcaacggcaacgccgccgccaccgccgaggagaacagccccaagaugcgggugauccgggugggcacccggaagagccagcuggcccggauccagaccgacagcgugguggccacccugaaggccagcuaccccggccugcaguucgagaucaucgccaugagcaccaccggcgacaagauccuggacaccgcccugagcaagaucggcgagaagagccuguucaccaaggagcuggagcacgcccuggagaagaacgagguggaccugguggugcacagccugaaggaccugcccaccgugcugccgcccggcuucaccaucggcgccaucugcaagcgggagaacccgcacgacgccgugguguuccaccccaaguucgugggcaagacccuggagacccugcccgagaagagcguggugggcaccagcagccugcggcgggccgcccagcugcagcggaaguucccucaccuggaguuccggagcauccggggcaaccugaacacccggcugcggaagcuggacgagcagcaggaguucagcgccaucauccuggccaccgccggccugcagcggaugggcuggcacaaccgggugggccagauccugcaccccgaggagugcauguacgccgugggccagggcgcccugggcguggaggugcgggccaaggaccaggacauccuggaccuggugggcgugcugcacgaccccgagacccugcugcggugcaucgccgagcgggccuuccugcggcaccuggagggcggcugcagcgugcccguggccgugcacaccgccaugaaggacggccagcuguaccugaccggcggcguguggagccuggacggcagcgacagcauccaggagaccaugcaggccaccauccacgugcccgcccagcacgaggacggccccgaggacgacccucagcuggugggcaucaccgcccggaacaucccacggggcccucagcuggccgcccagaaccugggcaucagccuggccaaccugcugcugagcaagggcgccaagaacauccuggacguggcccggcagcugaacgacgcccacugauaauaggcuggagccucgguggccuagcuucuugccccuugggccuccccccagccccuccuccccuuccugcacccguacccccuccauaaaguaggaaacacuacaguggucuuugaauaaagucugagugggcggc

SEQ ID NO: 146 - RNA, 1294 nt, Artificial Sequence
  CONSTRUCT #25
gggaaauaagagagaaaagaagaguaagaagaaauauaagagccaccauguccggaaacggaaacgccgccgcuaccgccgaggaaaauagcccgaagaugagagugauccggguggguaccaggaagucccagcucgccaggauccaaacggacucggugguggccacccucaaggcuagcuacccgggccugcaauucgagaucauugcuauguccaccaccggcgacaagauccuggauacggcccuguccaagaucggcgaaaagagccucuucaccaaggagcuggaacacgcgcucgagaagaacgagguggaccuggucguccacagccucaaggaccugccuacggugcugccgccgggauucaccaucggcgccaucuguaagcgggagaauccgcacgacgccgugguguuccacccuaaguucgugggcaagacccucgagacacugccggaaaaguccgucgugggcaccuccucccugagaagggccgcucagcuccagagaaaguucccgcaccuggaauucaggagcauccggggcaaccugaauacccggcuucgcaagcuggacgagcagcaggaguucagcgccaucauccuggccaccgccggccugcagcggaugggcuggcacaaccgggugggccagauccugcacccggaggagugcauguaugccgugggucagggagcccugggcguggagguccgggccaaggaccaggacauccuggaccucgugggcgugcuccacgacccugaaacccuccugaggugcaucgccgagagggccuuccuccggcaccuggagggcggcuguuccgucccuguggccgugcauaccgccaugaaggacggacagcuguaccugaccggcggcguguggucccuggacggcuccgacagcauccaggaaaccaugcaggccacuauccacgugccggcccagcacgaagacggcccagaggaugacccgcaacuggucggcauuaccgccaggaacauaccaaggggcccgcagcuggccgcccagaaccugggcaucucccuggccaaccugcugcuguccaagggagccaagaacauucuggacguggccaggcagcucaaugaugcccacugauaauaguccauaaaguaggaaacacuacagcuggagccucgguggccaugcuucuugccccuugggccuccccccagccccuccuccccuuccugcacccguaccccccgcauuauuacucacgguacgaguggucuuugaauaaagucugagugggcggc

SEQ ID NO: 147 - RNA, 1294 nt, Artificial Sequence
  CONSTRUCT #26
gggaaauaagagagaaaagaagaguaagaagaaauauaagagccaccaugagcggcaacggcaacgccgccgccaccgcagaggagaauagcccgaagaugagggugauccgagugggcaccaggaagucccagcuugcgcgaauucagaccgacagcgugguggccacccucaaggccuccuacccgggacuccaguucgagaucaucgccaugagcaccacgggagacaagauccuggacaccgcccuguccaagaucggcgaaaagagccucuucaccaaggagcuggagcacgcccuggagaagaacgaggucgaucugguggugcacagccugaaggaccugccgaccguccugccgccgggauucaccaucggugccaucuguaagcgggagaacccgcacgacgccgugguguuccacccgaaguucgucggcaagacccuggaaacccugccggagaaguccguggugggcaccagcagccugaggcgggccgcccagcugcagcggaaguucccgcaccuggaauucaggagcauccggggcaaccugaacacccggcugcggaagcuggacgagcagcaggaguucagcgccaucauccuggccaccgcaggccuccagcgcaugggauggcacaacaggguaggccaaauccugcacccggaggaguguauguacgccgugggccagggagcccugggcguggaggugagagccaaggaccaggacauccuagaccuggucggcgugcugcacgacccggagacacugcugagaugcaucgcggagagagccuuccugcgacaccuggagggcggcugcuccgugccgguggccgugcacaccgccaugaaggacggccagcuguaucugaccggcggcguguggagccuggacggcagcgacuccauccaagaaaccaugcaggcuaccauccacgugccggcccagcacgaggauggaccagaggacgauccucaacuggugggcaucacugccaggaacaucccaagaggcccgcagcuggccgcccagaaccugggcaucagccuggccaaccugcugcuguccaagggcgccaagaacauucucgauguggccaggcagcugaacgaugcccacugauaauaguccauaaaguaggaaacacuacagcuggagccucgguggccaugcuucuugccccuugggccuccccccagccccuccuccccuuccugcacccguaccccccgcauuauuacucacgguacgaguggucuuugaauaaagucugagugggcggc

SEQ ID NO: 148 - RNA, 1294 nt, Artificial Sequence
  CONSTRUCT #27
gggaaauaagagagaaaagaagaguaagaagaaauauaagagccaccaugucgggaaacggcaacgccgccgccacggccgaggagaacagcccgaagaugagagugauuagggugggcacccggaagucccaacucgcgcggauccagaccgacuccgugguggccacccucaaggccagcuacccgggccuccaguucgagauuaucgccauguccaccacaggcgacaagauccucgacaccgcacucucgaagaucggcgagaagucccuguucaccaaggaacuggagcacgcccuggagaagaacgagguggaccugguggugcacucccugaaggaccugccgaccgugcucccaccaggcuucaccaucggcgcaaucuguaagcgcgagaauccgcacgacgccgugguguuccacccaaaguucgugggcaagacccucgaaacccucccggaaaagagcgugguggguaccagcucccugcggagagcugcccagcugcagagaaaguucccgcaucuggaauucaggagcaucaggggaaaucugaauaccagacugcgcaagcuggacgagcagcaggaguucagcgccaucauccuggccaccgccggccugcagcggaugggcuggcacaacagggugggccagauacugcauccggaggaguguauguacgccgugggccagggcgcccucggcguggaggugagagccaaggaccaagacauccuggaccuagugggcgugcugcaugacccugaaacccugcucaggugcaucgccgagagggccuuccugcggcaccuggagggcggcugcagcgugccgguggccguccacaccgccaugaaggacggccagcuguaccugaccggcggcgucuggagccuggacggauccgacagcauccaggaaaccaugcaggccaccauccacgugccggcccagcacgaggacggcccugaggacgacccucagcuggugggcaucaccgcuaggaacaucccaaggggcccgcagcuggccgcccagaaccucggcaucagccuggccaaccugcugcuguccaagggcgccaagaauauccuggacguggccaggcagcugaacgacgcccacugauaauaguccauaaaguaggaaacacuacagcuggagccucgguggccaugcuucuugccccuugggccuccccccagccccuccuccccuuccugcacccguaccccccgcauuauuacucacgguacgaguggucuuugaauaaagucugagugggcggc

SEQ ID NO: 149 - RNA, 164 nt, Artificial Sequence
  3'UTR (miR142+miR126 variant 1)
ugauaauaguccauaaaguaggaaacacuacagcuggagccucgguggccaugcuucuugccccuugggccuccccccagccccuccuccccuuccugcacccguaccccccgcauuauuacucacgguacgaguggucuuugaauaaagucugagugggcggc

SEQ ID NO: 150 - RNA, 164 nt, Artificial Sequence
  3'UTR (miR142+miR126 variant 2)
ugauaauaguccauaaaguaggaaacacuacagcuggagccucgguggccuagcuucuugccccuugggccuccccccagccccuccuccccuuccugcacccguaccccccgcauuauuacucacgguacgaguggucuuugaauaaagucugagugggcggc

SEQ ID NO: 151 - RNA, 142 nt, Artificial Sequence
  3'UTR (miR142)
ugauaauaggcuggagccucgguggccuagcuucuugccccuugggccuccccccagccccuccuccccuuccugcacccguacccccuccauaaaguaggaaacacuacaguggucuuugaauaaagucugagugggcggc

SEQ ID NO: 152 - protein, 361 aa, Artificial Sequence
  PBGD GoF I291M/N340S
MSGNGNAAATAEENSPKMRVIRVGTRKSQLARIQTDSVVATLKASYPGLQFEIIAMSTTGDKILDTALSKIGEKSLFTKELEHALEKNEVDLVVHSLKDLPTVLPPGFTIGAICKRENPHDAVVFHPKFVGKTLETLPEKSVVGTSSLRRAAQLQRKFPHLEFRSIRGNLNTRLRKLDEQQEFSAIILATAGLQRMGWHNRVGQILHPEECMYAVGQGALGVEVRAKDQDILDLVGVLHDPETLLRCIAERAFLRHLEGGCSVPVAVHTAMKDGQLYLTGGVWSLDGSDSMQETMQATIHVPAQHEDGPEDDPQLVGITARNIPRGPQLAAQNLGISLASLLLSKGAKNILDVARQLNDAH

SEQ ID NO: 153 - DNA, 1083 bp, Artificial Sequence
  I291M / N340S
atgagcgggaacggcaacgcggcagccaccgctgaggaaaactctccaaaaatgagagtcattagggtgggcaccagaaagagtcaactcgcaaggatccagaccgactctgtggtggccactctaaaagcgagctaccccggactccagttcgaaatcatcgcgatgagcaccaccggcgataaaatcctagataccgccttgagcaagatcggcgagaagagcctctttaccaaggagctggagcacgccctggagaaaaacgaggtggatctggtggtccatagcctaaaggatctccctacagtgctgccccccgggtttaccatcggcgccatttgtaagcgggagaacccgcacgacgcagtggtcttccaccccaagtttgtgggcaagacactggagaccctgccggaaaagtccgtggtgggcacctccagcctgagacgagccgcccagctgcagcgcaagtttccccacctggagtttaggagcatcaggggaaacctcaacaccagactgagaaagctggacgaacagcaggagttcagcgccatcatcctggcgactgcaggactccagaggatgggctggcataatagggtgggacaaattctgcaccccgaggaatgcatgtatgctgtggggcagggcgcactcggggtggaggtgcgggccaaggatcaggacatcctggacctcgtgggcgtgcttcacgacccggaaaccctgctgaggtgcatagcagaaagagctttcctgcggcacctggaggggggatgcagcgtccctgtggccgtgcatacagccatgaaggacggccagctgtacttgactggtggcgtctggtcccttgatggctctgacagcatgcaggaaacaatgcaggccactatccacgtgcctgcccagcacgaggacggccccgaggacgaccctcagctggtgggcattaccgccagaaatatccctaggggaccccagctggctgcccaaaacttgggcatcagcctggccagcctgctgctgagcaaaggagctaaaaacatcctggatgtggccaggcagctgaatgacgcccac

SEQ ID NO: 154 - protein, 604 aa, Artificial Sequence
  APOA1-PBGD
MDEPPQSPWDRVKDLATVYVDVLKDSGRDYVSQFEGSALGKQLNLKLLDNWDSVTSTFSKLREQLGPVTQEFWDNLEKETEGLRQEMSKDLEEVKAKVQPYLDDFQKKWQEEMELYRQKVEPLRAELQEGARQKLHELQEKLSPLGEEMRDRARAHVDALRTHLAPYSDELRQRLAARLEALKENGGARLAEYHAKATEHLSTLSEKAKPALEDLRQGLLPVLESFKVSFLSALEEYTKKLNTQSGNGNAAATAEENSPKMRVIRVGTRKSQLARIQTDSVVATLKASYPGLQFEIIAMSTTGDKILDTALSKIGEKSLFTKELEHALEKNEVDLVVHSLKDLPTVLPPGFTIGAICKRENPHDAVVFHPKFVGKTLETLPEKSVVGTSSLRRAAQLQRKFPHLEFRSIRGNLNTRLRKLDEQQEFSAIILATAGLQRMGWHNRVGQILHPEECMYAVGQGALGVEVRAKDQDILDLVGVLHDPETLLRCIAERAFLRHLEGGCSVPVAVHTAMKDGQLYLTGGVWSLDGSDSMQETMQATIHVPAQHEDGPEDDPQLVGITARNIPRGPQLAAQNLGISLASLLLSKGAKNILDVARQLNDAH

SEQ ID NO: 155 - DNA, 1812 bp, Artificial Sequence
  APOA1-PBGD
atggacgaaccaccccagtcaccctgggatagagtcaaagacctggccactgtgtacgtggacgtgctgaaagatagcgggcgggattacgtctcgcagttcgagggctccgccttaggcaaacagctgaacctcaaactgctggacaattgggactccgtcactagcacattctccaagctgagagagcagctgggacctgtgactcaggagttctgggacaatctggagaaggaaactgagggcctgaggcaggagatgtccaaggatctggaggaggttaaggcaaaggtgcaaccctacctcgacgacttccagaaaaaatggcaagaagagatggagctataccggcaaaaggtggagcctctccgggccgagctccaggagggcgctcggcaaaagctgcatgagctgcaggagaagctgagccccctcggcgaggaaatgcgtgatagagcacgtgcccacgtggacgccctgcggacacatctggctccctacagcgatgagcttaggcagagactggccgccagactcgaagctctgaaggagaatggcggcgctcggctggccgagtatcatgccaaggccaccgagcatttgtccactctgagtgagaaggctaagcctgccctggaggacctgaggcagggcctgttacccgtgctggagagcttcaaggtgagctttctgagcgccttggaggagtacaccaaaaaactgaacacccagagcggcaacggaaacgccgccgctaccgccgaggagaacagccctaagatgagggtgatcagggtgggcacccgcaagtcccagcttgcacgaatccagaccgattcagtcgtggcgaccctgaaggcatcttaccccggcctgcagttcgagattatcgccatgtctacaaccggcgacaagatcctcgataccgccctgagcaagatcggcgaaaagagcctgttcaccaaagagctagagcacgccctcgagaaaaacgaggtggaccttgtggtgcatagcctcaaggatcttcctaccgtgctgccccccggtttcaccattggggcaatctgcaagagggagaatccccacgatgccgtggtgttccatcccaaattcgtgggcaaaacgttggagaccctgcccgagaaaagtgtggtcggcactagcagcctgagaagagcggcccaacttcagagaaagtttcctcacctggagttcaggagcatccggggcaacctgaacacccggctgcggaagctggacgagcagcaagagttcagcgctatcattctagcaacagccggcctgcagcgcatgggatggcataacagggtgggacagattctccaccccgaggaatgcatgtacgccgttggccaaggcgcgctgggggtggaggtcagagcaaaggaccaggacattcttgatctggtcggggtgctgcacgaccccgagacactgctgagatgcatagctgagcgggccttcctgcggcatctggagggcggctgctcagtccccgtggccgtgcacacagccatgaaggacggccagctgtacctgaccggaggggtgtggagcttggacggcagcgattcaatgcaggagacaatgcaggcaaccatccacgttccagctcagcacgaggatggccccgaagatgaccctcagctggtggggattactgctagaaacatcccccgcggcccccagctggccgcccaaaacctgggaatctctctggcctccctgctcctctctaaaggagccaagaatattctggacgtggcacggcagctcaacgatgcacac

SEQ ID NO: 156 - RNA, 85 nt, Artificial Sequence
  miR-126
cgcuggcgacgggacauuauuacuuuugguacgcgcugugacacuucaaacucguaccgugaguaauaaugcgccguccacggca

SEQ ID NO: 157 - RNA, 22 nt, Artificial Sequence
  miR 126-3p sequence
ucguaccgugaguaauaaugcg

SEQ ID NO: 158 - RNA, 22 nt, Artificial Sequence
  miR-126-3p binding site
cgcauuauuacucacgguacga

SEQ ID NO: 159 - RNA, 21 nt, Artificial Sequence
  miR 126-5p sequence
cauuauuacuuuugguacgcg

SEQ ID NO: 160 - RNA, 21 nt, Artificial Sequence
  miR-126-5p binding site
cgcguaccaaaaguaauaaug

SEQ ID NO: 161 - RNA, 133 nt, Artificial Sequence
  3'UTR with miR 142-3p binding site
gcuggagccucgguggccaugcuucuugccccuugggccuccccccagccccuccuccccuuccugcacccguacccccuccauaaaguaggaaacacuacaguggucuuugaauaaagucugagugggcggc

SEQ ID NO: 162 - RNA, 141 nt, Artificial Sequence
  3'UTR with miR 126-3p binding site
ugauaauaggcuggagccucgguggccaugcuucuugccccuugggccuccccccagccccuccuccccuuccugcacccguaccccccgcauuauuacucacgguacgaguggucuuugaauaaagucugagugggcggc

SEQ ID NO: 163 - RNA, 119 nt, Artificial Sequence
  (3' UTR, no miR binding sites variant 2)
ugauaauaggcuggagccucgguggccuagcuucuugccccuugggccuccccccagccccuccuccccuuccugcacccguacccccguggucuuugaauaaagucugagugggcggc

SEQ ID NO: 164 - RNA, 141 nt, Artificial Sequence
  (3' UTR with miR 126-3p binding site variant 3)
ugauaauaggcuggagccucgguggccuagcuucuugccccuugggccuccccccagccccuccuccccuuccugcacccguaccccccgcauuauuacucacgguacgaguggucuuugaauaaagucugagugggcggc

SEQ ID NO: 165 - RNA, 188 nt, Artificial Sequence
  3' UTR with 3 miR 142-3p binding sites
ugauaauaguccauaaaguaggaaacacuacagcuggagccucgguggccaugcuucuugccccuugggccuccauaaaguaggaaacacuacauccccccagccccuccuccccuuccugcacccguacccccuccauaaaguaggaaacacuacaguggucuuugaauaaagucugagugggcggc

SEQ ID NO: 166 - RNA, 140 nt, Artificial Sequence
  3'UTR with miR 142-5p binding site
ugauaauaggcuggagccucgguggccaugcuucuugccccuugggccuccccccagccccuccuccccuuccugcacccguacccccaguagugcuuucuacuuuaugguggucuuugaauaaagucugagugggcggc

SEQ ID NO: 167 - RNA, 182 nt, Artificial Sequence
  3'UTR with 3 miR 142-5p binding sites
ugauaauagaguagugcuuucuacuuuauggcuggagccucgguggccaugcuucuugccccuugggccaguagugcuuucuacuuuauguccccccagccccuccuccccuuccugcacccguacccccaguagugcuuucuacuuuaugguggucuuugaauaaagucugagugggcggc

SEQ ID NO: 168 - RNA, 184 nt, Artificial Sequence
  3'UTR with 2 miR 142-5p binding sites and 1 miR 142-3p binding site
ugauaauagaguagugcuuucuacuuuauggcuggagccucgguggccaugcuucuugccccuugggccuccauaaaguaggaaacacuacauccccccagccccuccuccccuuccugcacccguacccccaguagugcuuucuacuuuaugguggucuuugaauaaagucugagugggcggc

SEQ ID NO: 169 - RNA, 142 nt, Artificial Sequence
  3'UTR with miR 155-5p binding site
ugauaauaggcuggagccucgguggccaugcuucuugccccuugggccuccccccagccccuccuccccuuccugcacccguacccccaccccuaucacaauuagcauuaaguggucuuugaauaaagucugagugggcggc

SEQ ID NO: 170 - RNA, 188 nt, Artificial Sequence
  3' UTR with 3 miR 155-5p binding sites
ugauaauagaccccuaucacaauuagcauuaagcuggagccucgguggccaugcuucuugccccuugggccaccccuaucacaauuagcauuaauccccccagccccuccuccccuuccugcacccguacccccaccccuaucacaauuagcauuaaguggucuuugaauaaagucugagugggcggc

SEQ ID NO: 171 - RNA, 188 nt, Artificial Sequence
  3'UTR with 2 miR 155-5p binding sites and 1 miR 142-3p binding site
ugauaauagaccccuaucacaauuagcauuaagcuggagccucgguggccaugcuucuugccccuugggccuccauaaaguaggaaacacuacauccccccagccccuccuccccuuccugcacccguacccccaccccuaucacaauuagcauuaaguggucuuugaauaaagucugagugggcggc

SEQ ID NO: 172 - RNA, 142 nt, Artificial Sequence
  3'UTR with miR 142-3p binding site, P3 insertion
ugauaauaggcuggagccucgguggccaugcuucuugccccuugggccuccauaaaguaggaaacacuacauccccccagccccuccuccccuuccugcacccguacccccguggucuuugaauaaagucugagugggcggc

SEQ ID NO: 173 - RNA, 22 nt, Artificial Sequence
  miR 146-3p sequence
ccucugaaauucaguucuucag

SEQ ID NO: 174 - RNA, 22 nt, Artificial Sequence
  miR 146-5p sequence
ugagaacugaauuccauggguu

SEQ ID NO: 175 - RNA, 22 nt, Artificial Sequence
  miR 155-3p sequence
cuccuacauauuagcauuaaca

SEQ ID NO: 176 - RNA, 23 nt, Artificial Sequence
  3' UTR
uuaaugcuaaucgugauaggggu

SEQ ID NO: 177 - RNA, 22 nt, Artificial Sequence
  miR 16-3p sequence
ccaguauuaacugugcugcuga

SEQ ID NO: 178 - RNA, 22 nt, Artificial Sequence
  miR 16-5p sequence
uagcagcacguaaauauuggcg

SEQ ID NO: 179 - RNA, 21 nt, Artificial Sequence
  miR 21-3p sequence
caacaccagucgaugggcugu

SEQ ID NO: 180 - RNA, 22 nt, Artificial Sequence
  miR 21-5p sequence
uagcuuaucagacugauguuga

SEQ ID NO: 181 - RNA, 22 nt, Artificial Sequence
  miR 223-3p sequence
ugucaguuugucaaauacccca

SEQ ID NO: 182 - RNA, 22 nt, Artificial Sequence
  miR 223-5p sequence
cguguauuugacaagcugaguu

SEQ ID NO: 183 - RNA, 22 nt, Artificial Sequence
  miR 24-3p sequence
uggcucaguucagcaggaacag

SEQ ID NO: 184 - RNA, 22 nt, Artificial Sequence
  miR 24-5p sequence
ugccuacugagcugauaucagu

SEQ ID NO: 185 - RNA, 21 nt, Artificial Sequence
  miR 27-3p sequence
uucacaguggcuaaguuccgc

SEQ ID NO: 186 - RNA, 22 nt, Artificial Sequence
  miR 27-5p sequence
agggcuuagcugcuugugagca

SEQ ID NO: 187 - RNA, 23 nt, Artificial Sequence
  miR 155-5p sequence
uuaaugcuaauugugauaggggu

SEQ ID NO: 188 - RNA, 23 nt, Artificial Sequence
  miR 155-5p binding site
accccuaucacaauuagcauuaa

SEQ ID NO: 189 - RNA, 70 nt, Artificial Sequence
  5' UTR with miR142-3p binding site at position p1
gggaaauaagaguccauaaaguaggaaacacuacaagaaaagaagaguaagaagaaauauaagagccacc

SEQ ID NO: 190 - RNA, 70 nt, Artificial Sequence
  5' UTR with miR142-3p binding site at position p2
gggaaauaagagagaaaagaagaguaauccauaaaguaggaaacacuacagaagaaauauaagagccacc

SEQ ID NO: 191 - RNA, 70 nt, Artificial Sequence
  5' UTR with miR142-3p binding site at position p3
gggaaauaagagagaaaagaagaguaagaagaaauauaauccauaaaguaggaaacacuacagagccacc

SEQ ID NO: 192 - RNA, 188 nt, Artificial Sequence
  (3' UTR with 3 miR 142-3p binding sites variant 2)
ugauaauaguccauaaaguaggaaacacuacagcuggagccucgguggccuagcuucuugccccuugggccuccauaaaguaggaaacacuacauccccccagccccuccuccccuuccugcacccguacccccuccauaaaguaggaaacacuacaguggucuuugaauaaagucugagugggcggc

SEQ ID NO: 193 - RNA, 142 nt, Artificial Sequence
  (3'UTR with miR 142-3p binding site, P1 insertion variant 2)
ugauaauaguccauaaaguaggaaacacuacagcuggagccucgguggccuagcuucuugccccuugggccuccccccagccccuccuccccuuccugcacccguacccccguggucuuugaauaaagucugagugggcggc

SEQ ID NO: 194 - RNA, 142 nt, Artificial Sequence
  (3'UTR with miR 142-3p binding site, P2 insertion variant 2)
ugauaauaggcuggagccucgguggcuccauaaaguaggaaacacuacacuagcuucuugccccuugggccuccccccagccccuccuccccuuccugcacccguacccccguggucuuugaauaaagucugagugggcggc

SEQ ID NO: 195 - RNA, 181 nt, Artificial Sequence
  (3'UTR with 3 miR 142-5p binding sites)
ugauaauagaguagugcuuucuacuuuauggcuggagccucgguggccaugcuucuugccccuugggccaguagugcuuucuacuuuauguccccccagccccucuccccuuccugcacccguacccccaguagugcuuucuacuuuaugguggucuuugaauaaagucugagugggcggc

SEQ ID NO: 196 - RNA, 142 nt, Artificial Sequence
  (3'UTR with miR 142-3p binding site, P3 insertion variant 2)
ugauaauaggcuggagccucgguggccuagcuucuugccccuugggccuccauaaaguaggaaacacuacauccccccagccccuccuccccuuccugcacccguacccccguggucuuugaauaaagucugagugggcggc

SEQ ID NO: 197 - RNA, 142 nt, Artificial Sequence
  (3'UTR with miR 155-5p binding site variant 2)
ugauaauaggcuggagccucgguggccuagcuucuugccccuugggccuccccccagccccuccuccccuuccugcacccguacccccaccccuaucacaauuagcauuaaguggucuuugaauaaagucugagugggcggc

SEQ ID NO: 198 - RNA, 188 nt, Artificial Sequence
  (3' UTR with 3 miR 155-5p binding sites variant 2)
ugauaauagaccccuaucacaauuagcauuaagcuggagccucgguggccuagcuucuugccccuugggccaccccuaucacaauuagcauuaauccccccagccccuccuccccuuccugcacccguacccccaccccuaucacaauuagcauuaaguggucuuugaauaaagucugagugggcggc

SEQ ID NO: 199 - RNA, 188 nt, Artificial Sequence
  (3'UTR with 2 miR 155-5p binding sites and 1 miR 142-3p binding site variant 2)
ugauaauagaccccuaucacaauuagcauuaagcuggagccucgguggccuagcuucuugccccuugggccuccauaaaguaggaaacacuacauccccccagccccuccuccccuuccugcacccguacccccaccccuaucacaauuagcauuaaguggucuuugaauaaagucugagugggcggc